European Patent Application EP 4 737 566 A1, published May 6, 2026. Title: Cas12蛋白及其应用. Applicant: 广州瑞风生物科技有限公司. The sequence listing filed with the application follows.

SEQUENCE LISTING (287 sequences)

SEQ ID NO: 1 - protein, 891 aa, synthetic construct
MKLSNTLRIPRTIQLKVILDPKIKNELDLVISKSHSKMLDFGMAIIALRGEETHIRREKTIEILDSGYWKEYRKDRLGDYNEGHEEKLKSVFDAVAAKGKTRDFLCPIFRKITKANASNLSDIKALRQDGVLPFALNTTELTSTDHVNDYACWRSITSHIAGWKSNDARTKSAYSNLLKVVGENTPDEVGMGLLNELIDKFGSFITEKFLKKFTKFGFDIRSLGEEMAWAKSKESKVSIWKKLFRYQIAKTQLDRSRPMACLNLPDGTTHTRQIPYGDCYVPFAISIDGNGEFFVSLGTKTPIKLKCMKTNHIRDVKITYETVASPTKQNPEKTREARVFYFRRGNHSDKQLVRAELAEIALQRNGDDYYIVLPLQIDIERNVNAVDLYNRRFEEPKLPYAPLATNQTITCLDLGIDPLGAFGVWTIEGGRKIEIAKGAIGGVVDSSYNRKIRELRSKMRKVGQIIDYLKVVQFGKEVPSRNREKWKNAFRDLGVPVIDDFLSKSLVFDHVENKPWKGKKWTLTIDSDVVDILRTFISEKKRECDRTYRELKRYDIYPSRHCGVASETFGFACLVKEHISLTKKWKFYGRPPLGKFELRAGFESETEYLKNLKKDSIKKNAHAFVNDGCLKYGSKTIVIENLDFNRSGNSSDNEFLALWSSNTLIKWINHFADQYGIVVATVNKWGTSQRDPVTGLWGFRPKDQKWHSYGNKKDLNVRRDGKIVTINSDIDAATENLLNVYLDPTFHVYSMRVEEIADPGSIGIGPGRAFKPVWKEELESEDSASSKKWKLSTIKHQLIRMYNSYRVFILESGDVINVSADLFLSVKTKGEEQTFTREGVRWISRDQRDEIESQIREKMGCKSMDLNWISANLYEQEVCDKKQKNTLSRAG

SEQ ID NO: 2 - protein, 854 aa, synthetic construct
MYAFQPFSELMVEFYEEFIKSRRGRSFSSFLYSSNTLKETSKLSQKFFFLRKAGVFPIGLPPEVEYSAMFYNVVAEVHQKLGQFESTLENYLEARAEWEAALVGAKLSEIKLYEAFLFSFKDKNDMEKLNARGYTRFIRSWNGKLNKKDEVEIESMHQYFVELQKTNPDKVFEEKDRYRFGYGPDVLNLIYNDYRNLWDVIGDSSYVDIIKGSFNWLKKEIHISSFNRPISIIFGHNFSGYGLDVSNEHLTFDLNMNMTKDKVSVVKSGGNLLLRGRSKRLRDAKIVAADVDNCAYRLYHKKSDNPEAPTFEGNIKEPSLRCKPETRELWMDIPLSNSTSSNSIEKMWELRAHFSSAYAPSKRQKKHKIEDGPYRIAAYDVGMANPFVCVIFEIEMKNNQVVDIDRVATEKCYYNDDSNLQRIKDLKDKIIVTKKLISYSVRLCYGEITTIPLLFGKRGQYNWIEILGLRKNDRQTDQEICDEYIESVKKLPVVDEDIVKHWRTKLVETPLKDIMHSISIEISKLRNKCKLKGQERSDYIKANSTVDMGLFLMAETIKEFVSLQKKFSYKEEDCCKNYWKYYNGLRRKIGSSLASAMVNCAIKHKACLMVMEELDVTMSSGDLSGENRMKAIWAMGQTKVWLKNKANLEGILIAEVDAFLTSQIDPETQKMGYRKGRYIYVNRNNKYVKIDSDEAAAVNVFMKFISHGTTIARLNFRQLEGDTYVASVSDYVTIKGKADGKTENIPQKRRQGIFLACFGDKKSIKLKMAENGEFIVAKSSPTKKQLEGLNALPVKEVKKVEVFRNGDKIVGYAALKDGIKKEFEELVKEDEQKAIIPVAKVLNKNKVRILGKQE

SEQ ID NO: 3 - protein, 887 aa, synthetic construct
MPKKNENWDVMRCQALRFAVPLDEKTAKFYSDMQSDFNDLYPRMMMWSLIPHIQEDKDGIVKVKHVDDVLTELKKDVPAELLEDVLLIGDVISRRPRDEASSFYGLFSKSYKSTGKANFNDAKIKFLNSLGNLTDEELSVFISKDESFKLMSVAEWRTVQADIDSGTKIKKAWEKISKKIANKVNASYARVRNAFKQMSRQPNSRGYCSTLAELLRRQISSAYKKYVVHLADGKKISEQSAIIQKSNEVLFNAIAELWNRLDALGNGLSEKTLMRAVKMAAEKEDPLNSNIEEMATEVQKPEFDCIIKADHKDVRKAYRGVKLKRRYDQRKIYPSMSSLKNDQKIPFGLTSLANFEAKMSEGRLIVSFEGGPGLACQRSHYFNDLDCVKIANKKHYQITFNHRLKSKKKYAVSKKYIGVIKEIGLQQKNGSYYITLPYTLTHSPINRNLECFFKTAQPDVKKYDLPDEIRVAGFDLNVGDPLVGGIAVFKKNGDGPLIALDYGKGHMVQQPETICPDTKLSNRIRALTKITYKIVHAIRGYKKSVNNNMPLDEKIESFLKKIKSPSPVIRCRIQTWVKQIGIRLRKLHHLVRASGYKELSESLRLLEAQDAMKSLIESFKRIHLKKGQSLPKKKEFDTTRQNFRKDISRRYASKVIQYSKGCNLIVIEDLKSDFDRDNKNNSLLRLFSSGSLIKSIQDAAHKEGIGVVLADPAGTSRTDCVTGEIGYRNTKIDKTRLYVVRDGVLGTVNADKNAVINVIARGVGHSVVPYKVFVRSTVEKTTVEDEEEKNIGKRVKRFYTTLYGSTKPVFTLEDNKTIKVVKKASKKMQKLTNCYIYVRGKRLVTEAEHRAEEKRIENRVTSGEISVGMKLEPCPVKGFLAFKYNDK

SEQ ID NO: 4 - protein, 1068 aa, synthetic construct
MAKKDFIARPYNSFLLPNDRKLAYLEETWNAYKSIKTVLHRFLIAAYGAIPFQTFAKTIENTQEDELQLAYAVRMFRLVPKDFSKNESNISPDMLIRKLCSYTNINEVPANVASYVNSNYDPEKYKWIDSRNEAISLSKEIGIKLDELADYATTMLWEDWLPLNKDTVNGWGTTSGLFGAGKKEDRTQKVQMLNALLLGLKNNPPKDYKQYSTILLKAFDAKSWEEAVKIYKGECSGRTSSYLTEKHGDISPETLEKLIQSIERDIADKQHSINLPKREEIKAYLERQSGTPYNLNLWSQALHNAMSSIKKTDTRNFNSTLEKYEKEIQLKECLQDGDDVELLGNKFFSSPYHKTNDVFVICSEHIGTNRKYNVVEQMYQLASEHADFETVFTLLKDEYEEKGIKTPIKNILEYIWNNKNVPVGTWGRIAKYNHLKDRLAGIKAHPTVECNRGMTFGNSAMVGEVMRSNRISTSTKNKGQILAQMHNDRPVGSNNMIWLEMTLLNNGKWQKHHIPTHNNKFFEEVHAFNPELKQSVNVRNRMYRSQNYSQLPTSLTDGLKGNPKAKIFKRQYRALNNMTANVIDPKLSFIVNKKDGRFEISIIHNVEVIRARRDVLVGDYLVGMDQNQTASNTYAVMQVVQPNTPDSHEFRNQWVKFIESGKIESSTLNSRGEYIDQLSHDGVDLQEIKDSEWIPAAEKFLNKLGAINKDGTPISISNTSKRAYTFNSIYFKILLNYLRANDVDLNLVREEILRIANGRFSPMRLGSLSWTTLKMLGNFRNLIHSYFDHCGFKEMPERESKDKTMYDLLMQTITKLTNKRAERTSRIAGSLMNVAHKYKIGTSVVHVVVEGSLSKTDKSSSKGNNRNTTDWCSRAVVKKLEDMCVFYGFNLKAVSAHYTSHQDPLVHRADYDDPKVALRCRYSSYSRADFEKWGEKSFAAVIRWATDKKSNTCYKVGAVEFFKNYKIPEDKITKKLTIKEFLEIMCAESHYPNEYDDILIPRRGGRIYLTTKKLLSDSTHQRESVHSHTAVVKMNGKEYYSSDADEVAAINICLHDWVVPCKRKPKDE

SEQ ID NO: 5 - protein, 1068 aa, synthetic construct
MAKKDFIARPYNSFLLPNDRKLAYLEETWNAYKSIKTVLHRFLIAAYGAIPFQTFAKTIENTQEDELQLAYAVRMFRLVPKDFSKNENNIPPDMLISKLASYTNINQSPTNVLSYVNSNYDPEKYKWIDSRNEAISLSKEIGIKLDELADYATTMLWEDWLPLNKDTVNGWGTTSGLFGAGKKEDRTQKVQMLNALLLGLKNNPPKDYKQYSTILLKAFDAKSWEEAVKIYKGECSGRTSSYLTEKHGDISPETLEKLIQSIERDIADKQHSINLPKREEIKAYLERQSGTPYNLNLWSQALHNAMSSIKKTDTRNFNSTLEKYEKEIQLKECLQHGDDVELLGNKFFSSPYHKTNDVFVICSEHIGTNRKYNVVEQMYQLASEHADFETVFTLLKDEYEEKGIKTPIKNILEYIWNNKNVPVGTWGRIAKYNQLKDRLAGIKANPTVECNRGMTFGNSAMVGEVMRSNRISTSTKNKGQILAQMHNDRPVGSNNMIWLEMTLLNNGKWQKHHIPTHNNKFFEEVHAFDPELKQSVNVRNRMYRSQNYSQLPTSLTDGLQGNPKAKIFKRQYRALNNMTANVIDPKLSFIVNKKDGRFEISIIHNVEVIRARRDVLVGDYLVGMDQNQTASNTYAVMQVVKPNTPDSHEFRNQWVKFIESGKIESSTLNSRGEYIDQLSHDGVDLQEIKDSEWIPAAEKFLNKLGAINKDGTPISISNTSKRAYTFNSIYFKILLNYLRANDVDLNLVREEILRIANGRFSPMRLGSLSWTTLKMLGNFRNLIHSYFDHCGFKEMPERESKDKTMYDLLMQTITKLTNKRAERTSRIAGSLMNVAHKYKIGTSVVHVVVEGSLSKTDKSSSKGNNRNTTDWCSRAVVKKLEDMCVFYGFNLKAVSAHYTSHQDPLVHRADYDDPKVALRCRYSSYSRADFEKWGEKSFAAVIRWATDKKSNTCYKVGAVEFFKNYKIPEDKITKKLTIKEFVEIMCAESHYPNEYDDILIPRRGGRIYLTTKKLLSDSTHQRESVHSHTAVVKMNGKEYYSSDADEVAAINICLHDWVVPCKRKPKDE

SEQ ID NO: 6 - protein, 956 aa, synthetic construct
LSYVNSNYDPEKYKWIDSRNEAISLSKEIGIKLDELADYATTMLWEDWLPLNKDTVNGWGTTSGLFGAGKKEDRTQKVQMLNALLLGLKNNPPKDYKQYSTILLKAFDAKSWEEAVKIYKGECSGRTSSYLTEKHGDISPETLEKLIQSIERDIADKQHSINLPKREEIKAYLERQSGTPYNLNLWSQALHNAMSSIKKTDTRNFNSTLEKYEKEIQLKECLQDGDDVELLGNKFFSSPYHKTNDVFVICSEHIGTNRKYNVVEQMYQLASEHADFETVFTLLKDEYEEKGIKTPIKNILEYIWNNKNVPVGTWGRIAKYNHLKDRLAGIKAHPTVECNRGMTFGNSAMVGEVMRSNRISTSTKNKGQILAQMHNDRPVGSNNMIWLEMTLLNNGKWQKHHIPTHNNKFFEEVHAFNPELKQSVNVRNRMYRSQNYSQLPTSLTDGLQGNPKAKIFKRQYRALNNMTANVIDPKLSFIVNKKDGRFEISIIHNVEVIRARRDVLVGDYLVGMDQNQTASNTYAVMQVVQPNTPDSHEFRNQWVKFIESGKIESSTLNSRGEYIDQLSHDGVDLQEIKDAEWIPAAEKFLNKLGATNKDGTPISISNMSKRVYVFNSIYFKILLNYLRANDVDLNLVREEILRIANGRFSPMRLGSLSWTTLKMLGNFRNLIHSYFDHCGFKEMPERESKDKTMYDLLMQTITKLTNKRAERTSRIAGSLMNVAHKYKIGTSVVHVVVEGSLSKTDKSSSKGNNRNTTDWCSRAVVKKLEDMCVFYGFNLKAVSAHYTSHQDPLVHRADYDDPKVALRCRYSSYSRADFEKWGEKSFAAVIRWATDKKSNTCYKVGAVEFFKNYKIPEDKITKKLTIKEFVEIMCAESHYPNEYDDILIPRRGGRIYLTTKKLLSDSTHQRESVHSHTAVVKMNGKEYYSSDADEVAAINICLHDWVVPCKRKPKDE

SEQ ID NO: 7 - protein, 1068 aa, synthetic construct
MAKKDFIARPYNSFLLPNDRKLAYLEETWNAYKSIKTVLHRFLIAAYGAIPFQTFAKTIENTQEDELQLAYAVRMFRLVPKDFSKNESNISPDMLIRKLCSYTNINEVPANVASYVNSNYDPEKYKWIDSRNEAISLSKEIGIKLDELADYATTMLWEDWLPLNKDTVNGWGTTSGLFGAGKKEDRTQKVQMLNALLLGLKNNPPKDYKQYSTILLKAFDAKSWEEAVKIYKGECSGRTSSYLTEKHGDISPETLEKLIQSIERDIADKQHSINLPKREEIKAYLERQSGTPYNLNLWSQALHNAMSSIKKTDTRNFNSTLEKYEKEIQLKECLQDGDDVELLGNKFFSSPYHKTNDVFVICSEHIGTNRKYNVVEQMYQLASEHADFETVFTLLKDEYEEKGIKTPIKNILEYIWNNKNVPVGTWGRIAKYNQLKDRLAGIKANPTVECNRGMTFGNSAMVGEVMRSNRISTSTKNKGQILAQMHNDRPVGSNNMIWLEMTLLNNGKWQKHHIPTHNNKFFEEVHAFNPELKQSVNVRNRMYRSQNYSQLPTSLTDGLKGNPKAKIFKRQYRALNNMTANVIDPKLSFIVNKKDGRFEISIIHNVEVIRARRDVLVGDYLVGMDQNQTASNTYAVMQVVQPNTPDSHEFRNQWVKFIESGKIESSTLNSRGEYIDQLSHDGVDLQEIKDAEWIPAAEKFLNKLGATNKDGTPISISNMSKRVYVFNSIYFKILLNYLRANDVDLNLVREEILRIANGRFSPMRLGSLSWTTLKMLGNFRNLIHSYFDHCGFKEMPERESKDKTMYDLLMQTITKLTNKRAERTSRIAGSLMNVAHKYKIGTSVVHVVVEGSLSKTDKSSSKGNNRNTTDWCSRAVVKKLEDMCVFYGFNLKAVSAHYTSHQDPLVHRADYDDPKVALRCRYSSYSRADFEKWGEKSFAAVIRWATDKKSNTCYKVGAVEFFKNYKIPEDKITKKLTIKEFVEIMCAESHYPNEYDDILIPRRGGRIYLTTKKLLSDSTHQRESVHSHTAVVKMNGKEYYSSDADEVAAINICLHDWVVPCKRKPKDE

SEQ ID NO: 8 - protein, 909 aa, synthetic construct
MDQEQRKFQRCGVLKLEKISEKSESYYNDFQEDYRKFFNLIFSWMEKGYRYFDEDEKIHYVKPKKTALAKTQNYDKETCRLIDDFMSVLIKGGTDASSCYCLFYEKYNPKDSKKYTEFVKLSLENLHNQELQDETIEKLDPDSSISKDEWINVHIPNLKDPENRKSYWENTLGKLLVNQGRSLGKNIRERLQISCKHPSDVTYCNRLIKAIGEQIRSFYEKANLHEQERDELFAQIKSFENDDLYQKVCEFGIVLEYEGSGLSKYVLNHGVKQALKPVNDSTIKFQVDILSQDRFRSIVEANEKDLLAAYKKYKLRSKLANKLMTCKYVAKSSLKNDFKISIGQSSLGSFRFNQENGKLVVSSDIGDFNCIPSHYFSQLDCKVIKNSKKQIVGYEISFCHKQKRKPSTKSNLPYFGNKITGIVKELGLQRKNGEFFLSFPYAIHHDHTNFKLATYFNSASPNVNELEHLPDEFVAAGIDLNISYPLPIAIAKIGKSINGNLIAKDYGRGNVISLNHLIEDTLLCTKIRSLKSLCQKTNFAIRELKTCNKTNTRISDKTFQQLCKTRLNIKLIRNPESVEDFNKVARFYIQTQIKKIKKLLNKIKYKCRATGYNNISEMIQLLDCMDKYNSLISSFDRIHLKPNQILPAKSRNDNSRANFRLLILRKLAAILVRECQKHHVNVVFAEDLQNNQDSDKSSFDNTLSRLFSPRLMLDTIQLALEKVGIGFVSNVDLRGTSKTDSMTGKIGYRDKFSKRDLYVLRDGKYVRIDSDLNAALNVLIRGLNHSICPYKFFVAKEDDKKREKIGKRLTQFLKDLFNQNSVHFYKQEDGSVIGSAKKLKNLKILENCYLYYREGKFLTFEQHRNEETFLSNKIKDLLVEDGNLPKTDVIQNGIKTYLNFQHLEMHESP

SEQ ID NO: 9 - protein, 906 aa, synthetic construct
MDQKQRKFQRCGVLKLEKISGKTESYYNDFQEDYRKFFNLIFSWLEKGYRYFDEDEKIHYVKPKKSALAKTQNYDKETCRLIDDFMSVLIKGGTDASSCYSLFYEKYNPKDSKKYTEFVKLSLENLHNQELQDETIEKLDPDSSISKDEWINVHIPNLKDPENRKSYWENTLGKLLVNQGRSLGKNIRERLQISCKHPSDVTYCNRLIKAIGEQIRSFYEKANLHEQERDELFAQIKSFENDDLYQKVCEFGIVLEYEGSGLSKYVLNHGVKQVLNPVNDSTIKFQVDILSQDRFRSIVETNEKDLLAAYKKYKLRSKLANKLMTCKYVAKSSLKNDFKISIGQSSLGSFRFNQENGKLVVSSDIGDFNCIPSHYFSQLDCKVIKNSKKQIVGYEISFCHKQKRKPSTKSNLPDFGNKITGVVKELGLQRKNGEFFLSFPYAIHHDHTNFKLATYFNSASPNVNELEHLPDEFVAAGIDLNISYPLPIAVAKIGKSINGALIAKDYGRGNVISLNHLIEDTSLCTKIRNLKSLCQKTNFAIRELKTCNKTNTRISDKTFQQLCKTRLNIKLIRNPESVEDFNKVARLYIQTQIKKIKKLLNKIKYKCRATGYNNISEMIQLLDCMDKYNSLISTFDRIHLKPNQILPAKSRNDNSRANFRLLILRKLAAILVRECQKHHVNVVFAEDLQNNQDSDKSSFDNTLSRLFSPRLMLDTIQLALEKVGIGFVSNVDLRGTSKTDSMTGKIGYRDKFSKRDLYVLRDGKYARIDSDLNAALNVLIRGLNHSICPYKFFVAKEDDKKIEKMGKRLTQFLKDLFNQNSVHFYKKEDGSVIGSAKKLKNLKILENCYLYYREGKFLTFEEHRNEENFLSNKIKDLLVEDGNLLKTDVIQNGVKTYLNFQHLGDA

SEQ ID NO: 10 - protein, 1234 aa, synthetic construct
MAKSDKATRPYNSVLRLIERKERDVERTLYYIECVELALFRVIGASMAFCNASIAEDLVDEVKDSSDENEDGADEGEERGQEKKARKLTKAELIEMLCAFSSFRAVPEAWDATLPEPRDANERIRLGEHMAKEHRLRFGDGPSEPVTAYFEGTSRTEPQKGGRARRSQSRWQDNLLAANEVVRISGGLLNLEKFKRFSECLLRNKAVIKSKGGKGATNAISQIFGNGEKADSRAQAVIEKSLSDACLQAHSRWVSTVRAAVAAKVGEVAKADHPGLHAFLAGKFGDLPKDSLTQKVRGDSSILTPSAENIACDVIDSIDYPTVGDVLAVSAKALGHADSNAMAKAYGYTGRKSSCRILMGNSPDGHVDLPKMAKDLSKAAKDHANKTDDLPHRGAVASLLMNEVTRLMRQRYRGFRFEDAKELSSKDKKAWEEAWKNFAATVNGKFERNCAFALEKLELQAEIKENVGDDIVPATAAIKSYMDTLDADLRWVPAPYHVAGLDSYRSHLEAAALSPDVKEEDRHEVAWSNFKQGFDPGSPKPSRPLVEHLTAHGVAEEHAAKACRILTAQDKLSSRRPHSLSPNLPSCTYGPSNMHGRIMAPSEKFNGEFCGHRPDVWATLVLANEDGTWSEHHIPVSNSRYKAEVHASRFNPDGSPALEERDYPRDRKHGYKSSGAFGPDALGRVRSSGRTKAAKRYERAVADLRWNVRWDNTTTFTLRKCAPGRFSRPYMATINHRIPKSELEAKVVVGDTIAGVDLGQYKPAAFVAIRCVPDDEPGHESRRRRWQVVEATKIDPQISVRGGKVLNQLTNMGIDYGLPGSGYDEVVLGCRAFLESQAHLWTPKERTKPPVEALDALCAKSPPLYEFHLGYARILRSLMYSAADMAKLGCDALSDDERLERVRQAMRPFRDHIGWWLLQERETPSGRLSPMRLRGLTNKALDASKKVIDLMNSYLSLMGWKKDEEREQGDRELLGANKKLYASLVNRRIEVVRVTESNVIRLCRGSGATHLAVEKELPKQGPGASRSANSGRQDWRSRELAKRLCGENKDGSAFLAGIRCRRVRSWMTSHMIPFLHTPDSECYSARYKRLRVDEISDKDAESISSILLSNKKGPLYDLYRASMLRFAADHGLDAEEMKRRKDGQYYRDRLPAGSEVFVPRHFGDVFLSPNRVASGETVTVGGRTLWVEDADIVAAANIALSYLDDSRPKKTGRPKKTGKPKKTGKPKKKGRKAS

SEQ ID NO: 11 - protein, 962 aa, synthetic construct
MLNKKSSIESYSNSSVRSTPIALHTNAMQGTYALNFMEDATLINNELLKILMAFNQAPYIMDGTLHDGEKEFSELCKQKGIDLNLFSDVCKRFIKWFTVADDVTNSCYVYLLSNKPCTLDKKIRVKNPNFIKGTNEKHIDVPVDFGLLRPLFFPITKIVTKDKIVDVSKYKTGELKSIIKSFATSFSSYIEKEAEYKLKKEEYNNAIKESTLPVDTIERYSEFLINIGKLKYFASFDGEQYKRFINNWTNEKDSKISLRNKLISISNEKGFDYKFKQIEQEFFIGYRIDFIQMIYSDFKDLWYNEDIIGNEEYVSFVRKSFHWRKEGVNLPSFDSYGKFVPILLGDNCIHHVISLIDSKKGIFQISFNINKQLISFRTSANYYFQNLELSLETPEKKVAPNCNMKLIFSSDSKCATRYQAFMREPKIRYSKKNNRFELDCSLSDVEEVDCESKKCCEFFDNDKPINEMKIFTFLRTSYNENEWKKKSFTYRAMGVDFGLANFFAATVREITKNKGETEVTTKFIDQFSNISNTVKIKLANNSEVTLKDYYKSANDKFVVARALMKKVIRFYNQYGTFDNIDSKNFEHYVKTSRNGEGICWTTTLDISYDSFIRDLKELPKPVDNCAHYIAYWLRIGNSDKTYFTTFKKVISDLSKVFSIIKSSTNHLDPSIANRVDSSTFYKLKAVKSYISFQQSIGNGLLSGDDTKELLNGTYVNKKDTSFKNISKDNLSNLRNYYNGLLRHIRNYIAGAIVNSARERKVGIIYIEDLESVYNRDKANIDCAFMDLWSVTGMIKALIEKARKHRIIVSSINPYMTSQIDAESGEVGYRDGRELTVQRNGETVILDADLNASDNILMQGATGSTLISKVKVVKTSETGYRTIEGGDTKIRKAFMNKVFKSDNIKFNVTGDLINMDSIEESKKKRGESESEIKPDGYITITNYGTVKMYLVKYKEKENRAVQS

SEQ ID NO: 12 - protein, 929 aa, synthetic construct
MTKSVNKVVVLKTTAVNQSTEVRFTQAFEQAFKATKLLFNEVPSWGLDEVYTKDSVTTDSEGNITFIPKDLKTARKALYEYTNKTVTYDQFEKMLKVMYLALTSASQSRGMVSAIIGASQNDEKLIPSDFDTIDEFISNWNLKTANESGLIYKIANTLKDIGFRNRVPYTFDLSPGERYSVVSNVHRMLTSWIECDKERAKTYKDEEEEIQKAYSEIDVSNITPIKQFNDYCINNNVIKHFDPRVHAYLRDCIVPALKGNIVPTEHFFLDKDGNKIAYNLSEGFFKILKDNPSLWNTATPLILEKIHILEKIMNHTHHHPNAFYPFIGDNDIHRFQYNFGDNYTKYDFETKGEDLEDIKVSIVTGKETVDTEFVKGCKVNDVFLNFSRSKEDNDTISFRIHTKDKYHSGSFNPNNYFNDLSIWKIKNGKCTNLLQFPRKGITVQATVKEPSIVKIDGYYAIRVNMTVVTKNDTTNNENLKWYLSTALPSAKSDRSAMQDTPANIERLKSITGKAFKFLGVDLGQRTPFSWAVGESTINGPVNTVNILTTGEYAVTNNDEYWNLLNDFKSFSKIIGITKTLSKGASADFNNVFIKKTIQNVIQYMASHNHGNDEKFETIKKFINDTNHLNTLKEQLLKCNNDLSILKKDYNFIGTIVLKYLSLRFNSLKNDRKYHLKHNDVSTKLNQEFKWLKIIESMKRALRSVSYLGTDNTRTPINLDKITDYFNGCKDNFLKVIASSIVEVAIKNNCNVIVMEGLNKNGTRTSLNKRNENFLHSLWSPARVTGAIENAANWHGITVAEVSESQTSQVHFETQTYGYRDKTKLYYLDNGEVKDTHADINAAKNIILKFVTRHASTTQVSINSVSEKDDEGKRMKGFLTHKFGTIKTAQDYFKKDFSGVDFVYLNGNKWISKEDKIVLQNSIKEKVLNK

SEQ ID NO: 13 - protein, 968 aa, synthetic construct
MNKDNKTVNTVVKTTTAKVKNSQDKLTLFKIYIDLHNVAAKVNRDIATLSGMEYKNSEGEVVLDSPKQITYWEAMHKIEDSNKFKENLQSAYEKFTSASMIRGHVPFICRDAITQNDEYACYMPLRDCGLLPLRYTGTEYDVLNSSNGYHYATIGAIHDRQSSWIECNKTTNEDYTKLRTQITEVENRIIQKFSNEELSDFKSFLDECKRLESDPAPCFFNFNGKFVSFYNNNLREALVNGNPISEGKWTTKSGKEVSYSCDKRVVDILYKYKSLWNSAKSILNDANISGMSSEKNTSPAWEDSDTIPTNTITELYSLLERKKEYASFKDINLIDSPIKLKLGNNYVGYAIAHDPDTYTLTFEVGKPKSLTNPDDKKKLKLSCSYKRVGHGTKCYLNDLVVEEQMTVITDKNKVAKHNGNYVFKYKINGKRERTSILREPSIRLVIKNKKMDINNPKLSDFDLYIDLCFNTEVQANHGISEKELFNIRKELSTSFPEIKDLGKQKNIVVEKESVINTVNKPIRVMGIDLGIKNPYAYSIIEFDKSGNHKQITSGLIKFDKNAEISKSYRDLNGVCFSLKKILSATKYYVTEGNKNLLDPRIKGMFNYVNEYFTKNFPVDSSNTISHEEYVKWIDEHMQRVVDPNGNVELSKFKSKTYNWKFREWTYKLRKIIIKLNKQRSTYSEYCSHFDWIYALESYRKLMNSFNKVGTESKFNKNRKVVNFKKIYDQVNNLKLDYIKKLASSIAETAHANGVCIVVTEKLDSMRGNVMNDKDKNSMFNMWPVGQIKDSIDKAISVYGILNADAEERNTSQVRCETGEWGYRGEREEIDILYFSDKDYVNADVNAAKNICLRYMNQHTDFHALSFYKQSDKYYVPVASIDERKRERGFLSKQFGSSKLVFELNEENRLVKSKKSIKDIKKKNELKNSKGQKETWYSLDNTFNVWISKDERKAKIETIENIVKKSKIA

SEQ ID NO: 14 - protein, 955 aa, synthetic construct
MTSTINKVICLKAKPDSNIQKNFEKNFLQTYKATQQLLNEIVCFGHDSVFSKDSVQTNPDGSTEFIAKDLTAERKRLYDCTDKSVTFEQFSDMTKGLYLGLVNAKQSRSMVSAIIGFPQSEEVLQKSDYKIVAALAEKWDDQVAKDNEIITKISNTLKSIGFRDREPYNILLAPGERYTVVANVHRMLTSWIECDTARSSTYDQEKTIINDAINSIDMKYRIHINDFFTECISNNWIKHFDPRIHAYLSDCVIPALKANKEITEHFICNRDSEHIPFSLHTGFSEYLKKNPILWQDDEPIILKNIHILEKIMSNKSHHPHAFYPFMSENDIHRFQYLLGDNYTKYGFEAIGKSVNDTSVDITSYGEVTTHQFINGVHADNLFMTFKRSKDDAEVMRLRIHTQDKRWNIQPHNGDFSLNPNSYFDDLTVWGISDKKCTNLLEFSRKGNKVRATVKEPSIVYNDGHYEVRMNMVVITDNDVEETEALKWYLSTALPASSTARSVVKDTPKNADRLKMIKGKTYKFLGVDLGQRTPYSYAVGESKITGMVNDLKILKTGEFASIYNEEYSNMLFEMKGYSKIIGITRGIAKGTSESSFADKGGAIYNVINKAKEYFRSHISKMNDDKKNTYQSFIDDKTPYDTLVSIVKSHNNDLVAVKKDYNFIGSIILKYLRLRFGAMKNDRKYHLSRESVSTKLNQEFKWLKIIEGMKRILRSASYLGTDNTRVPIELNTMTEYFNGVKDNFLKTIASSMVDIAVQNGCKIIVLENLDNQNVVLNKRNENFLHSLWSPKRVQAAIENAANWHGILIATVSESQTSQVHFESGVFGYRHGTSLYYYDNKNKLQTTHADMNAAKNIILKFVTRHASTRQANLGIFSEKDDAEKGKQRKGFLSYTFGTVKKAKEFFDKKFQGVDFAYLHGDTWISKEDKKKIQEDIKVIVDESLAKEKLMKKNSMNKS

SEQ ID NO: 15 - protein, 619 aa, synthetic construct
MAENLVIRNLNQVFTGEVLYPTLTRYNRLEARPRTDNFGRALRAEVRDALWMLCKQWQMGEFLGDDAGTPVYAKIHVEGQCITKYQPVGDPVQKFDHNTPLEATVERRPIPFAIGTQDIALDLRLQMGRRWLKMIPATAAQAFKDFYKIEQPDPTTKADAAVCAHPEVWQQFKAVAGRAMDGAGLYFHLKTPGALASDGVAGLTAGDKTAADLAGPLFVAWFEKLYFQAKPEEGDAWQPERLEYQFDCAVPDGKGGEKVLNAEEYYHERLDWYNFDWDKSKNKLDEPAEAAPEAPVESKYTTQSFIPAPARFDGMPDTRWWAFEDGKTNFGDIKPGTTDLAKLLLVEFGLVYANDWFVLPYTVPAGSVLNIEGLAVTNTFGERYWIEAAGRGSDESWQRWNMFSLNIKGQKDEPADLTLLVLPTVPKIQESQPLEEIALIRDEMANMVWGIETAVPMPHGRTRAGNIAAAEFHDFLQSFVPPLDPNDETEFKAPFRYDIMTTVPENWIPFVPEHVEGSNRQIQLRRAAMPRFLVGEKPPTFERVRPRTVLLREGLDQGNPYRLHEEEVPRAGIHVMQTFQRTRWTNGKVFTWVGVKKRTGRGEGHSGLAFDRIIPSKKG

SEQ ID NO: 16 - protein, 853 aa, synthetic construct
MFGNPGTHCNVVAPTLWGKNGAGQVEKERKAKSAESYALKMTVRTEVLPSLPPIRGSVTTNLWEYTWAPEGQIAKNTTVSKYWYSLNSSVLSRLGSLNTWGELMQKSFTEKENTLVKFNETSLSKFSPEETNSLLEFYSFAEDNFGRIDRHFTKFVQTSVEKTGTPQQGSIGKNEYSISPVIHAELMRRPELWKSNGILFVDGIGDYVELCMKLRLPTDNPPGRGLLKREPNYKSPNYNTSPVGIEFSTDGNKVPILSISCDNTHCVMVVSTVLPSGEPIDLRFSYGTRIRKIHRNGKSIKPEHQHSRNRKLINDLVITSLVKGKTNTDETNVNTPGTITFKNQRGELQSGTWTNLNIRPSGGGHVELKLAYKTPGKVLGEEYNNARRAYPSTIKLENQVSIVNGGLFTPPVGTRFVGVDWGINPLATCSVMEVVTQATATSFVTLKTICTKKWETLPINAQIKRSYLDLLRDMRLLRTLVYRTKVYAKNVATDTPAKNNAKLEEINDLLGQLRISVKTPEYLAATETYQKEKATEIKRRYGMMVNERRKVTHDVCLIKTWYEVNKKYISTRNSVYKSGRINEKIGFANYKDTFKAIRIRMQNMLDIFNAELASEILRFSDSNNAKFIVTEELTNSRSADNSKYKNEQEARLALATFKRYLTGSEDPDNFINLKYGIGILEVDENNTSRTIFDTKELGYRNFMEDKTKLYDSNGKAYDADIEASNNIVQRWVDQHSDLCTIWGKHVGEYVVLSPTINKNSATDGIEKTNGKRVEGAITKQFGGIKDVLFKVVKTPAGIKLKQIKDPQNVNEVVKLARASKQKQERFYRIRPNEWVNEPEYKNHTNKIAEKIKT

SEQ ID NO: 17 - protein, 534 aa, synthetic construct
MDRSAKETLSAGHKMVKDANLQNVSSTLGCVLSNSSSDLIKTLATSTLTHPKMLMGRQQTILYLRSRRPDLEQTWNTRFARLAEIEGELGTFFTRDGKEKDSLEDDAVGQLSFQYECLKPLNHIPWFLFAVSLFKIWLVPAMSILLPVFMWILPYFLLRFVYALPITQEQYMHILQTMLSGNLAIPTLRNLAPVEAEPLNLKTIFQYSMFAFTFAQSMIQPIQNAMHLYKTDAICVKLGQQILEVRKFLQEFRADLGPVNGIHAKLSFSLEHFSDQDIRTAFISIQETPENIHMVFRDLAHLETLWRISQSQLLNPVMFVKDRFSLVGCSDISLNVKNAVESSIELGEKSHSILTGPNGGGKSSFLRAVLQSVLIGHAFGFAPAKEAFMPRFIWIASGLQLRDTPGKYSMFETEVKFAADSIRAANIDGPGLVLFDELFHSTNPPDSQRSAIQFLHRLWKKTQTFSIVSTHLFPLISAAPSNVQAICCHATQLEDGSIDFSYGVQPGVCEVSSVHKVWETFGLARYRQVPTVVL

SEQ ID NO: 18 - protein, 891 aa, synthetic construct
MAVQNDSWDIQRCQKLKLGKKELSPINAKFYDDIQEDYRKLFPLILSFTLTPYTFEDENGVEHVVSSEQVLKTLENSVGKSLIDDVLIIGSTVAEMPQASASSFYGLFYNNYSCNDKAKWTQAKSDFLDKLLTYTDEQLEAKLEGDSCLRQMPLVEWKKVKEKLLEGNDKKEVWESVSGKLANKVNSSYSRVRKELEIQVRQPDNREYCSTLSEMLRLQVKSCYQKNLDHQKVTQELLTKVNNCSQTNPKIFDLIANFSDRLYSIGTGLSKNVLLRSIDCVNKGTLASNPTYKIAIAELLKPEFSEILTLKKEELIRAYNGVKIRDQLKRRKVYPRLPSFKNDYKVMFGLSSLAKFKIRVEDKKIKIAFSNGEEELFMNSHYFHDLEVVFDESNKTAKQFIIKFRHKLKSNKKFAVSDLITGYVKQIGLQKKNGSFYVTLMFTMKHDEKILKLERFFKTASPDMSKYTDLPDKIRVAGFDLNISNPVVGCIAEIDKNGKGPLNSIDFGKGNLVAGPDIVCQDTLMSNRVKRCKQLIFKVKDAIKDCKFSNSNNTKMNDATISFLKRLASPSQSPRCMIQTWIKNLKKRLKKLHSIIRASGYVNISEGLRMLEAQDAMKSLISSYERFHLKSGEMLAAKKNITANNRRQNFRQFISRKIASKIVQYSKGCDVIFIEDLSLDFDSDNKNNSLIRLFSADGLIKCITDAAYKAGIGVVLVDPMGTSKTDPVTAKVGYRNLKNKNYLYVERDGVLGWVDADKIASLNVLIRGLGHSIVPYKFYVKGKKKDVIGVDLVEKEVGKRLQRYFTMQHGSIKQPIFKIDNDKVTLLKKANKGDNLIENAFLYAHGDDFCTADNHRNQGKEIMHRVDSGEPVVEFDLTPCSESGYKSFQAK

SEQ ID NO: 19 - protein, 1068 aa, synthetic construct
IVKPKSIKSYSSMLDVDHRKNEILSRTFDYLNNGSSVFLWTFLSIFGGITKEIATQILSQKTEDELDDSNPELLLAIYWFRLVPVSRKSNNVLPPLLPKLFKKYLGEEPTTEVLEYFSSNFDQEKYVWQDMKAEFNNLCSQIGVSNANFVLDVGLMANEGYIGLKCGKTWGTISGLFGTGEKADRKPKVDILNSVIAAVEKNPPATRAEFASLILQCSGCTNIEQLKLKYGNIGRASFVIVRAEEINSSASIDDKYLKQIKRKLAADLKKQSNDLSWLCNTQLKNYLISKIGDYYQPSWSEMSNNALPIIQGKTTKNYNFVLEQVRCKSELDPSMQIKWELVNAYFASKFFTADNVFSICKFHIGAGEELKKLWNSWNDLSDDELEETVSAFCHSINENGRMPIYSLLMYFNSISGKITLKDVLEGITYGETKSKIERQKLNPIVEGKASFNWGNVSKISGCIISPKEKEKHIVGSKHNHDSSIWIEITVLNKDNKWVKHHFRMFNTRFYEEVYHPGNAESVPNKSVPIRSRRFGFNNQVVLSEDQINTIRNASKSMRKAMKRQVRIVAARQNNQLPEFVWNDDFNINISNDERGYRTTLSYKIEKERVETADVFVGFDQNQTARHTYSVLQLVDPKDAEAISFCGLGIKLLDVGYISSSQLVNDKSFDQLSYDGISWDRFQSWRDQREAFVTKWKNCVSKNRKAQDVPIDMLEILNRSSKYMPCLYDYNARYCGHIKKIMKGKSEKDLIEIRGEIMAFIKDGQFSVLRLSSLNHNSFSMLRNAKGIISAYFNNLIGKHCTDEQKCDADEELFMLRIELEEKRQNKAISKKNLISNRLVTIALEVRKIIGSNVVIVGENISNTTSKSNKSKQNARAMDWLSRGVADKTKQMTEMHEGIRFRDINPAYTSHQNPFIHRNPDKSVVSMRARFKSVSPKEMTEVDFKYLVKLCKSDEITYYTEGARHFTSHYGITKSDMTQITFSAFKILMTNILEKRNETNLIFPRSGGRLYLATHKIGECLPYCYDDEDGWFCDSDCVAAVNIALVGIEFERLSAAKKVVITRNAKVVN

SEQ ID NO: 20 - protein, 760 aa, synthetic construct
MKTLIRKTYVMLVVDNDQKKYLNGLMSSIYKRAASIMTHLLSWKKVGPNGYQHSLGGEILPLETASDEELDVLYQHIIDNDNSARIIRGPFALPPGKCKTGMKSEKDLEQKLRKLLDEGKLPLNLGEWEGTPGNDFVAFKIAVSSLKSWDDRNKVTEANYAKALEELNKNTPDEAGIKALNEWLDSNKLFLTKKVASKFKKFGWDTRIANYPWEILRTVNSDASYWAKMFTWQVAKQRVFGLRPTSLCTLPELAVSEREIPYGVNYENFSLELAGDRLKFVLGKREFQALRTLYFKDLKVIPAKNSYVFKYRRGNNSTLDEQVEAVLKEITLYRKNGNYYVGLSLNLQVDGDNKNCRTVKDYYFFKRASLPNGARIMAIDLGITNPASYVHVSTKKKGHEVIGSGIIGVDKEFNFLHPKYVAKLKKFKASLSEAFAAITELHPIKKVLHSQEEWSKLRYPISQMIEKLSKEMRQLRRGDLNVRNHGTSHEQMQFILVYKNFVDLLKKWTYFGSKPAAKKERRKGFEKHIRRLENLKKDFRKKLACEIVREARRKGSDLIVIEDLEHFTPDSTKDSNLNELLMLWGSGQIGKWIEHFADQYNIGVLKVDPRMTSQIDPLTGKIGYRSKYDKRKFFVKRGNKIEVIHADLAAAENIAKRVTNRMLPFVKAEKTQDGYVAWCSDDDNSRRRHVLDLTFGSHKILFRDGQPEVLEEKPSVGEEVYLYRMDDGWWPGEVKYAYLQQLAKQCEGGSRQTANGQNVA

SEQ ID NO: 21 - protein, 880 aa, synthetic construct
MTATVSTVKTAIVKIKSLPQEIKEYYDDIQADYKRYVTLFFSLSAIPYCDFEGNVFDKNLEEKRNQILQTLFCGTDLRVSMQRAIQFVDNVATKGQTENSSSYNVFYKDFKSAGAKINKHVKQFFERCLTENFDDCYSELENNICLKEKKSNYDKQFEAMFLSVDPIFWRKASQQLKGLNKKQAEKSIKELWREIQPNFTLDDRLLGQYFREDFGITCKRPNNVNYCKQLFEMVRKTLMSVKGKYTLHVNETKEIVDLKNNLLEEITKSVPDLMSQLTSMRIFLKSNYVSIGKYFFDSYSKAIEGKDAKHNAQFFKKLVDDGSYKEIFEFCKNSNNKEKFISLESLISRLEIRKQYPAFNFDMNNYGVPFGESYIPFEISIKDGKLIASFKGFPEFEFYQSDYLGNLSVSKSNRIHQIQFQHKKKIKNQESVPYGSIIKAELKELNLLCKNGSFNLYLNYSIHHPKANKDLEFFLKSSKIKSVDGFDNHIKIAAIDLNISNPITACKAEIHKGDFSHPLHCLGYGSGNWISKPEKLVFDGQYNNTLIKITNESKKLVWAIRNYKKLKNNNIPMPKEDMQFIGATLEDSQSYIRFRINTKLKSINTDMKSARENLTKSGMKNISECIRLIETEDAFASLISSYERIHLKPNESLPQTKKFDTKRANFRKFVTRRLAYKISEYASDCNIVFVENLEFDKDNYLMKLFSCKTLLSYIEEALNKKGICMVQVEKMGTSKIDPVTGKLGFRSKKDKSRLYVRRDDEICYIDSDLSACVNVMLVGLSHSICKYKIVENKEGKRSNEFMSMIGQRLKGVNYCYSDKIISEQDHNKEYDEWKRWYNETGKAQEELGMFSRNIVEQDPIIDGKNCVAFSMLNKMISENL

SEQ ID NO: 22 - protein, 1008 aa, synthetic construct
MASKHVVRPFNSVCTAKGDRLRYVTDTMDYLNGVENYLHQFMGACLSYVDETIAKELFDAEEALIAPCLSRFRLVPKELPCNIKGGILDVFAKEFGRSPTDIEKAYLTSGFDGEKYSWQNTRELAVRVSGEMGLSLEQFGDLAKTCLLNDMVLNCDAGAGSNNAVSMLFGDGPKSDYSMKAVIASKAADALEAFKPKTLEACRQVVMDVCGYSNPEDLVVAYGKTGSPSAMARFISDKNTGPVDEKVLLSKVKKFRTDAKKQGRKKLIPHLASVRNWLLVATGADVEFYARAWSAAWANSASEINAKFTHNCTFIADKIKALAELDAIEKSTEGLGAAISVLADYMKTVAEDCRYVLAPYHLGDIQTVRNFMAGCTGNFEEVFNGAWENYLEGIDFNQKPPVRELVKFIIEKGGKISSAALGSACKWLSQKDRIDNVYPHPFVQGKQGYTFGPSNIEGAINDPMMQIKSGGIAGERPMMWVTTKLLDNWKWINHHLPFANSRYYEEVYCSKEGLEFKPEARDGKHSFVLGKTIDAFATGRIKTSVGRQKAAKAIERIKANLTHNVIFDPKTTFCLRRKESRFVIAINHRHLLTPMPKEMGIGDRSMGVDQNEGAPTCYAIREKVSEGGILHSDGSRSKVIRMGKVSSIQSGKDVFTYSGVHVEDKANGFDVLWNECREFLAQHGTPEDVAYYQRSREWCKTLYPWHGLYFRMLGKLIRKTKAETLPVFREHLNHVLLKSPLSPVRLHSLSLKSLESTKKVISCISSYFSVCNMKTVEEKEKGDKYLYGVWNKLYASLVERRKERVKLSAGLIIRMCREHGVTFLRVEGDLPTVASGKSRQNNSGKQDWCARELAKRVAEMAVVVGIRCVPVFPQWTSHQDPFVHSKKNKAMRARYTRIEASKFSDRDALALRNIINSKSTGTAEYYRLAVKKFAEKHGLNLLEMKKRKDGLWYRERLSGEVFVPMRGGRVYLSTHRLCSDETYVDGNGEVLYINDADEVAALNVDLVS

SEQ ID NO: 23 - protein, 1080 aa, synthetic construct
MNNKNVKSYNCQILTNDRKKGFLDETFKALNFGSKVCLDLGMALLGGIDMNLAIEMAKDKKEDVQEAEEKNTKASKKTNKTEEKKAVISAELILAACLFRIVPKSNNEVVVAAALPSLFERYSGTQINEQVKEYFSSNFNSEKYMWKDMRCEFQKLASELNVSEKDLFSDVATMVEAKFIGLKFGEIWGIVSNLFGTGDKVPKDPKINLVSDCIARIRESNPETEDELSKIFLECSNCEDAQSMYLKYFISGRKPSEYFYANKIGSSAKIDQKKVISKLNKNLKKYKIVLDWKCNNQIKSYLANKIFAFNQKAWSEIFNASWPIIQSKTTRNLNFVLEQLQDKAQIDYSHEKFYNKVNQFFESSYFKTDNKFIIKSKHVGGEDLYNLWQDWDSWEENKIEKNLEKFSESIEDNSSKPDLMLLKYIHSIRKEISCDQVLNGIRFGQQKFKIENRFLNPIVDNSYSYNWGDKSKLNGCIISPDKKSKFNLKNNRPDYDYGIWMELEVLNNGNWEKHHFLVSNTRFMEEVYCFPKSGAKPIVCLPNGFRTKRNGFDNNVVLSDQQIQNIRNAPKHRRRAIKRQMRLEALREQNKLPLFNWNNDYNINISKSNNGYRAIISKKFEIEICKDVKVVLGVDQNQSANHTYAAFLLCDKNEEGAIAYCGQFVRPIESGFVVSKQAVGKNENKREFDQLSYNGIKWGEFNDLHEHRKNFLEQWGNVFKVNKFGVKSNVSLKDSLIALEKNNPVLYYYNMKYLNFLKNILYKKSKIDLFKIREEIFETIRDGKFSVMKLSSLSGLSFSMIRSAKSLISSYFGNLLEGTTTDDQKYESDPEMFELRQKLEKKRKDKQKSKKELTANKIVSKAIELQKKYGTVLIVLEDIGNMTSNSNKNSVNSASMDWLARGVANKVKQLSKMHEGILYYSINPFMTSHQMPLVHNNPDRAFKARFGACEPKYLFEKDFKAIKKFSKECKDTRQTTVYYRQAMKDFMEHYDISEEDMSKIDFLSFKSMMSYKLRQREEVEMLYPKMGGRVYLSTHQLDDSEQMLFNGVKYWKSNADIIAAFNIALAKIGKNETSSDAKTP

SEQ ID NO: 24 - protein, 1082 aa, synthetic construct
MNNKNVKSYNCQILTNDRKKGFLDETFKALNIGSKVCLDLGMALLGGIDMNLAIEMAKDKKEDVQEAEEKKTKASKKTNKTEEKKAVISAELILAACLFRIVPKSNNEVVVAAAALPSLFERYSGTQINEQVKEYFSSNFNSEKYMWKDMRCEFQKLASELNVSEKDLFSDVATMVEAKFIGLKFGEIWGIVSNLFGTGDKVPKDPKINLVSDCIARIRESNPETEDELSKIFLECSNCEDAQSMYLKYFISGRKPSEYFYANKIGSSAKIDQKKVISKLNKNLKKYKIALDWKCNNQIKSYLANKIFAFNQKAWSEIFNASWPIIQSKTTRNLNFVLEQLQDKALIDYSHEKFYNKVNQFFESSYFKTDNKFIIKSKHVGGEDLYNLWQDWDSWEENKIEKNLEKFSESIEDNSSKPDLMLLKYIHSIRKEISCDQVLNGVRFGQQKFKIENRFLNPIVDNSYSYNWGDKSKLNGCIISPDKKSKFNLKNNRPDYDYGIWMEIEVLNNGNWEKHHFLVSNTRFMEEVYCFPKSGAKPIVCLPNGFRTKRNGFDNNVVLSDQQIQNIRNAPKHRRRAIKRQMRLEALREQNKLPLFNWKNDYNINISKNNNGYRAIISKKFEIEICKDVKVVLGVDQNQSANHTYAAFLLCDKNEEGAIAYCGQFVRPIESGFVVSKQAVGKNENKREFDQLSYNGIKWGEFNDLHEHRKNFLEQWGSVVKVNKFGVKSNVSLKDSLIALEKNNPVLYYYNMKYLNFLKNILYKKSKIDLCKIREEIFETIRDGKFSVMKLSSLSGLSFSMIRSAKSLISSYFGNLLEGTTTDDQKYESDPEMFELRQKLEKKRKDKQKSKKELTANKIVSKAIELQKKYGTVLIVLEDIGNMTSNSNKKSVNSASMDWLARGVANKVKQLSKMHEGILYYSINPFMTSHQVPLVHNNPDRAFKARFGACEPKYLFEKDFKAIKKFSKDCKDTRQTTVYYRQAMKDFMEHYDISEEDMSKIDFLSFKSMMSYKLRQREEVEAVVSICPHINWMTLNRCCLMESNIGSLMLILLLLSILLWSKLEKTRPSVMQKHLDPLDWRK

SEQ ID NO: 25 - protein, 939 aa, synthetic construct
VINDLYTHCQRQTPDLDISKSEFRAMLKFLYLQILFASNGGREFATSIFGGCSLDQGATKAEIQGIVQFMVDYESSKGDVVDKAARNKLNTSLLNELMINKCLEHTIQPGETAVDIRNKYKSSTGAPPSTVGFFKKRVECEGVKGRITDDTELPSGQILKIKNNPVEFTKRVCRTLADMGFFNRYPFDVDRLNGYGILWAVKAQVDSWDDRAQNAKQNYQEHNQRVTELVQAMTAKQRDVFRSFIGFCATTNIIKKIDVRLKLHLEHCVIPAFKKGKMPDKYFYLGKNEEQKAYSLHSDFYAELMKQTTLWEGDEPFILSHLDAVAEMVVLNRIRDYACCPFVGSNDYHRFKMILGSNYLSYRLDAEGQVDEEGNTILSHNDRLRMVVKNGKAEFEFNIHTQDYSTPKNGDRPATGLNPSSFFKDLTIRKVKNCEYHLSFKKRGKTVQAILKQPEIVRVKQKGGNFDFCVRLSMNVIIEVDPNIFKLVSGKQRAPYSSFFQSALPYQESPTSNVQDASSKYWPDIQGKHVRALGVDLGMNRPLAYSVVESCLQSPVLKQEDLFVLDRGHCLASEQNPYHNLYYELKTLSKFIGKLKGCSKGFAADLDTEELRLLVTSAQKLIGQLKPTSEQRKRIFKAFSKASPSNLIVEAKKQAEQGDLKNTKKDPASLISLLQKYVDKRFKAIRNTRKYTTTGEAKVNDTFTWLRVIEQMKRIKRSLSYLGEDLQKNPDLKVELSSLSAYNLRVKDDFLKQIAAKILKVALENECNIIFVEDLEKELRPDKKENELFSFWSPKAILGAIQNAAQWHGIPVVEVSPIGTSKMHCETGKIGYRYRDKLYYEENDDLVWVDADINAAQNIAVRGLTRHGNLTQINLSSTPQKRINGFLYKIGNGEGVKQAFANLKQKFPDERYIHYDSGHWLTTKELKEKQDRIKSRVEK

SEQ ID NO: 26 - protein, 965 aa, synthetic construct
MKKWQRSYDFSLDISEEDALHLLDCVKKYNELSKTYMDHMFKLKEDHKDDLDVCKVIDRLQNGGVNERRALATCIFGGRKKSEDVFLRVKSYKKALALINSGEAKTYEDLSKSLGKKSGLRLKTNSLFKEPKKEGQRKDRTGLLKEDQAKKIKNMLDADLGIVSALNLCKRGLLPIPEFVANVEKINKDVLYGIIAQAGTRFQSFLKSDDSTQQNYLNLKEILKSYRLEYNLDEFKEQEASYQQWLSRMKSLDSFALTHRFLQGWAKRWRKQFLAGKDLSWTLGEEATKICKEYQHLFVDNDFIYLFGKEDLLKLKVEERKQNAQFTLPDVINSPIYPQLGNNSQGFGLEQVDNDIYLIIQSCFVDRPNIRAKIVPHKKTSVWSLEQEANPVDANPVDAKPSKKKNPQIDKDKIPYKLILRRAADRYEKQIEISECRLQHRFCSGKANFHVVFSLKGEANDTLDKVSTLFLTATQKPVSEWSKNNLPKQMRVAFVDIGLNPPLSMSIYDYNQEDNSGENPVYAGADQQIPFGSANLVREDQIGNVYNQNLKRRIQELNDKIFFASSCVSFYKNISSLEGATVELVGGRQVMCRRFDEEKIKDLYSVPVKSLRELGLDHFFGLPEDLDQQNVESAIFYIENHIHHNNLTRESFLSFRCKVWDYIHEKILPEFSVIQNGRHFQFNKQFCSEAYSWMFLIHSMIRLKKSLSYSHSEPLKKGEPATFVFKNLQNYFNNFSKNVLKTVASKLRDYCTTHNVSLCVVEDLEKFRTSSLNSKDKNRLLSIWSHRNVVQRFEEVLTEVGITIISNDARHSSQLDPVTMDWAYRDEQDKSKLWVKRDGEIDYINADISSTQVQAKRFFSRYADIVYMKTLLKKDDNGALRKLVVSDTSTRIQSYLLRIIHSKYAILEQDKLVPINQEEYNQIAGLKTSGVEEIYRHGESWVNLITHKALQKEIGASANVQSKSP

SEQ ID NO: 27 - protein, 909 aa, synthetic construct
MDQEQRKFQRCGVLKLEKISEKSESYYNDFQEDYRKFFNLIFSWMEKGYRYFDEDEKIHYVKPKKTALAKTQNYDKETCRLIDDFMSVLIKGGTDASSCYCLFYEKYNPKDSKKYTEFVKLSLENLHNQELQDETIEKLDPDSSISKDEWINVHIPNLKDPENRKSYWENTLGKLLVNQGRSLGKNIRERLQISCKRPNDVTYCNRLIKAIGEQIRSFYEKANLHEQERDELFAQIKSFENDDLYQKVCEFGIVLEYEGSGLSKYVLNHGVKQALKPVNDSTIKFQVDILSQDRFRSIVEANEKDLLAAYKKYKLRSKLANKLMTCKYVAKSSLKNDFKISIGQSSLGSFRFNQENGKLVVSSDIGDFNCIPSHYFSHLDCKVIKNPEKKIVGYEISFCHKQKRKPSTKSNLPDFGNKITGVVKELGLQRKNGGFFLSFPYAIHHDYTNFKLATYFNSASPNVNELENLPDEFVAAGIDLNISYPLPIAVAKIGKSINGALIAKDYGRGNVVSLNHLIEDTSLCTKIRNLKSLCQKTNFAIRELKTCNKTNTRISDKTFQQLCKTRLNIKLIRSPESVEDFNKVARLYIQTQIKKIKKLLRKIKYKCRATGYNNISEMIQLLDCMDKYNSLISSFDRIHLKPNQILPAKSRNDNSRANFRLLILRKLAAILVRECQKHHVNVVFAEDLQNNQDSDKSSFDNTLSRLFSPRLMLDTIQLALEKVGIGFVSNVDLRGTSKTDSMTGKIGYRDKFSKRDLYVLRDGKYVRIDSDLNAALNVLIRGLNHSICPYKFFVAKEDDKKREKMGKRLTQFLKDLFNQNSVHFYKQEDGSVIGSGKKLKNLKILENCYLYYREGKFLTFEQHRNEETFLSNKIKDLLVEDGNLPKTDVIQNGIKTYLNFQHLEMHESP

SEQ ID NO: 28 - protein, 909 aa, synthetic construct
MDQEQRKFQRCGVLKLEKISEKSESYYNDFQEDYRKFFNLIFSWMEKGYRYFDEDEKIHYVKPKKTALAKTQNYDKETCRLIDDFMSVLIKGGTDASSCYCLFYEKYNPKDSKKYTEFVKLSLENLHNQELQDETIEKLDPDSSISKDEWINVHIPNLKDPENHKNYWKNTLGKLLVDQGRSVGKKIRERLQISCKRPNDVTYCNRLMEAIGGQIRSFYEKANLHEQERDELFAQIKSFENDDLYQKVCEFGIVLEYEGSGLSKYVLNHGVKQALKPVNDSTIKFQVDILSQDRFRSIVEANEKDLLAAYKKYKLRSKLANKLMTCKYVAKSSLKNDFKISIGQSSLGSFRFNQENGKLVVSSDIGDFNCIPSHYFSHLDCKVIKNPEKKIVGYEISFCHKQKRKPSTKSNLPDFGNKITGVVKELGLQRKNGGFFLSFPYAIHHDYTNFKLATYFNSASPNVNELENLPDEFVAAGIDLNISYPLPIAVAKIGKSINGALIAKDYGRGNVVSLNHLIEDTSLCTKIRNLKSLCQKTNFAIRELKTCNKTNTRISDKTFQQLCKTRLNIKLIRSPESVEDFNKVARLYIQTQIKKIKKLLRKIKYKCRATGYNNISEMIQLLDCMDKYNSLISSFDRIHLKPNQILPAKSRNDNSRANFRLLILRKLAAILVRECQKHHVNVVFAEDLQNNQDSDKSSFDNTLSRLFSPRLMLDTIQLALEKVGIGFVSNVDLRGTSKTDSMTGKIGYRDKFSKRDLYVLRDGKYVRIDSDLNAALNVLIRGLNHSICPYKFFVAKEDDKKREKMGKRLTQFLKDLFNQNSVHFYKQEDGSVIGSGKKLKNLKILENCYLYYREGKFLTFEQHRNEETFLSNKIKDLLVEDGNLPKTDVIQNGIKTYLNFQHLEMHESP

SEQ ID NO: 29 - protein, 1061 aa, synthetic construct
MQSNEFRKAYNGYLSFNAIKEGAHKNALRKEDLVKSTFDHLEKGSLVFFDTLISLYGGLNPKTIESKLSEVQNKKPKKPKNPKKNAKKKDVEDVEKTDIKLICAIFWFRVVPKDNYEKFSIPQPILEKKFKKYFGEDCSELASVYFKSNIDIEKYHWIDCRQKYESFCKEAKFQEDFSHDLEILVSEGLLPVQKGKIADKTWATVSNMFGDGKKEDRPSKVEAYKKIIAAVESHKDQIQNADDLKRVVFDAVEVKTNAEFYKKIAGAGGGSPPRICNIIKKSVFDEKTYQNVIDTCNKNIGNKSKDLTWKEIKNFKKYIEKKIDAPFYQNSWSEMLKNALGDIQSKNSRNINFSQEQLSLKKELATLEVGNTLNKYFQSSFFTTQDEFVIAPYHIGGRELPKLFKAWDNSDDIEQCIQEYCDEIKTTLAKDPIQNILRYLHSVRNECNAESILAEAKYNKLIEKFESQSIHPTIKGNNWFTWGDSALDGKVVPPNKRRVNKFSTPDTSIWIEVKLFNSREKRWEKHHVPFFNTQFYEEVYAYNPASENQVLLRTKRFGHNFNEPLKPELIDFIKNSKTKKSAKRIARVEAQIQSGLMPNVEWKDCAICIKKEDSRFKISVIYKFKTQNKTKYEIGDVIVAYDQNQTAAHSYAVLKIVDGTSFRNYNLEVLETGKIESNVSCASNTIDQLSYAGLPFKQFRSWRKHAYSFVKSFNDKDLLDKFKKIIRRRPNLYRFNCDYARLLKKSMEGKSCQELIQKIRNEIIRFLDTKECSIRHVCSLSHDSFSAIVACKAIINAYFSNKLGKCTDEEKLADDPELFNIRKDLERRRKNKGREKINRTCNSILKIAIENNAQFVVGEADLSTGDKNNKKKQNSKNMDWLARGVAKKIATACTMHSIKFLGVGPHYTSHQDALEHQKDFDNPKSVMRARYTKLPPSKLSEYDIKKMSSFLKNNSEGTTAKYYNEAMKDFLKNYNIEFLENDIKSKKIKFWELSKRLEQYDEIIFPRRGGRFYLATHRLTTNATKIKYAEKEYWFSDADEIAAINIGLAIFPTKKSNAVDP

SEQ ID NO: 30 - protein, 830 aa, synthetic construct
MSKKEKDPNEFKAAHYKCVSACLCLTDRQVQFFVKNMFSKQAEQLYRLFLHGWMGRDDGLHQEIGQGMTATAFLDTCEELRQGLLCTDKVKTGRKNAKGNDEYHSLKVTSRALAAPIFGDSKVGSSTCNCQEPLLKLRAAGVLPLPRMPVIADEFGVVETALESLRSYVACDKSTRESYQKEAAYLQKLQQVDISSLQEIEDDPENPDKHGDAQLLRRLHEQVEHGRAETLEEALVGIVKAQEKRLTELRSSARLTLPTPQKPMAYRLGSNYVDYALKLDGPYLELTILGGSLKGVYRCAYGTKNKKNLLSNLKLETVPGATTRYTFEYAENGKRPRLAICREPRIIYRRGRIYLEIPLGFEETLPSYFWATPGKGCSFNSYFPKPVKIDFTELRVLGIDLNINPAIAYAVGYAKEFENGVAGRLEIEDTGILKGTPFSERIRALNSLMQDLKRVLKNCVAARIRGLTLPEHIKKWKDPGAFVRMAQRFYPDVEELYKEVERLPLETRYTVEAKKYISVRQWRFCGWSLGQHMRDLLNQYKELMQYRRTQAVANLTDGVEWQRLLRSRAELQTSWHTMGGQARLGGELLSRFHKQKLRAQIDNRKKMARMIIDLAIRFGCRLIAVEDLEREDRRDFAGNYLWDLWSAKSMITLLMEMAAVEGIGVVRVQPDCTSKTAYGLFVPAYRNEKDRRKVHYLTDDEQVETVDADINAACNVAYLAVTRHRYPLYFWVRRDPETGRVTFLKKDDNKDDKKDAVPARGKKKKKKSKTNAEEYAKKIKAMFGDCECWQHLQVGEKPTKIYRYKNTWITWAEREILIEEIKERLRKVAG

SEQ ID NO: 31 - protein, 1012 aa, synthetic construct
MSGNVVRSYKSVLRPNIRKRELLDATFNWFDRAYKKFFDVFVCLYGGVEHDTVHSALLKETTDPDLVCATMWFRVVPKSSCDGISAQEMIRRFGVYAGHEPSAVAMSYLTGNFDDKKNHWIDCREKFVALARDMVVKPESLSIDIKSMIEHKILPICSQDNWQAWNAISQLFGEGKKENKAEKAQIFVDVVSMLSNNSVQTWEDYKEVISKATGCRTAGEINSKFGGRPGILSVDFSKDDTGSLPKDFIERRIKDLSQKAKEKSAAYELPNRMRLRELIASVIGPYRLETWSSVAQRACGDIRSKNSNNLLYASERFNRTKEIEEILSAKGDVARAQQILGQFRSGEFNEFAVEKRHLGNLESLYNIWSKSDMDTGIEEYSSIHKDEYDRDPIVDLYRHIYPHREVISAKNFIDAAVLNKLLRLNASRHVHPTVFGKTVISFSPKSSAYGRITPPSEIVRGRPAGSHGMIWVTMELFDDGKWIEHHLPFHNSRYYEEVYCYQEGLPVKDEPRSPMFGYRVGNAIADTSKIDNRRRKASKQFLRAQQNITHNVSFDENTAFSVARNGEDFSITISSRLKASNAKSLMTIGDRIMGIDQNQTAANTYSIWEVVGDGDAGSIQHGNLSLKRIEDGHITSIIRGRGGNFDQLNYGGLSYAKFSEWRSARLGFISSLNAELASKMNWDWCCLYEWNARYASALRKIIYSHKGIDIERVFRREIEDFVEGVLRIGSLSSDALQCLTNAKSLISSYFFLNGKKEPEEQRQFDQGLFDLSAKIDKKRVNKRQQKTKRIMSSIMQIARDRGVSFIVVEGKLSTATKDNKSKANQKAIDWCARAVVENLEHSCSLVGIKLVAIDPMNTSHLDPFVYVLKTSLGKEARFASVVPAKINARHMKNFKSWSSLLAGKGKSKKTTDAIYVGAFQDFCREYGFVAEDISKMSQSEIQDKLSSHQFVLVPQRGGRVYMSTHPVSSEAKKIVYAGRERWYNNADVVAAVNITLRGCERLSASRKTASTR

SEQ ID NO: 32 - protein, 1168 aa, synthetic construct
VKDSSDDKEDGADDGHERGQEKKARKLTQAELIDMLCAFSSFRAVPEGWDATLPEPRDAEQRIRLGEHMAEEHRRTFGDGPSEPVAAYFEGTSRTETHESWRAARSQSRWQDNLLAAKQVVRVSGGLLNWEKFQRFSECLLRNKAVIKCKAPNGPCNAISQIFGKGKKADSAAQAVIENSLSDACLQAHSRWVSMVRAAVAAKVGEVAKADHPGLHAFLAGKFGDLPKNSLTQKVRGDCSILTPSAENIACDVIDSIDYPTVGDVISVSARALGHPDAKAMADAYGYSGRESSCRILMGKSPDGHVNLPVVAKKLSSDAKSHSNKTAVLPYRDAMASLLMNEVTRLMRRRYRGFRFQEANELSPNDKQAWIEAWKNFAATVNGKFERNCAFALEKLELQAEIKENVGDDIVPATAAIKSYMDTLEADRRWVPAPYHVAGLDSYRSHLEAATLSPDVKEEDRHDMAWSNLEQGFEQGSLKPSRSLVERLTAHGVAEKHAAKACRLLTAQDKLSSRRPHSLSPNLPSCTYGPSNMKGRIMAPSEKFNGEFCGHRPDVWATLVLANEDGTWSEHHVPVSNSRYKAEVHSSRFNPDGSPALEERDYPRDRKHGYKSSGAFGPDALGRVRSSGSGRTKAAKRYERAVADLRWNVRWDDSTTFTLRKCAPNRFSHPFMVTINHRIPKSKLEAKVVVGDTIAGVDLGQYKPAAFVAIRCVPDDEPGHDSRRRRWQVVEATKIDPQISVRGGKVLNQLTNMGIDYGLPGSGYDEVVLGCRAFLESQAHLWTPKERTKPPVEALDALCAKSPPLYEFHLGYARILRSLMYSAADMAKLGCDGLSDDERLERVRQAMRPFRDHIGWWLLQERETPSGRLSPMRLRGLTNKALDASKKVIDLMNSYLSLMGWKKDEEREQGDRELLVANKKLYASLVNRRLEVVKVTESNVIRLCRGSGATHLAVENELPKQGSGASRSANSGRQDWRSRELAKRLCGENRDGSAFLAGIRCRRVRSWMTSHMIPFLHTPDSECFSARYKRLRVDDISDKDAESIRSILSAEKGPLHDVYRASMLRFAADHGLDVEEMKRRKDGQYYRDRLPAGSEVFVPRHFGEVFLSPNRVASGETVTVGGRALWVEDADIVAAANIAMSYLDDSRPKKTGKPKNTGKPKKKGRKAS

SEQ ID NO: 33 - protein, 1010 aa, synthetic construct
MTEQDKFELPREGGDTRTKMLALRPSPEAESQLMSLMDKAVPIANDTLRLLLTMMGEPYSIDNQFFSREDVSLQMKKLAQEHGLLATEETFRMFRLVSGRIVNTRNSANSVYNYMYGAGDFGVPLRIQKKKAFALNADGTFVEVEEGKGTHHQLHDGQIVLSQDDDYTIPAAFGESKGEPDIREEALALRKSGIFPIGDMSHFTSSARRGLCKSIVEGELRSYVEIRKAYEEEKERWNKKVAAIRDGESKEFDWDVVREFEQLLAQLEECPDFGKFDGRSFGRLVGRLRGGKVENSKPTVYCWAQGILHYFQQFRPGHVFSFHGKKFGYGKEVLQVLFDSILWTRPVVTPGQEDYSSSLLVNQEYVSLIIDSYHFRKKAVNLSSHGVSRRKIPIRVEFEGNNCITAELSKETVRLRNAVVGEDGKPEGIDVSIVQSDYWKSARLSKKSPTVTAKDGTTKDGKKEKLFLEYSQDSKRKTWYQGFVRSGLIAYNDRKKGFYLYLCLSEHCEDGIPFDASISRMRRAFREAGSLLDLPETPERFRAMSVDYGISRPFCMSIYDVTRTASGFSMDKVFSRSSFERDNVLATVSRYRGITDRAVALKFAIYETEEYLHGEIERIDGVKTFRDGGREPILWAKKFGIDCREYERFLAPYVGTPDVFWALRRKESGWFVGAEIHRLRKDIKRIRGEYRNVRDKRAHCREFNFADASLFYKREMVSVTTDMLKVFSTIGMSTERSAKTRDGFAASLGNFYDGLTRKLHLDLSSAVINIAREYGVMLIAIEDLDSRTTIFNTVEENRTKRMLGYGGYTTRLADKSKKHNKGIVQVDPRLTSLTDPETGKLGCRDERNRKILYVERNGRIVEIDCDLAATDNIMRRALERHQDLRDHWSVEISDGVYVISGDRGKRNRAALMRWEGRDSFVLLRNADGTLSVRDEPPTEEELKACEKGGRKTEGKEKKPKFVKLFRDGDVWMVMDELREKMRATVEEYKNGGIALGPLEGQGDGDGRAAV

SEQ ID NO: 34 - protein, 1030 aa, synthetic construct
MATDTVYRPYTCKLLPDARKRGLLEDTDRMMRCGQEVFLDLYAAILGGIRPALVAVLYPEQDTQLLCAVSWFRLRPVTKNKTIISSSNMMQAFASYYGEEPNEFVATYLTSNYDADKYMWVDCRSLYSSLCSDLKVSPDSLSVDIESMMRQHDIMLYDAEAKGWAAMSHIFGEGEKANTNNQYKLCCDVIDRLEKSEIKTKEEYTAVVLEVFGAKDKKEVKKIWSPKRAASLIEDLDADTKDFNVENYKQRWIELKDEKSFSPSYPNNKALKKYIENKISDKFGMPAKYHMESWSVMYRNALTDICTKTTRNYNFSVEQIARKKELEKLDASALNILNGYFASSYFTTSDVFVIERRHIPNMKNLVDRYVALDNPTDADINNIINDVNDETKEDGCNTGIVQLQRYVLSICKCVSIEQIDSALKINKLNSDIKRQKANPLVMGNMSYTYGKSAMVGTIADPRAMHNGKVNGMTPEMWAYMSLYHEDTKEWRMHHVPFYHAKYYEEVYHYDPSHNDSVGIRTKRNKTKHTKSNIAYDEVSPNFTKKNIRTVSTMKNTHVNVDIIPSSFELRKRNGNYEITISQKIKKTEKRSGDLVMGFDQNQTRPNTYSIWRVNNDGGKHEFVCGGKITSIINLGDREIDVLSYDGADESSDYFLRFVEGRKKYINQIAHLDVFAKTPENKLKIDFDCYNELNNIKEKQLYRWQSKYLRLLLRIIKITKCNIPGIKREIMEVVETMDAKSSLSHTCIESIRRMKSLIHCWFSYLMNEKEPTNEKKESYDKDMYRLLQHIERRRNNKNKERVRKIAASIIDISIANNVNVIVGEGELNTIKKGKNKESNARAMDWCAREVAKKVEQGCDLTDITFWAVSPYNTSHQDPLEHTAKNKVMNPRMEIVALIERSEWAVKKLTNLCRAKPKNGTTGEYYNAGIDIFCQHYNVDKKKLEKIKTIKDIHGLLPGYTELLLPMRGGRYYLASHCATSSARLIEYAGSQRWLCDADEIAAANIALRYISDSQKNKEKKKNAVATIVATA

SEQ ID NO: 35 - protein, 1027 aa, synthetic construct
LVTSLFIQNKHQDTLNSVLGSTNSYKIASEVTPTKTFVNAESIIEKTVGIRNLAGVEEVPHVFTRELAADESLAIDVTEEATNGFVLLSDKVQDDANRKKSAADITNTEQSPSLRQFKNPQKEIRLDQETHNSALSDTSSIMSAIADEVNFQSKPSHDHHKEQHQEASNEPRDLTLVVTSSVLSNILVSRANHPQSTSSVDHHAELPPAEDASFIVSSLAKLKQVDPQFERHLNHHARLLQTKDADSTSSASTVAIAVDIPDGIAHEVTPPAPVAASRMHSVAATSIFNPPFRSNHPEIRKRRHGGTPAYATSNKQVTRMATSKQSFLSKDELKGALDNYVTQDCANMQDCDVGQIYGWPMNAWCVSNVTDMSWLFSNMYFFNENISSWDVSNVVSMVGMFYYAQAFNGNLSGWDVSNVVSMDYMFHYAQAFNGNLSGWDVSNVVNMYAMFNYAQAFNGDLSGWDVSNVVNMDYMFYYAQAFNGNMSGWNVSGVSYMARMFYGAKSFNQNLCLWANAFPYDSASSIFAESNCTYTSDPIRERLAPFCASTCGIGSNECFLSKAELKRAVDKYMTQDCANLPDCDVGQIYGWPMNAWCVSNVTDMSWLFYSMLYFNENISSWDVSNVVNMEYMFYYAQAFNGDLSGWNVSGVSNMAQMFYGAKSFNQDLCSWADAFPYDSASSIFAESNCTYTSDPIRERLAPFCASTCDNGSNECFLSKAELKRAVDNYMTQDCANLPDCDVGQIYGWPMNAWCVSNVTDMSWLFYSMPYFNENISSWDVSNVVSMYYMFCYAQAFNGDLSGWDVSNVVNMYYMFYYAQAFNGDLSGWNVSGVSNMAQMFYGAKSFNQDLCSWADAFPYNSASSIFAESNCTYRSDPLLFRGGSFCASMCADLPYILDVLPSDASDTGGIKIRLLGYNFVSSHATNTSTSFECQFGSAAKVNASLIFNNELNCVSPIVLLVNGALEVDLFVIIDGQTSFNSVPFQFYGLCPENQCNNGYCSFGQCEVSLHTVVATVQFSLFFHLCDE

SEQ ID NO: 36 - RNA, 37 nt, synthetic construct
  source 1..37: mol_type = other RNA
gtgccataatcgccgagtaagtatcgtcgatccgcac

SEQ ID NO: 37 - RNA, 37 nt, synthetic construct
  source 1..37: mol_type = other RNA
gtgcggatcgacgatacttactcggcgattatggcac

SEQ ID NO: 38 - RNA, 37 nt, synthetic construct
  source 1..37: mol_type = other RNA
aggtacaacagtaagaaatacttactgttattgtaac

SEQ ID NO: 39 - RNA, 37 nt, synthetic construct
  source 1..37: mol_type = other RNA
gttacaataacagtaagtatttcttactgttgtacct

SEQ ID NO: 40 - RNA, 36 nt, synthetic construct
  source 1..36: mol_type = other RNA
ggtacaacagtaagaaatacttactgttattgtaac

SEQ ID NO: 41 - RNA, 36 nt, synthetic construct
  source 1..36: mol_type = other RNA
gtgcatccagtcttcgtaagcagactcgataggcac

SEQ ID NO: 42 - RNA, 23 nt, synthetic construct
  source 1..23: mol_type = other RNA
gtgtgactatgcacacattctct

SEQ ID NO: 43 - RNA, 23 nt, synthetic construct
  source 1..23: mol_type = other RNA
agagaatgtgtgcatagtcacac

SEQ ID NO: 44 - RNA, 23 nt, synthetic construct
  source 1..23: mol_type = other RNA
agagaatgtgtgcaatgtcacac

SEQ ID NO: 45 - RNA, 23 nt, synthetic construct
  source 1..23: mol_type = other RNA
gtgtgacattgcacacattctct

SEQ ID NO: 46 - RNA, 25 nt, synthetic construct
  source 1..25: mol_type = other RNA
gtgtgacattgcacacattctctta

SEQ ID NO: 47 - RNA, 25 nt, synthetic construct
  source 1..25: mol_type = other RNA
taagagaatgtgtgcaatgtcacac

SEQ ID NO: 48 - RNA, 24 nt, synthetic construct
  source 1..24: mol_type = other RNA
agagaatgtgtgcatagtcacact

SEQ ID NO: 49 - RNA, 24 nt, synthetic construct
  source 1..24: mol_type = other RNA
agtgtgactatgcacacattctct

SEQ ID NO: 50 - RNA, 36 nt, synthetic construct
  source 1..36: mol_type = other RNA
gtgcttgcctactccgctaggggaagataaaagcac

SEQ ID NO: 51 - RNA, 36 nt, synthetic construct
  source 1..36: mol_type = other RNA
gtgcttgccgactccgctaggggaagataaaagcac

SEQ ID NO: 52 - RNA, 36 nt, synthetic construct
  source 1..36: mol_type = other RNA
gtgcttaccgactccgctaggggaagataaaagcac

SEQ ID NO: 53 - RNA, 36 nt, synthetic construct
  source 1..36: mol_type = other RNA
gtgcttttatcttcccctagcggagtcggtaagcac

SEQ ID NO: 54 - RNA, 36 nt, synthetic construct; identical to SEQ ID NO: 53
  source 1..36: mol_type = other RNA

SEQ ID NO: 55 - RNA, 36 nt, synthetic construct
  source 1..36: mol_type = other RNA
gtgcttttatcttcccctagcggagtcggcaagcac

SEQ ID NO: 56 - RNA, 36 nt, synthetic construct; identical to SEQ ID NO: 51
  source 1..36: mol_type = other RNA

SEQ ID NO: 57 - RNA, 36 nt, synthetic construct; identical to SEQ ID NO: 55
  source 1..36: mol_type = other RNA

SEQ ID NO: 58 - RNA, 36 nt, synthetic construct
  source 1..36: mol_type = other RNA
gtgcttttatcttcccctagcggagtaggcaagcac

SEQ ID NO: 59 - RNA, 36 nt, synthetic construct
  source 1..36: mol_type = other RNA
gccccatcactaggggcattcttgcgccaccctgag

SEQ ID NO: 60 - RNA, 36 nt, synthetic construct
  source 1..36: mol_type = other RNA
ctcagggtggcgcaagaatgcccctagtgatggggc

SEQ ID NO: 61 - RNA, 33 nt, synthetic construct
  source 1..33: mol_type = other RNA
tgtgccaactcgtacaagcgagtaaagtgcaac

SEQ ID NO: 62 - RNA, 33 nt, synthetic construct
  source 1..33: mol_type = other RNA
gttgcactttactcgcttgtacgagttggcaca

SEQ ID NO: 63 - RNA, 36 nt, synthetic construct
  source 1..36: mol_type = other RNA
attagtgccaacctatacaagtaggttaagtgcaac

SEQ ID NO: 64 - RNA, 36 nt, synthetic construct
  source 1..36: mol_type = other RNA
gttgcacttaacctacttgtataggttggcactaat

SEQ ID NO: 65 - RNA, 36 nt, synthetic construct
  source 1..36: mol_type = other RNA
gtgtcaatgatctgtgtttcagatccacactgttat

SEQ ID NO: 66 - RNA, 36 nt, synthetic construct; identical to SEQ ID NO: 65
  source 1..36: mol_type = other RNA

SEQ ID NO: 67 - RNA, 36 nt, synthetic construct
  source 1..36: mol_type = other RNA
ataacagtgtggatctgaaacacagatcattgacac

SEQ ID NO: 68 - RNA, 36 nt, synthetic construct; identical to SEQ ID NO: 65
  source 1..36: mol_type = other RNA

SEQ ID NO: 69 - RNA, 36 nt, synthetic construct; identical to SEQ ID NO: 67
  source 1..36: mol_type = other RNA

SEQ ID NO: 70 - RNA, 36 nt, synthetic construct
  source 1..36: mol_type = other RNA
gtggcatctcctagtagattctagagatacaaccac

SEQ ID NO: 71 - RNA, 36 nt, synthetic construct
  source 1..36: mol_type = other RNA
gtggttgtatctctagaatctactaggagatgccac

SEQ ID NO: 72 - RNA, 52 nt, synthetic construct
  source 1..52: mol_type = other RNA
gtggttgtatctctagaatctactagctagtagattctagagatacaaccac

SEQ ID NO: 73 - skipped

SEQ ID NO: 74 - RNA, 24 nt, synthetic construct
  source 1..24: mol_type = other RNA
gtggttgtatctctagaatctact

SEQ ID NO: 75 - RNA, 36 nt, synthetic construct
  source 1..36: mol_type = other RNA
ataacagtgcgattctgaaacacagaatattggcac

SEQ ID NO: 76 - RNA, 36 nt, synthetic construct
  source 1..36: mol_type = other RNA
gtgccaatattctgtgtttcagaatcgcactgttat

SEQ ID NO: 77 - RNA, 25 nt, synthetic construct
  source 1..25: mol_type = other RNA
cccaccgataaatcggtgggctgaa

SEQ ID NO: 78 - RNA, 25 nt, synthetic construct
  source 1..25: mol_type = other RNA
cccaccgataaatcggtgggttgaa

SEQ ID NO: 79 - RNA, 32 nt, synthetic construct
  source 1..32: mol_type = other RNA
agtcgtggcctgccacagcaggctgatgcgac

SEQ ID NO: 80 - RNA, 33 nt, synthetic construct
  source 1..33: mol_type = other RNA
gctgcagctgcagttagtacaaagactcccgct

SEQ ID NO: 81 - RNA, 33 nt, synthetic construct
  source 1..33: mol_type = other RNA
agcgggagtctttgtactaactgcagctgcagc

SEQ ID NO: 82 - RNA, 33 nt, synthetic construct; identical to SEQ ID NO: 80
  source 1..33: mol_type = other RNA

SEQ ID NO: 83 - RNA, 33 nt, synthetic construct; identical to SEQ ID NO: 81
  source 1..33: mol_type = other RNA

SEQ ID NO: 84 - RNA, 36 nt, synthetic construct
  source 1..36: mol_type = other RNA
gtgcgaaacggtctcgttagaggctggttcaagcac

SEQ ID NO: 85 - RNA, 36 nt, synthetic construct
  source 1..36: mol_type = other RNA
gtgcgaaacggtctcgttagaggctggttcaaacac

SEQ ID NO: 86 - RNA, 36 nt, synthetic construct
  source 1..36: mol_type = other RNA
gtgcgaaacggtttcgttagaggctggttcaagcac

SEQ ID NO: 87 - RNA, 36 nt, synthetic construct
  source 1..36: mol_type = other RNA
gtttcaatcgatgattattgtgcctgtcattggcac

SEQ ID NO: 88 - RNA, 37 nt, synthetic construct
  source 1..37: mol_type = other RNA
gtgccaatgacaggcacaataatcatcgattgaaacg

SEQ ID NO: 89 - RNA, 37 nt, synthetic construct
  source 1..37: mol_type = other RNA
cgtttcaatcgatgattattgtgcctgtcattggcac

SEQ ID NO: 90 - RNA, 38 nt, synthetic construct
  source 1..38: mol_type = other RNA
gtggataggccgccaatcattcttcagcggctaccact

SEQ ID NO: 91 - RNA, 38 nt, synthetic construct
  source 1..38: mol_type = other RNA
agtggtagccgctgaagaatgattggcggcctatccac

SEQ ID NO: 92 - RNA, 32 nt, synthetic construct
  source 1..32: mol_type = other RNA
gtgagattcaaacttgtgaaagtttgaatctg

SEQ ID NO: 93 - RNA, 36 nt, synthetic construct
  source 1..36: mol_type = other RNA
gtgagattcaaacttgtgaaagtttgaatctggcac

SEQ ID NO: 94 - RNA, 36 nt, synthetic construct
  source 1..36: mol_type = other RNA
gtgccagactcaaactttcacaagtctgaatctcac

SEQ ID NO: 95 - RNA, 36 nt, synthetic construct
  source 1..36: mol_type = other RNA
gtgccaaattcagactttcacaagtctgaatctcac

SEQ ID NO: 96 - RNA, 23 nt, synthetic construct
  source 1..23: mol_type = other RNA
gtgagattcagacttgtgaaagt

SEQ ID NO: 97 - RNA, 23 nt, synthetic construct
  source 1..23: mol_type = other RNA
actttcacaagtctgaatctcac

SEQ ID NO: 98 - RNA, 32 nt, synthetic construct
  source 1..32: mol_type = other RNA
cagactcaaactttcacaagtctgaatctcac

SEQ ID NO: 99 - RNA, 36 nt, synthetic construct; identical to SEQ ID NO: 94
  source 1..36: mol_type = other RNA

SEQ ID NO: 100 - RNA, 36 nt, synthetic construct
  source 1..36: mol_type = other RNA
gtgagattcagacttgtgaaagtttgagtctggcac

SEQ ID NO: 101 - RNA, 29 nt, synthetic construct
  source 1..29: mol_type = other RNA
gtcccactagcagggacattcttttgcct

SEQ ID NO: 102 - RNA, 29 nt, synthetic construct
  source 1..29: mol_type = other RNA
aggcaaaagaatgtccctgctagtgggac

SEQ ID NO: 103 - RNA, 29 nt, synthetic construct
  source 1..29: mol_type = other RNA
gtcccactagtagggacattcttttgcct

SEQ ID NO: 104 - RNA, 29 nt, synthetic construct
  source 1..29: mol_type = other RNA
aggcaaaagaatgtccctactagtgggac

SEQ ID NO: 105 - RNA, 29 nt, synthetic construct
  source 1..29: mol_type = other RNA
gtcccagtagtcgggacattcttttgcct

SEQ ID NO: 106 - RNA, 29 nt, synthetic construct
  source 1..29: mol_type = other RNA
aggcaaaagaatgtcccgactactgggac

SEQ ID NO: 107 - RNA, 29 nt, synthetic construct
  source 1..29: mol_type = other RNA
atcccactagtagggacattcttttgcct

SEQ ID NO: 108 - RNA, 29 nt, synthetic construct
  source 1..29: mol_type = other RNA
aggcaaaagaatgtccctactagtgggat

SEQ ID NO: 109 - RNA, 26 nt, synthetic construct
  source 1..26: mol_type = other RNA
gtcccatttgcagggacattcttttg

SEQ ID NO: 110 - RNA, 26 nt, synthetic construct
  source 1..26: mol_type = other RNA
caaaagaatgtccctgcaaatgggac

SEQ ID NO: 111 - RNA, 26 nt, synthetic construct
  source 1..26: mol_type = other RNA
gtcccactattagggacattcttttg

SEQ ID NO: 112 - RNA, 26 nt, synthetic construct
  source 1..26: mol_type = other RNA
caaaagaatgtccctaatagtgggac

SEQ ID NO: 113 - RNA, 26 nt, synthetic construct
  source 1..26: mol_type = other RNA
gtcccactagcagggacattcttttg

SEQ ID NO: 114 - RNA, 26 nt, synthetic construct
  source 1..26: mol_type = other RNA
caaaagaatgtccctgctagtgggac

SEQ ID NO: 115 - RNA, 36 nt, synthetic construct
  source 1..36: mol_type = other RNA
gtggcaatgtgtgaattttgtgcctctcattggcac

SEQ ID NO: 116 - RNA, 36 nt, synthetic construct
  source 1..36: mol_type = other RNA
gtgccaatgagaggcacaaaattcacacattgccac

SEQ ID NO: 117 - RNA, 36 nt, synthetic construct; identical to SEQ ID NO: 115
  source 1..36: mol_type = other RNA

SEQ ID NO: 118 - RNA, 36 nt, synthetic construct; identical to SEQ ID NO: 116
  source 1..36: mol_type = other RNA

SEQ ID NO: 119 - RNA, 36 nt, synthetic construct
  source 1..36: mol_type = other RNA
gtggtaatgtgtgaattttgtgcctctcattggcac

SEQ ID NO: 120 - RNA, 36 nt, synthetic construct
  source 1..36: mol_type = other RNA
gtgccaatgagaggcacaaaattcacacattaccac

SEQ ID NO: 121 - RNA, 31 nt, synthetic construct
  source 1..31: mol_type = other RNA
aatgtgtgaattttgtgcctctcattggcac

SEQ ID NO: 122 - RNA, 31 nt, synthetic construct
  source 1..31: mol_type = other RNA
gtgccaatgagaggcacaaaattcacacatt

SEQ ID NO: 123 - RNA, 36 nt, synthetic construct
  source 1..36: mol_type = other RNA
gtgtcattactctgctttacagagtcacactgtcag

SEQ ID NO: 124 - RNA, 36 nt, synthetic construct
  source 1..36: mol_type = other RNA
ctgacagtgtgactctgtaaagcagagtaatgacac

SEQ ID NO: 125 - RNA, 36 nt, synthetic construct
  source 1..36: mol_type = other RNA
gtgctacaaacgaagaagatcgtttgtgatttgcac

SEQ ID NO: 126 - RNA, 36 nt, synthetic construct; identical to SEQ ID NO: 125
  source 1..36: mol_type = other RNA

SEQ ID NO: 127 - RNA, 36 nt, synthetic construct
  source 1..36: mol_type = other RNA
gtgcaaatcacaaacgatcttcttcgtttgtagcac

SEQ ID NO: 128 - RNA, 36 nt, synthetic construct; identical to SEQ ID NO: 125
  source 1..36: mol_type = other RNA

SEQ ID NO: 129 - RNA, 36 nt, synthetic construct; identical to SEQ ID NO: 127
  source 1..36: mol_type = other RNA

SEQ ID NO: 130 - RNA, 33 nt, synthetic construct
  source 1..33: mol_type = other RNA
ctacaaacgaagaagatcgtttgtgatttgcac

SEQ ID NO: 131 - RNA, 33 nt, synthetic construct
  source 1..33: mol_type = other RNA
gtgcaaatcacaaacgatcttcttcgtttgtag

SEQ ID NO: 132 - RNA, 33 nt, synthetic construct
  source 1..33: mol_type = other RNA
gtgctacaaacgaagaagatcgtttgtgatttg

SEQ ID NO: 133 - RNA, 33 nt, synthetic construct
  source 1..33: mol_type = other RNA
caaatcacaaacgatcttcttcgtttgtagcac

SEQ ID NO: 134 - RNA, 27 nt, synthetic construct
  source 1..27: mol_type = other RNA
tcttcccctagcggagtaggcaagcac

SEQ ID NO: 135 - RNA, 27 nt, synthetic construct
  source 1..27: mol_type = other RNA
gtgcttgcctactccgctaggggaaga

SEQ ID NO: 136 - RNA, 37 nt, synthetic construct
  source 1..37: mol_type = other RNA
agtgcttttatcttcccctagcggagtaggcaagcac

SEQ ID NO: 137 - RNA, 37 nt, synthetic construct
  source 1..37: mol_type = other RNA
gtgcttgcctactccgctaggggaagataaaagcact

SEQ ID NO: 138 - RNA, 36 nt, synthetic construct
  source 1..36: mol_type = other RNA
gtcgaaactcttaagaattgtgtccttcgttgacac

SEQ ID NO: 139 - RNA, 36 nt, synthetic construct
  source 1..36: mol_type = other RNA
gtgtcaacgaaggacacaattcttaagagtttcgac

SEQ ID NO: 140 - RNA, 36 nt, synthetic construct; identical to SEQ ID NO: 138
  source 1..36: mol_type = other RNA

SEQ ID NO: 141 - RNA, 36 nt, synthetic construct; identical to SEQ ID NO: 139
  source 1..36: mol_type = other RNA

SEQ ID NO: 142 - RNA, 36 nt, synthetic construct
  source 1..36: mol_type = other RNA
gtagcgttgttccattttgctgtggaacattgacgc

SEQ ID NO: 143 - RNA, 36 nt, synthetic construct
  source 1..36: mol_type = other RNA
gcgtcaatgttccacagcaaaatggaacaacgctac

SEQ ID NO: 144 - RNA, 36 nt, synthetic construct; identical to SEQ ID NO: 142
  source 1..36: mol_type = other RNA

SEQ ID NO: 145 - RNA, 36 nt, synthetic construct; identical to SEQ ID NO: 142
  source 1..36: mol_type = other RNA

SEQ ID NO: 146 - RNA, 36 nt, synthetic construct; identical to SEQ ID NO: 143
  source 1..36: mol_type = other RNA

SEQ ID NO: 147 - RNA, 30 nt, synthetic construct
  source 1..30: mol_type = other RNA
ttgttccattttgctgtggaacattgacgc

SEQ ID NO: 148 - RNA, 30 nt, synthetic construct
  source 1..30: mol_type = other RNA
gcgtcaatgttccacagcaaaatggaacaa

SEQ ID NO: 149 - RNA, 37 nt, synthetic construct
  source 1..37: mol_type = other RNA
ggtagcgttgttccattttgctgtggaacattgacgc

SEQ ID NO: 150 - RNA, 37 nt, synthetic construct
  source 1..37: mol_type = other RNA
gcgtcaatgttccacagcaaaatggaacaacgctacc

SEQ ID NO: 151 - RNA, 36 nt, synthetic construct; identical to SEQ ID NO: 142
  source 1..36: mol_type = other RNA

SEQ ID NO: 152 - RNA, 36 nt, synthetic construct; identical to SEQ ID NO: 143
  source 1..36: mol_type = other RNA

SEQ ID NO: 153 - RNA, 36 nt, synthetic construct
  source 1..36: mol_type = other RNA
atcgcaacatctcagaaacccgtcctaagttgacgg

SEQ ID NO: 154 - RNA, 36 nt, synthetic construct
  source 1..36: mol_type = other RNA
gccccatcactaggggcattcttgtgccaccctgag

SEQ ID NO: 155 - RNA, 38 nt, synthetic construct
  source 1..38: mol_type = other RNA
gtacaggcatggtgggaaacaccatgtccattgtgaca

SEQ ID NO: 156 - RNA, 38 nt, synthetic construct
  source 1..38: mol_type = other RNA
tgtcacaatggacatggtgtttcccaccatgcctgtac

SEQ ID NO: 157 - RNA, 38 nt, synthetic construct
  source 1..38: mol_type = other RNA
gtacaggcatggtgagaaacaccatgtccattgtgaca

SEQ ID NO: 158 - RNA, 38 nt, synthetic construct
  source 1..38: mol_type = other RNA
tgtcacaatggacatggtgtttctcaccatgcctgtac

SEQ ID NO: 159 - RNA, 38 nt, synthetic construct
  source 1..38: mol_type = other RNA
gtacaggcatggtgggaaacaccatgtccattgtgact

SEQ ID NO: 160 - RNA, 38 nt, synthetic construct
  source 1..38: mol_type = other RNA
agtcacaatggacatggtgtttcccaccatgcctgtac

SEQ ID NO: 161 - RNA, 36 nt, synthetic construct
  source 1..36: mol_type = other RNA
cccgacgggggcgagaaactgtgactcttatgtcac

SEQ ID NO: 162 - RNA, 36 nt, synthetic construct
  source 1..36: mol_type = other RNA
gtgacataagagtcacagtttctcgcccccgtcggg

SEQ ID NO: 163 - RNA, 36 nt, synthetic construct; identical to SEQ ID NO: 161
  source 1..36: mol_type = other RNA

SEQ ID NO: 164 - RNA, 36 nt, synthetic construct; identical to SEQ ID NO: 162
  source 1..36: mol_type = other RNA

SEQ ID NO: 165 - RNA, 35 nt, synthetic construct
  source 1..35: mol_type = other RNA
cccgacgggggcgagaaactgtgactcttatgtca

SEQ ID NO: 166 - RNA, 35 nt, synthetic construct
  source 1..35: mol_type = other RNA
tgacataagagtcacagtttctcgcccccgtcggg

SEQ ID NO: 167 - RNA, 23 nt, synthetic construct
  source 1..23: mol_type = other RNA
tgaggctcgacttgccgctggga

SEQ ID NO: 168 - RNA, 23 nt, synthetic construct
  source 1..23: mol_type = other RNA
tcccagcggcaagtcgagcctca

SEQ ID NO: 169 - RNA, 23 nt, synthetic construct
  source 1..23: mol_type = other RNA
tgaggctcggcttgccgctggga

SEQ ID NO: 170 - RNA, 23 nt, synthetic construct
  source 1..23: mol_type = other RNA
tcccagcggcaagccgagcctca

SEQ ID NO: 171 - DNA, 8057 bp, synthetic construct
  source 1..8057: mol_type = other DNA
tgtagtcttatgcaatactcttgtagtcttgcaacatggtaacgatgagttagcaacatgccttacaaggagagaaaaagcaccgtgcatgccgattggtggaagtaaggtggtacgatcgtgccttattaggaaggcaacagacgggtctgacatggattggacgaaccactgaattgccgcattgcagagatattgtatttaagtgcctagctcgatacataaacgggtctctctggttagaccagatctgagcctgggagctctctggctaactagggaacccactgcttaagcctcaataaagcttgccttgagtgcttcaagtagtgtgtgcccgtctgttgtgtgactctggtaactagagatccctcagacccttttagtcagtgtggaaaatctctagcagtggcgcccgaacagggacttgaaagcgaaagggaaaccagaggagctctctcgacgcaggactcggcttgctgaagcgcgcacggcaagaggcgaggggcggcgactggtgagtacgccaaaaattttgactagcggaggctagaaggagagagatgggtgcgagagcgtcagtattaagcgggggagaattagatcgcgatgggaaaaaattcggttaaggccagggggaaagaaaaaatataaattaaaacatatagtatgggcaagcagggagctagaacgattcgcagttaatcctggcctgttagaaacatcagaaggctgtagacaaatactgggacagctacaaccatcccttcagacaggatcagaagaacttagatcattatataatacagtagcaaccctctattgtgtgcatcaaaggatagagataaaagacaccaaggaagctttagacaagatagaggaagagcaaaacaaaagtaagaccaccgcacagcaagcggccactgatcttcagacctggaggaggagatatgagggacaattggagaagtgaattatataaatataaagtagtaaaaattgaaccattaggagtagcacccaccaaggcaaagagaagagtggtgcagagagaaaaaagagcagtgggaataggagctttgttccttgggttcttgggagcagcaggaagcactatgggcgcagcgtcaatgacgctgacggtacaggccagacaattattgtctggtatagtgcagcagcagaacaatttgctgagggctattgaggcgcaacagcatctgttgcaactcacagtctggggcatcaagcagctccaggcaagaatcctggctgtggaaagatacctaaaggatcaacagctcctggggatttggggttgctctggaaaactcatttgcaccactgctgtgccttggaatgctagttggagtaataaatctctggaacagatttggaatcacacgacctggatggagtgggacagagaaattaacaattacacaagcttaatacactccttaattgaagaatcgcaaaaccagcaagaaaagaatgaacaagaattattggaattagataaatgggcaagtttgtggaattggtttaacataacaaattggctgtggtatataaaattattcataatgatagtaggaggcttggtaggtttaagaatagtttttgctgtactttctatagtgaatagagttaggcagggatattcaccattatcgtttcagacccacctcccaaccccgaggggacccgacaggcccgaaggaatagaagaagaaggtggagagagagacagagacagatccattcgattagtgaacggatctcgacggtatcggttaacttttaaaagaaaaggggggattggggggtacagtgcaggggaaagaatagtagacataatagcaacagacatacaaactaaagaattacaaaaacaaattacaaaattcaaaattttatcgatactagtattatgcccagtacatgaccttatgggactttcctacttggcagtacatctacgtattagtcatcgctattaccatggtgatgcggttttggcagtacatcaatgggcgtggatagcggtttgactcacggggatttccaagtctccaccccattgacgtcaatgggagtttgttttggcaccaaaatcaacgggactttccaaaatgtcgtaacaactccgccccattgacgcaaatgggcggtaggcgtgtacggtgggaggtttatataagcagagctcgtttagtgaaccgtcagatcgcctggagacgccatccacgctgttttgacctccatagaagattctagagctagcgaattgggatccctagagatccgacgccgccatctctaggcccgcgccggccccctcgcacagacttgtgggagaagctcggctactcccctgccccggttaatttgcatataatatttcctagtaactatagaggcttaatgtgcgataaaagacagataatctgttctttttaatactagctacattttacatgataggcttggatttctataagagatacaaatactaaattattattttaaaaaacagcacaaaaggaaactcaccctaactgtaaagtaattgtgtgttttgagactataaatatgcatgcgagaaaagccttgtttgccaccatggaacggctcggagatatccagcgtacggctctcatcaactccactggggaagaagtggccatgcgcaagctggtgcgctcagtgactgtggttgaggacgacgaggatgaggatggagatgacctgctccatcaccaccacggctcccactgcagcagctcgggggaccccgctgagtacaacctgcgctcgcgcaccgtgctgtgcgggacctgcgggcagcctgccgacaaggcatctgccagcggctcaggagcccaggtgggcggacccatctcctctggctcttctgcctccagtgtcacggtcactcgcagctaccgcagtgtggggggcagtgggggtggcagcttcggggacaatctggtcacccgctcctacctcctgggcaactccagcccccgaacccagagcccccagaactgcagcatcatgtaatctgtctagaagaattcctcgaggcggccgctaaatagttgaatttaaatagatctccagcacagtggtaaatagttgattcgaacaaggatctgcgatcgctccggtgcccgtcagtgggcagagcgcacatcgcccacagtccccgagaagttggggggaggggtcggcaattgaacgggtgcctagagaaggtggcgcggggtaaactgggaaagtgatgtcgtgtactggctccgcctttttcccgagggtgggggagaaccgtatataagtgcagtagtcgccgtgaacgttctttttcgcaacgggtttgccgccagaacacagctgaagcttcgaggggctcgcatctctccttcacgcgcccgccgccctacctgaggccgccatccacgccggttgagtcgcgttctgccgcctcccgcctgtggtgcctcctgaactgcgtccgccgtctaggtaagtttaaagctcaggtcgagaccgggcctttgtccggcgctcccttggagcctacctagactcagccggctctccacgctttgcctgaccctgcttgctcaactctacgtctttgtttcgttttctgttctgcgccgttacagatccaagctgtgaccggcgcctacgcccatgggcatggccaagcctttgtctcaagaagaatccaccctcattgaaagagcaacggctacaatcaacagcatccccatctctgaagactacagcgtcgccagcgcagctctctctagcgacggccgcatcttcactggtgtcaatgtatatcattttactgggggaccttgtgcagaactcgtggtgctgggcactgctgctgctgcggcagctggcaacctgacttgtatcgtcgcgatcggaaatgagaacaggggcatcttgagcccctgcggacggtgccgacaggtgcttctcgatctgcatcctgggatcaaagccatagtgaaggacagtgatggacagccgacggcagttgggattcgtgaattgctgccctctggttatgtgtgggagggctaagcacaattcgagctcgcgtcgacaatcaacctctggattacaaaatttgtgaaagattgactggtattcttaactatgttgctccttttacgctatgtggatacgctgctttaatgcctttgtatcatgctattgcttcccgtatggctttcattttctcctccttgtataaatcctggttgctgtctctttatgaggagttgtggcccgttgtcaggcaacgtggcgtggtgtgcactgtgtttgctgacgcaacccccactggttggggcattgccaccacctgtcagctcctttccgggactttcgctttccccctccctattgccacggcggaactcatcgccgcctgccttgcccgctgctggacaggggctcggctgttgggcactgacaattccgtggtgttgtcggggaaatcatcgtcctttccttggctgctcgcctgtgttgccacctggattctgcgcgggacgtccttctgctacgtcccttcggccctcaatccagcggaccttccttcccgcggcctgctgccggctctgcggcctcttccgcgtcttcgccttcgccctcagacgagtcggatctccctttgggccgcctccccgcctggtacctttaagaccaatgacttacaaggcagctgtagatcttagccactttttaaaagaaaaggggggactggaagggctaattcactcccaacgaagataagatctgctttttgcttgtactgggtctctctggttagaccagatctgagcctgggagctctctggctaactagggaacccactgcttaagcctcaataaagcttgccttgagtgcttcaagtagtgtgtgcccgtctgttgtgtgactctggtaactagagatccctcagacccttttagtcagtgtggaaaatctctagcagtagtagttcatgtcatcttattattcagtatttataacttgcaaagaaatgaatatcagagagtgagaggaacttgtttattgcagcttataatggttacaaataaagcaatagcatcacaaatttcacaaataaagcatttttttcactgcattctagttgtggtttgtccaaactcatcaatgtatcttatcatgtctggctctagctatcccgcccctaactccgcccatcccgcccctaactccgcccagttccgcccattctccgccccatggctgactaattttttttatttatgcagaggccgaggccgcctcggcctctgagctattccagaagtagtgaggaggcttttttggaggcctagacttttgcagagaccaaattcgtaatcatgtcatagctgtttcctgtgtgaaattgttatccgctcacaattccacacaacatacgagccggaagcataaagtgtaaagcctggggtgcctaatgagtgagctaactcacattaattgcgttgcgctcactgcccgctttccagtcgggaaacctgtcgtgccagctgcattaatgaatcggccaacgcgcggggagaggcggtttgcgtattgggcgctcttccgcttcctcgctcactgactcgctgcgctcggtcgttcggctgcggcgagcggtatcagctcactcaaaggcggtaatacggttatccacagaatcaggggataacgcaggaaagaacatgtgagcaaaaggccagcaaaaggccaggaaccgtaaaaaggccgcgttgctggcgtttttccataggctccgcccccctgacgagcatcacaaaaatcgacgctcaagtcagaggtggcgaaacccgacaggactataaagataccaggcgtttccccctggaagctccctcgtgcgctctcctgttccgaccctgccgcttaccggatacctgtccgcctttctcccttcgggaagcgtggcgctttctcatagctcacgctgtaggtatctcagttcggtgtaggtcgttcgctccaagctgggctgtgtgcacgaaccccccgttcagcccgaccgctgcgccttatccggtaactatcgtcttgagtccaacccggtaagacacgacttatcgccactggcagcagccactggtaacaggattagcagagcgaggtatgtaggcggtgctacagagttcttgaagtggtggcctaactacggctacactagaagaacagtatttggtatctgcgctctgctgaagccagttaccttcggaaaaagagttggtagctcttgatccggcaaacaaaccaccgctggtagcggtggtttttttgtttgcaagcagcagattacgcgcagaaaaaaaggatctcaagaagatcctttgatcttttctacggggtctgacgctcagtggaacgaaaactcacgttaagggattttggtcatgagattatcaaaaaggatcttcacctagatccttttaaattaaaaatgaagttttaaatcaatctaaagtatatatgagtaaacttggtctgacagttaccaatgcttaatcagtgaggcacctatctcagcgatctgtctatttcgttcatccatagttgcctgactccccgtcgtgtagataactacgatacgggagggcttaccatctggccccagtgctgcaatgataccgcgagacccacgctcaccggctccagatttatcagcaataaaccagccagccggaagggccgagcgcagaagtggtcctgcaactttatccgcctccatccagtctattaattgttgccgggaagctagagtaagtagttcgccagttaatagtttgcgcaacgttgttgccattgctacaggcatcgtggtgtcacgctcgtcgtttggtatggcttcattcagctccggttcccaacgatcaaggcgagttacatgatcccccatgttgtgcaaaaaagcggttagctccttcggtcctccgatcgttgtcagaagtaagttggccgcagtgttatcactcatggttatggcagcactgcataattctcttactgtcatgccatccgtaagatgcttttctgtgactggtgagtactcaaccaagtcattctgagaatagtgtatgcggcgaccgagttgctcttgcccggcgtcaatacgggataataccgcgccacatagcagaactttaaaagtgctcatcattggaaaacgttcttcggggcgaaaactctcaaggatcttaccgctgttgagatccagttcgatgtaacccactcgtgcacccaactgatcttcagcatcttttactttcaccagcgtttctgggtgagcaaaaacaggaaggcaaaatgccgcaaaaaagggaataagggcgacacggaaatgttgaatactcatactcttcctttttcaatattattgaagcatttatcagggttattgtctcatgagcggatacatatttgaatgtatttagaaaaataaacaaataggggttccgcgcacatttccccgaaaagtgccacctgacgtctaagaaaccattattatcatgacattaacctataaaaataggcgtatcacgaggccctttcgtctcgcgcgtttcggtgatgacggtgaaaacctctgacacatgcagctcccggagacggtcacagcttgtctgtaagcggatgccgggagcagacaagcccgtcagggcgcgtcagcgggtgttggcgggtgtcggggctggcttaactatgcggcatcagagcagattgtactgagagtgcaccatatgcggtgtgaaataccgcacagatgcgtaaggagaaaataccgcatcaggcgccattcgccattcaggctgcgcaactgttgggaagggcgatcggtgcgggcctcttcgctattacgccagctggcgaaagggggatgtgctgcaaggcgattaagttgggtaacgccagggttttcccagtcacgacgttgtaaaacgacggccagtgccaagctgacgcg

SEQ ID NO: 172 - DNA, 68 bp, synthetic construct
  source 1..68: mol_type = other DNA
tgtttgccaccatggaacggctcggagatcatcattgcgnnnnnnnaccgagtacaagcccacggtgc

SEQ ID NO: 173 - DNA, 52 bp, synthetic construct
  source 1..52: mol_type = other DNA
taaattcaactatttagcggccgcctcgagtcaggcaccgggcttgcgggtc

SEQ ID NO: 174 - DNA, 8231 bp, synthetic construct
  source 1..8231: mol_type = other DNA
tgtagtcttatgcaatactcttgtagtcttgcaacatggtaacgatgagttagcaacatgccttacaaggagagaaaaagcaccgtgcatgccgattggtggaagtaaggtggtacgatcgtgccttattaggaaggcaacagacgggtctgacatggattggacgaaccactgaattgccgcattgcagagatattgtatttaagtgcctagctcgatacataaacgggtctctctggttagaccagatctgagcctgggagctctctggctaactagggaacccactgcttaagcctcaataaagcttgccttgagtgcttcaagtagtgtgtgcccgtctgttgtgtgactctggtaactagagatccctcagacccttttagtcagtgtggaaaatctctagcagtggcgcccgaacagggacttgaaagcgaaagggaaaccagaggagctctctcgacgcaggactcggcttgctgaagcgcgcacggcaagaggcgaggggcggcgactggtgagtacgccaaaaattttgactagcggaggctagaaggagagagatgggtgcgagagcgtcagtattaagcgggggagaattagatcgcgatgggaaaaaattcggttaaggccagggggaaagaaaaaatataaattaaaacatatagtatgggcaagcagggagctagaacgattcgcagttaatcctggcctgttagaaacatcagaaggctgtagacaaatactgggacagctacaaccatcccttcagacaggatcagaagaacttagatcattatataatacagtagcaaccctctattgtgtgcatcaaaggatagagataaaagacaccaaggaagctttagacaagatagaggaagagcaaaacaaaagtaagaccaccgcacagcaagcggccactgatcttcagacctggaggaggagatatgagggacaattggagaagtgaattatataaatataaagtagtaaaaattgaaccattaggagtagcacccaccaaggcaaagagaagagtggtgcagagagaaaaaagagcagtgggaataggagctttgttccttgggttcttgggagcagcaggaagcactatgggcgcagcgtcaatgacgctgacggtacaggccagacaattattgtctggtatagtgcagcagcagaacaatttgctgagggctattgaggcgcaacagcatctgttgcaactcacagtctggggcatcaagcagctccaggcaagaatcctggctgtggaaagatacctaaaggatcaacagctcctggggatttggggttgctctggaaaactcatttgcaccactgctgtgccttggaatgctagttggagtaataaatctctggaacagatttggaatcacacgacctggatggagtgggacagagaaattaacaattacacaagcttaatacactccttaattgaagaatcgcaaaaccagcaagaaaagaatgaacaagaattattggaattagataaatgggcaagtttgtggaattggtttaacataacaaattggctgtggtatataaaattattcataatgatagtaggaggcttggtaggtttaagaatagtttttgctgtactttctatagtgaatagagttaggcagggatattcaccattatcgtttcagacccacctcccaaccccgaggggacccgacaggcccgaaggaatagaagaagaaggtggagagagagacagagacagatccattcgattagtgaacggatctcgacggtatcggttaacttttaaaagaaaaggggggattggggggtacagtgcaggggaaagaatagtagacataatagcaacagacatacaaactaaagaattacaaaaacaaattacaaaattcaaaattttatcgatactagtattatgcccagtacatgaccttatgggactttcctacttggcagtacatctacgtattagtcatcgctattaccatggtgatgcggttttggcagtacatcaatgggcgtggatagcggtttgactcacggggatttccaagtctccaccccattgacgtcaatgggagtttgttttggcaccaaaatcaacgggactttccaaaatgtcgtaacaactccgccccattgacgcaaatgggcggtaggcgtgtacggtgggaggtttatataagcagagctcgtttagtgaaccgtcagatcgcctggagacgccatccacgctgttttgacctccatagaagattctagagctagcgaattgggatccctagagatccgacgccgccatctctaggcccgcgccggccccctcgcacagacttgtgggagaagctcggctactcccctgccccggttaatttgcatataatatttcctagtaactatagaggcttaatgtgcgataaaagacagataatctgttctttttaatactagctacattttacatgataggcttggatttctataagagatacaaatactaaattattattttaaaaaacagcacaaaaggaaactcaccctaactgtaaagtaattgtgtgttttgagactataaatatgcatgcgagaaaagccttgtttgccaccatggaacggctcggagatcatcattgcgnnnnnnnaccgagtacaagcccacggtgcgcctcgccacccgcgacgacgtccccagggccgtacgcaccctcgccgccgcgttcgccgactaccccgccacgcgccacaccgtcgatccggaccgccacatcgagcgggtcaccgagctgcaagaactcttcctcacgcgcgtcgggctcgacatcggcaaggtgtgggtcgcggacgacggcgccgcggtggcggtctggaccacgccggagagcgtcgaagcgggggcggtgttcgccgagatcggcccgcgcatggccgagttgagcggttcccggctggccgcgcagcaacagatggaaggcctcctggcgccgcaccggcccaaggagcccgcgtggttcctggccaccgtcggcgtctcgcccgaccaccagggcaagggtctgggcagcgccgtcgtgctccccggagtggaggcggccgagcgcgccggggtgcccgccttcctggagacctccgcgccccgcaacctccccttctacgagcggctcggcttcaccgtcaccgccgacgtcgaggtgcccgaaggaccgcgcacctggtgcatgacccgcaagcccggtgcctgactcgaggcggccgctaaatagttgaatttaaatagatctccagcacagtggtaaatagttgattcgaacaaggatctgcgatcgctccggtgcccgtcagtgggcagagcgcacatcgcccacagtccccgagaagttggggggaggggtcggcaattgaacgggtgcctagagaaggtggcgcggggtaaactgggaaagtgatgtcgtgtactggctccgcctttttcccgagggtgggggagaaccgtatataagtgcagtagtcgccgtgaacgttctttttcgcaacgggtttgccgccagaacacagctgaagcttcgaggggctcgcatctctccttcacgcgcccgccgccctacctgaggccgccatccacgccggttgagtcgcgttctgccgcctcccgcctgtggtgcctcctgaactgcgtccgccgtctaggtaagtttaaagctcaggtcgagaccgggcctttgtccggcgctcccttggagcctacctagactcagccggctctccacgctttgcctgaccctgcttgctcaactctacgtctttgtttcgttttctgttctgcgccgttacagatccaagctgtgaccggcgcctacgcccatgggcatggccaagcctttgtctcaagaagaatccaccctcattgaaagagcaacggctacaatcaacagcatccccatctctgaagactacagcgtcgccagcgcagctctctctagcgacggccgcatcttcactggtgtcaatgtatatcattttactgggggaccttgtgcagaactcgtggtgctgggcactgctgctgctgcggcagctggcaacctgacttgtatcgtcgcgatcggaaatgagaacaggggcatcttgagcccctgcggacggtgccgacaggtgcttctcgatctgcatcctgggatcaaagccatagtgaaggacagtgatggacagccgacggcagttgggattcgtgaattgctgccctctggttatgtgtgggagggctaagcacaattcgagctcgcgtcgacaatcaacctctggattacaaaatttgtgaaagattgactggtattcttaactatgttgctccttttacgctatgtggatacgctgctttaatgcctttgtatcatgctattgcttcccgtatggctttcattttctcctccttgtataaatcctggttgctgtctctttatgaggagttgtggcccgttgtcaggcaacgtggcgtggtgtgcactgtgtttgctgacgcaacccccactggttggggcattgccaccacctgtcagctcctttccgggactttcgctttccccctccctattgccacggcggaactcatcgccgcctgccttgcccgctgctggacaggggctcggctgttgggcactgacaattccgtggtgttgtcggggaaatcatcgtcctttccttggctgctcgcctgtgttgccacctggattctgcgcgggacgtccttctgctacgtcccttcggccctcaatccagcggaccttccttcccgcggcctgctgccggctctgcggcctcttccgcgtcttcgccttcgccctcagacgagtcggatctccctttgggccgcctccccgcctggtacctttaagaccaatgacttacaaggcagctgtagatcttagccactttttaaaagaaaaggggggactggaagggctaattcactcccaacgaagataagatctgctttttgcttgtactgggtctctctggttagaccagatctgagcctgggagctctctggctaactagggaacccactgcttaagcctcaataaagcttgccttgagtgcttcaagtagtgtgtgcccgtctgttgtgtgactctggtaactagagatccctcagacccttttagtcagtgtggaaaatctctagcagtagtagttcatgtcatcttattattcagtatttataacttgcaaagaaatgaatatcagagagtgagaggaacttgtttattgcagcttataatggttacaaataaagcaatagcatcacaaatttcacaaataaagcatttttttcactgcattctagttgtggtttgtccaaactcatcaatgtatcttatcatgtctggctctagctatcccgcccctaactccgcccatcccgcccctaactccgcccagttccgcccattctccgccccatggctgactaattttttttatttatgcagaggccgaggccgcctcggcctctgagctattccagaagtagtgaggaggcttttttggaggcctagacttttgcagagaccaaattcgtaatcatgtcatagctgtttcctgtgtgaaattgttatccgctcacaattccacacaacatacgagccggaagcataaagtgtaaagcctggggtgcctaatgagtgagctaactcacattaattgcgttgcgctcactgcccgctttccagtcgggaaacctgtcgtgccagctgcattaatgaatcggccaacgcgcggggagaggcggtttgcgtattgggcgctcttccgcttcctcgctcactgactcgctgcgctcggtcgttcggctgcggcgagcggtatcagctcactcaaaggcggtaatacggttatccacagaatcaggggataacgcaggaaagaacatgtgagcaaaaggccagcaaaaggccaggaaccgtaaaaaggccgcgttgctggcgtttttccataggctccgcccccctgacgagcatcacaaaaatcgacgctcaagtcagaggtggcgaaacccgacaggactataaagataccaggcgtttccccctggaagctccctcgtgcgctctcctgttccgaccctgccgcttaccggatacctgtccgcctttctcccttcgggaagcgtggcgctttctcatagctcacgctgtaggtatctcagttcggtgtaggtcgttcgctccaagctgggctgtgtgcacgaaccccccgttcagcccgaccgctgcgccttatccggtaactatcgtcttgagtccaacccggtaagacacgacttatcgccactggcagcagccactggtaacaggattagcagagcgaggtatgtaggcggtgctacagagttcttgaagtggtggcctaactacggctacactagaagaacagtatttggtatctgcgctctgctgaagccagttaccttcggaaaaagagttggtagctcttgatccggcaaacaaaccaccgctggtagcggtggtttttttgtttgcaagcagcagattacgcgcagaaaaaaaggatctcaagaagatcctttgatcttttctacggggtctgacgctcagtggaacgaaaactcacgttaagggattttggtcatgagattatcaaaaaggatcttcacctagatccttttaaattaaaaatgaagttttaaatcaatctaaagtatatatgagtaaacttggtctgacagttaccaatgcttaatcagtgaggcacctatctcagcgatctgtctatttcgttcatccatagttgcctgactccccgtcgtgtagataactacgatacgggagggcttaccatctggccccagtgctgcaatgataccgcgagacccacgctcaccggctccagatttatcagcaataaaccagccagccggaagggccgagcgcagaagtggtcctgcaactttatccgcctccatccagtctattaattgttgccgggaagctagagtaagtagttcgccagttaatagtttgcgcaacgttgttgccattgctacaggcatcgtggtgtcacgctcgtcgtttggtatggcttcattcagctccggttcccaacgatcaaggcgagttacatgatcccccatgttgtgcaaaaaagcggttagctccttcggtcctccgatcgttgtcagaagtaagttggccgcagtgttatcactcatggttatggcagcactgcataattctcttactgtcatgccatccgtaagatgcttttctgtgactggtgagtactcaaccaagtcattctgagaatagtgtatgcggcgaccgagttgctcttgcccggcgtcaatacgggataataccgcgccacatagcagaactttaaaagtgctcatcattggaaaacgttcttcggggcgaaaactctcaaggatcttaccgctgttgagatccagttcgatgtaacccactcgtgcacccaactgatcttcagcatcttttactttcaccagcgtttctgggtgagcaaaaacaggaaggcaaaatgccgcaaaaaagggaataagggcgacacggaaatgttgaatactcatactcttcctttttcaatattattgaagcatttatcagggttattgtctcatgagcggatacatatttgaatgtatttagaaaaataaacaaataggggttccgcgcacatttccccgaaaagtgccacctgacgtctaagaaaccattattatcatgacattaacctataaaaataggcgtatcacgaggccctttcgtctcgcgcgtttcggtgatgacggtgaaaacctctgacacatgcagctcccggagacggtcacagcttgtctgtaagcggatgccgggagcagacaagcccgtcagggcgcgtcagcgggtgttggcgggtgtcggggctggcttaactatgcggcatcagagcagattgtactgagagtgcaccatatgcggtgtgaaataccgcacagatgcgtaaggagaaaataccgcatcaggcgccattcgccattcaggctgcgcaactgttgggaagggcgatcggtgcgggcctcttcgctattacgccagctggcgaaagggggatgtgctgcaaggcgattaagttgggtaacgccagggttttcccagtcacgacgttgtaaaacgacggccagtgccaagctgacgcg

SEQ ID NO: 175 - DNA, 790 bp, synthetic construct
  source 1..790: mol_type = other DNA
tctagagcgagaaaagccttgtttgccaccatggaacggctcggagatcatcattgcgtcgcgaggtgagcaagggcgaggagctgttcaccggggtggtgcccatcctggtcgagctggacggcgacgtaaacggccacaagttcagcgtgtccggcgagggcgagggcgatgccacctacggcaagctgaccctgaagttcatctgcaccaccggcaagctgcccgtgccctggcccaccctcgtgaccaccctgacctacggcgtgcagtgcttcagccgctaccccgaccacatgaagcagcacgacttcttcaagtccgccatgcccgaaggctacgtccaggagcgcaccatcttcttcaaggacgacggcaactacaagacccgcgccgaggtgaagttcgagggcgacaccctggtgaaccgcatcgagctgaagggcatcgacttcaaggaggacggcaacatcctggggcacaagctggagtacaactacaacagccacaacgtctatatcatggccgacaagcagaagaacggcatcaaggtgaacttcaagatccgccacaacatcgaggacggcagcgtgcagctcgccgaccactaccagcagaacacccccatcggcgacggccccgtgctgctgcccgacaaccactacctgagcacccagtccaagctgagcaaagaccccaacgagaagcgcgatcacatggtcctgctggagttcgtgaccgccgccgggatcactctcggcatggacgagctgtacaagtaagcggccgc

SEQ ID NO: 176 - DNA, 5239 bp, synthetic construct
  source 1..5239: mol_type = other DNA
atcataagatgatcttcttgagatcgttttggtctgcgcgtaatctcttgctctgaaaacgaaaaaaccgccttgcagggcggtttttcgaaggttctctgagctaccaactctttgaaccgaggtaactggcttggaggagcgcagtcaccaaaacttgtcctttcagtttagccttaaccggcgcatgacttcaagactaactcctctaaatcaattaccagtggctgctgccagtggtgcttttgcatgtctttccgggttggactcaagacgatagttaccggataaggcgcagcggtcggactgaacggggggttcgtgcatacagtccagcttggagcgaactgcctacccggaactgagtgtcaggcgtggaatgagacaaacgcggccataacagcggaatgacaccggtaaaccgaaaggcaggaacaggagagcgcacgagggagccgccagggggaaacgcctggtatctttatagtcctgtcgggtttcgccaccactgatttgagcgtcagatttcgtgatgcttgtcaggggggcggagcctatggaaaaacggctttgccgcggccctctcacttccctgttaagtatcttcctggcatcttccaggaaatctccgccccgttcgtaagccatttccgctcgccgcagtcgaacgaccgagcgtagcgagtcagtgagcgaggaagcggaatatatcctgtatcacatattctgctgacgcaccggtgcagccttttttctcctgccacatgaagcacttcactgacaccctcatcagtgccaacatagtaagccagtatacactccgctagcgctgatgtccggcggtgcttttgccgttacgcaccaccccgtcagtagctgaacaggagggacagctgatagaaacagaagccactggagcacctcaaaaacaccatcatacactaaatcagtaagttggcagcatcacccgacgcactttgcgccgaataaatacctgtgacggaagatcacttcgcagaataaataaatcctggtgtccctgttgataccgggaagccccgggccaacttttggcgaaaatgagacgttgatcggcacgtaagaggttccaactttcaccataatgaaataagatcactaccgggcgtattttttgagttatcgagattttcaggagctaaggaagctaaaatggagaaaaaaatcactggatataccaccgttgatatatcccaatggcatcgtaaagaacattttgaggcatttcagtcagttgctcaatgtacctataaccagaccgttcagctggatattacggcctttttaaagaccgtaaagaaaaataagcacaagttttatccggcctttattcacattcttgcccgcctgatgaatgctcatccggaattccgtatggcaatgaaagacggtgagctggtgatatgggatagtgttcacccttgttacaccgttttccatgagcaaactgaaacgttttcatcgctctggagtgaataccacgacgatttccggcagtttctacacatatattcgcaagatgtggcgtgttacggtgaaaacctggcctatttccctaaagggtttattgagaatatgtttttcgtctcagccaatccctgggtgagtttcaccagttttgatttaaacgtggccaatatggacaacttcttcgcccccgttttcaccatgggcaaatattatacgcaaggcgacaaggtgctgatgccgctggcgattcaggttcatcatgccgtttgtgatggcttccatgtcggcagaatgcttaatgaattacaacagtactgcgatgagtggcagggcggggcgtaatttggtacatctcaaataaaacgaaaggctcagtcgaaagactgggcctttcgttttatctgttgtttgtcggtgaacgctctcgttaactagctatactgatttcgtcagactcacagtcaaacatgccggtcagttggcctggtgatggcgggatcgttgtatatttcttgacaccttttcggcaccgccctaaaattctgcgtcctcataatatatgaggcgatttattacgtgtttacgaagcaaaagctaaaaccaggagctatttaatgccggcagctaagaaaaagaaactggatggcagcgtcgacatggccgtgcagaacgacagctgggacattcagagatgtcagaagctgaagctgggcaagaaggagctgagccccatcaacgccaagttctacgacgacatccaagaggactacagaaagctgttccccctgatcctgagcttcaccctgaccccctacaccttcgaggacgagaacggcgtggagcacgtggtgagcagcgagcaagtgctcaagaccctggagaacagcgtgggcaagagcctgatcgatgatgtgctgatcatcggcagcaccgtggccgagatgccccaagcctccgcctcctccttctacggcctcttctacaacaactacagctgcaacgacaaggccaagtggacccaagccaagagcgacttcctggacaagctgctgacctacaccgacgagcagctggaggccaagctggagggcgacagctgcctgagacagatgcccctggtggagtggaagaaggtgaaggagaagctgctggagggcaacgacaagaaagaggtgtgggagagcgtgagcggcaagctggccaacaaggtgaacagcagctacagcagagtgagaaaggagctggagatccaagtgagacagcccgacaacagagagtactgcagcaccctgagcgagatgctgagactgcaagtgaagagctgctatcagaagaacctggaccatcagaaggtgacccaagagctgctgaccaaggtgaacaactgcagccaaaccaaccccaagatcttcgacctgatcgccaacttcagcgacagactgtacagcatcggcaccggcctgagcaagaacgtgctgctgagaagcatcgactgcgtgaacaagggcaccctggcctccaaccccacctacaagatcgccatcgccgagctgctgaagcccgagttcagcgagatcctgaccctgaagaaggaggagctgatcagagcctacaacggcgtgaagatcagagatcagctgaagagaagaaaggtgtaccctagactgcctagcttcaagaatgactacaaggtgatgttcggcctgagcagcctggccaagttcaaaatcagagtggaggacaagaagatcaagatcgccttcagcaacggcgaggaagagctgttcatgaacagccactacttccacgacctggaggtggtgttcgacgagagcaacaagaccgccaagcagttcatcatcaagttcagacacaagctgaagtccaacaagaagttcgccgtgagcgacctgatcaccggctatgtgaaacaaatcggcctgcagaagaaaaacggctccttctatgtgaccctgatgttcaccatgaagcacgacgagaagatcctgaagctggagagattcttcaagaccgcctcccccgacatgagcaagtacaccgacctgcccgacaagatcagagtggccggcttcgacctgaacatcagcaaccccgtggtgggctgcatcgccgagatcgacaagaacggcaagggccccctgaacagcatcgacttcggcaagggcaacctggtggccggccccgacatcgtgtgccaagacaccctgatgagcaacagagtgaagagatgcaagcagctgatcttcaaggtgaaggacgccatcaaggactgcaagttcagcaacagcaacaacaccaagatgaacgacgccaccatcagcttcctgaagagactggcctccccctcccaaagccctagatgcatgattcagacctggatcaagaacctgaagaagagactgaagaagctgcacagcatcatcagagcctccggctatgtgaacattagcgagggcctgagaatgctggaggcccaagacgccatgaaaagcctgatcagcagctacgagagattccacctgaagagcggcgagatgctggccgccaagaagaacatcaccgccaacaaccggagacagaacttcagacagttcatcagcagaaagatcgcctccaagatcgtgcagtacagcaagggctgcgacgtgatcttcatcgaggacctgagcctggacttcgacagcgacaacaagaacaacagcctgatcagactgttcagcgccgacggcctgatcaagtgcatcaccgacgccgcctacaaggccggcatcggcgtggtgctggtggaccccatgggcacaagcaagaccgaccccgtgaccgccaaggtgggctacagaaacctgaagaacaagaactacctgtacgtggagcgggacggcgtgctgggctgggtggacgccgacaagatcgcctccctgaacgtgctgatcagaggcctgggccacagcatcgtgccctacaagttctacgtgaagggcaagaaaaaggacgtgatcggcgtggacctggtggagaaagaggtgggcaagagactgcagagatacttcaccatgcagcacggcagcatcaagcagcccatcttcaagatcgacaacgacaaggtgaccctgctgaagaaggccaacaagggcgacaacctgatcgagaacgccttcctgtacgcccacggcgacgacttctgcaccgccgacaaccacagaaaccaaggcaaggagatcatgcacagagtggacagcggcgagcccgtggtggagttcgacctgaccccctgcagcgagagcggctacaagagcttccaagccaagacaggcggcggccccggcggcggcgccgccgccggcagcggcagccctaagaaaaaacgaaaagttggcagcggaagcaaaaggccggcggccacgaaaaaggccggccaggcaaaaaagaaaaagctcgagtacccatacgatgttccagattacgcttgagaattcggtaccttgacagctagctcagtcctaggtataatactagtgtgcgaaacggtctcgttagaggctggttcaagcaccgcaatgatgatctccgagccgttcggccggcatggtcccagcctcctcgctggcgccggctgggcaacatgcttcggcatggcgaatgggaccgtacgtcgacgctagcataaccccttggggcctctaaacgggtcttgaggggttttttggat

SEQ ID NO: 177 - DNA, 5770 bp, synthetic construct
  source 1..5770: mol_type = other DNA
atcataagatgatcttcttgagatcgttttggtctgcgcgtaatctcttgctctgaaaacgaaaaaaccgccttgcagggcggtttttcgaaggttctctgagctaccaactctttgaaccgaggtaactggcttggaggagcgcagtcaccaaaacttgtcctttcagtttagccttaaccggcgcatgacttcaagactaactcctctaaatcaattaccagtggctgctgccagtggtgcttttgcatgtctttccgggttggactcaagacgatagttaccggataaggcgcagcggtcggactgaacggggggttcgtgcatacagtccagcttggagcgaactgcctacccggaactgagtgtcaggcgtggaatgagacaaacgcggccataacagcggaatgacaccggtaaaccgaaaggcaggaacaggagagcgcacgagggagccgccagggggaaacgcctggtatctttatagtcctgtcgggtttcgccaccactgatttgagcgtcagatttcgtgatgcttgtcaggggggcggagcctatggaaaaacggctttgccgcggccctctcacttccctgttaagtatcttcctggcatcttccaggaaatctccgccccgttcgtaagccatttccgctcgccgcagtcgaacgaccgagcgtagcgagtcagtgagcgaggaagcggaatatatcctgtatcacatattctgctgacgcaccggtgcagccttttttctcctgccacatgaagcacttcactgacaccctcatcagtgccaacatagtaagccagtatacactccgctagcgctgatgtccggcggtgcttttgccgttacgcaccaccccgtcagtagctgaacaggagggacagctgatagaaacagaagccactggagcacctcaaaaacaccatcatacactaaatcagtaagttggcagcatcacccgacgcactttgcgccgaataaatacctgtgacggaagatcacttcgcagaataaataaatcctggtgtccctgttgataccgggaagccccgggccaacttttggcgaaaatgagacgttgatcggcacgtaagaggttccaactttcaccataatgaaataagatcactaccgggcgtattttttgagttatcgagattttcaggagctaaggaagctaaaatggagaaaaaaatcactggatataccaccgttgatatatcccaatggcatcgtaaagaacattttgaggcatttcagtcagttgctcaatgtacctataaccagaccgttcagctggatattacggcctttttaaagaccgtaaagaaaaataagcacaagttttatccggcctttattcacattcttgcccgcctgatgaatgctcatccggaattccgtatggcaatgaaagacggtgagctggtgatatgggatagtgttcacccttgttacaccgttttccatgagcaaactgaaacgttttcatcgctctggagtgaataccacgacgatttccggcagtttctacacatatattcgcaagatgtggcgtgttacggtgaaaacctggcctatttccctaaagggtttattgagaatatgtttttcgtctcagccaatccctgggtgagtttcaccagttttgatttaaacgtggccaatatggacaacttcttcgcccccgttttcaccatgggcaaatattatacgcaaggcgacaaggtgctgatgccgctggcgattcaggttcatcatgccgtttgtgatggcttccatgtcggcagaatgcttaatgaattacaacagtactgcgatgagtggcagggcggggcgtaatttggtacatctcaaataaaacgaaaggctcagtcgaaagactgggcctttcgttttatctgttgtttgtcggtgaacgctctcgttaactagctatactgatttcgtcagactcacagtcaaacatgccggtcagttggcctggtgatggcgggatcgttgtatatttcttgacaccttttcggcaccgccctaaaattctgcgtcctcataatatatgaggcgatttattacgtgtttacgaagcaaaagctaaaaccaggagctatttaatgccggcagctaagaaaaagaaactggatggcagcgtcgacatcgtgaagcccaagagcatcaagagctacagcagcatgctggatgtggaccatagaaagaacgagatcctgagcagaaccttcgactacctgaacaacggcagcagcgtgttcctgtggaccttcctgagcatcttcggcggcatcaccaaggagatcgccacacagatcctgagccaaaagaccgaggacgagctggacgacagcaaccccgagctgctcctggccatctactggttcagactggtgcccgtgagcagaaagagcaacaacgtgctgccccccctgctgcccaagctgttcaagaagtacctgggcgaggagcccaccaccgaggtgctggagtatttcagcagcaacttcgaccaagagaagtacgtgtggcaagacatgaaggccgagttcaacaacctgtgtagccaaatcggcgtgagcaacgccaacttcgtgctcgacgtgggcctgatggccaacgagggctacatcggcctgaagtgcggcaagacctggggcaccatcagcggcctgttcggcaccggcgagaaggccgacagaaagcccaaggtggacatcctgaacagcgtgatcgccgccgtggagaagaacccccccgccacaagagccgagttcgcctccctgatcctgcagtgcagcggctgcaccaacatcgagcagctgaagctgaagtacggcaacatcggcagagcctccttcgtgatcgtgagagccgaggagatcaacagcagcgcctccatcgacgacaagtacctgaagcagatcaagagaaagctggccgccgacctgaagaagcagagcaacgacctcagctggctctgcaacacacagctgaagaactatctgatcagcaaaattggcgactactatcagcctagctggagcgagatgagcaacaacgccctgcccatcatccaaggcaagaccaccaagaattacaacttcgtgctggagcaagtgagatgcaagagcgagctggaccctagcatgcagatcaagtgggagctggtgaacgcctacttcgcctccaagttcttcaccgccgacaacgtgttcagcatctgcaagttccacatcggcgccggcgaggagctgaagaagctgtggaacagctggaacgatctgagcgacgacgaactggaagagacagtgagcgccttctgccacagcatcaacgagaacggcagaatgcccatctacagcctgctgatgtacttcaacagcatcagcggcaagatcaccctgaaggacgtgctggagggcatcacctacggcgaaaccaagagcaagatcgagagacagaagctgaaccccatcgtggagggcaaggcctccttcaactggggcaacgtgagcaagatcagcggctgcatcatcagccccaaggagaaagaaaagcacatcgtgggcagcaagcacaaccacgacagcagcatctggatcgagatcaccgtgctgaacaaggacaacaagtgggtgaagcaccacttcagaatgttcaacacaagattctacgaagaggtgtaccaccccggcaacgccgagagcgtgcccaacaaaagcgtgcccatcagaagcagaagattcggcttcaacaaccaagtggtgctgagcgaggatcagatcaacaccatcagaaacgcctccaagagcatgagaaaggccatgaagagacaagtgagaatcgtggccgctagacagaacaatcagctgcccgagttcgtgtggaatgacgactttaacattaacatcagcaacgacgaaagaggctacagaaccaccctgagctacaagatcgagaaggagagagtggaaaccgccgacgtgttcgtgggcttcgatcagaatcagaccgctagacacacctacagcgtgctgcagctggtggaccccaaggacgccgaggccatcagcttctgcggcctgggcatcaagctgctggacgtgggctacatcagcagcagccaactggtcaacgacaagagcttcgatcagctgagctacgacggcatcagctgggacagatttcagagctggagagatcagagagaggccttcgtgaccaagtggaagaactgcgtgagcaagaacagaaaggcccaagacgtgcccatcgacatgctggagatcctgaacagaagcagcaagtacatgccctgcctgtacgactacaacgctagatactgcggccacatcaagaagatcatgaagggcaagagcgagaaggacctgatcgagatcagaggcgagatcatggccttcatcaaggacgggcagttcagcgtgctgagactgagcagcctgaaccacaacagcttcagcatgctgcggaacgctaagggcatcatcagcgcctacttcaataacctgatcggcaagcactgcaccgacgagcagaagtgcgacgccgacgaggagctgttcatgctgagaatcgagctggaggagaagagacagaacaaggccatcagcaagaagaacctgatcagcaacagactggtgaccatcgccctggaggtgagaaagatcatcggcagcaacgtggtgatcgtgggcgagaacatcagcaatacaacaagcaaaagcaacaagagcaagcagaacgctagagccatggactggctgagcagaggcgtggccgacaagaccaagcagatgaccgagatgcacgagggcatcagattcagagacatcaaccccgcctacacaagccatcagaaccccttcatccacagaaaccccgacaagagcgtggtgagcatgagagctagattcaagagcgtgagccccaaggagatgacagaggtggacttcaagtacctggtgaagctgtgcaagagcgacgagatcacctactacaccgagggcgctagacacttcacaagccactacgggatcaccaagagcgacatgacacagatcaccttcagcgccttcaagatcctgatgaccaacatcctggagaagagaaacgaaaccaacctgatcttccctagaagcggcggcagactgtacctggccacccacaagatcggcgaatgcctgccctactgctacgacgacgaggacggctggttctgcgacagcgactgcgtggccgccgtgaacatcgccctggtgggcatcgagttcgagagactgagcgccgccaagaaggtggtgatcacccggaacgccaaggtggtcaacacaggcggcggccccggcggcggcgccgccgccggcagcggcagccctaagaaaaaacgaaaagttggcagcggaagcaaaaggccggcggccacgaaaaaggccggccaggcaaaaaagaaaaagctcgagtacccatacgatgttccagattacgcttgagaattcggtaccttgacagctagctcagtcctaggtataatactagtgtttcaatcgatgattattgtgcctgtcattggcaccgcaatgatgatctccgagccgttcggccggcatggtcccagcctcctcgctggcgccggctgggcaacatgcttcggcatggcgaatgggaccgtacgtcgacgctagcataaccccttggggcctctaaacgggtcttgaggggttttttggat

SEQ ID NO: 178 - DNA, 4848 bp, synthetic construct
  source 1..4848: mol_type = other DNA
atcataagatgatcttcttgagatcgttttggtctgcgcgtaatctcttgctctgaaaacgaaaaaaccgccttgcagggcggtttttcgaaggttctctgagctaccaactctttgaaccgaggtaactggcttggaggagcgcagtcaccaaaacttgtcctttcagtttagccttaaccggcgcatgacttcaagactaactcctctaaatcaattaccagtggctgctgccagtggtgcttttgcatgtctttccgggttggactcaagacgatagttaccggataaggcgcagcggtcggactgaacggggggttcgtgcatacagtccagcttggagcgaactgcctacccggaactgagtgtcaggcgtggaatgagacaaacgcggccataacagcggaatgacaccggtaaaccgaaaggcaggaacaggagagcgcacgagggagccgccagggggaaacgcctggtatctttatagtcctgtcgggtttcgccaccactgatttgagcgtcagatttcgtgatgcttgtcaggggggcggagcctatggaaaaacggctttgccgcggccctctcacttccctgttaagtatcttcctggcatcttccaggaaatctccgccccgttcgtaagccatttccgctcgccgcagtcgaacgaccgagcgtagcgagtcagtgagcgaggaagcggaatatatcctgtatcacatattctgctgacgcaccggtgcagccttttttctcctgccacatgaagcacttcactgacaccctcatcagtgccaacatagtaagccagtatacactccgctagcgctgatgtccggcggtgcttttgccgttacgcaccaccccgtcagtagctgaacaggagggacagctgatagaaacagaagccactggagcacctcaaaaacaccatcatacactaaatcagtaagttggcagcatcacccgacgcactttgcgccgaataaatacctgtgacggaagatcacttcgcagaataaataaatcctggtgtccctgttgataccgggaagccccgggccaacttttggcgaaaatgagacgttgatcggcacgtaagaggttccaactttcaccataatgaaataagatcactaccgggcgtattttttgagttatcgagattttcaggagctaaggaagctaaaatggagaaaaaaatcactggatataccaccgttgatatatcccaatggcatcgtaaagaacattttgaggcatttcagtcagttgctcaatgtacctataaccagaccgttcagctggatattacggcctttttaaagaccgtaaagaaaaataagcacaagttttatccggcctttattcacattcttgcccgcctgatgaatgctcatccggaattccgtatggcaatgaaagacggtgagctggtgatatgggatagtgttcacccttgttacaccgttttccatgagcaaactgaaacgttttcatcgctctggagtgaataccacgacgatttccggcagtttctacacatatattcgcaagatgtggcgtgttacggtgaaaacctggcctatttccctaaagggtttattgagaatatgtttttcgtctcagccaatccctgggtgagtttcaccagttttgatttaaacgtggccaatatggacaacttcttcgcccccgttttcaccatgggcaaatattatacgcaaggcgacaaggtgctgatgccgctggcgattcaggttcatcatgccgtttgtgatggcttccatgtcggcagaatgcttaatgaattacaacagtactgcgatgagtggcagggcggggcgtaatttggtacatctcaaataaaacgaaaggctcagtcgaaagactgggcctttcgttttatctgttgtttgtcggtgaacgctctcgttaactagctatactgatttcgtcagactcacagtcaaacatgccggtcagttggcctggtgatggcgggatcgttgtatatttcttgacaccttttcggcaccgccctaaaattctgcgtcctcataatatatgaggcgatttattacgtgtttacgaagcaaaagctaaaaccaggagctatttaatgccggcagctaagaaaaagaaactggatggcagcgtcgacatgaaaaccctgatcagaaagacctacgtgatgctggtggtggacaacgatcagaagaagtacctgaacggcctgatgagcagcatctacaagagagccgcctccatcatgacccacctgctgagctggaagaaggtgggccccaacggctatcagcacagcctgggcggcgagatcctgcccctggaaaccgcctccgacgaggagctggacgtgctgtatcagcacatcatcgacaacgacaacagcgctagaatcattagaggccccttcgccctgccccccggcaagtgcaaaaccggcatgaagagcgagaaggacctggagcagaagctgagaaagctgctggacgagggcaagctgcccctgaacctgggcgagtgggagggcacccccggcaacgacttcgtggccttcaagatcgccgtgagcagcctgaagagctgggacgacagaaacaaggtgaccgaggccaactacgccaaggccctggaggagctgaacaagaacacccccgacgaggccggcatcaaggccctgaacgagtggctggacagcaacaagctgttcctgaccaagaaggtggcctccaagttcaagaagttcggctgggacacaagaatcgccaactacccctgggagatcctgagaaccgtgaacagcgacgcctcctactgggccaagatgttcacctggcaagtggccaagcagagagtgttcggcctcagacccacaagcctgtgcaccctgcccgagctggccgtgagcgagagagagatcccctacggcgtgaactacgagaacttcagcctggagctggccggcgacagactgaagttcgtgctgggcaagagagagttccaagccctgagaaccctgtacttcaaggacctgaaggtgatccccgccaagaacagctacgtgttcaagtacagaagaggcaacaacagcaccctggacgagcaagtggaggccgtgctgaaggagatcaccctgtacagaaagaacggcaactactacgtgggcctgagcctgaacctgcaagtggacggcgacaacaagaactgcagaaccgtgaaggactactacttcttcaagagagcctccctgcccaacggcgctagaatcatggccatcgacctgggcatcaccaaccccgcctcctacgtgcacgtgagcaccaagaaaaagggccacgaggtgatcggcagcggcatcatcggcgtggacaaggagttcaacttcctgcaccccaagtacgtggccaagctgaagaagttcaaggcctccctgagcgaggccttcgccgccatcaccgagctgcaccccatcaagaaggtgctgcacagccaagaggagtggagcaagctgagataccccatcagccaaatgatcgagaagctgagcaaggagatgagacagctgagaagaggcgacctgaacgtgagaaaccacggcacaagccacgagcagatgcagttcatcctggtgtacaagaacttcgtggacctgctgaagaagtggacctacttcggcagcaagcccgccgccaagaaggagagaagaaagggcttcgaaaagcacatccggagactggagaacctgaagaaggacttcagaaagaagctggcctgcgagatcgtgagagaggcccggagaaaaggcagcgacctgatcgtgatcgaggacctggagcacttcacccccgacagcaccaaggacagcaacctgaacgagctgctgatgctgtggggcagcgggcagatcggcaagtggatcgagcacttcgccgatcagtacaacatcggcgtgctgaaggtggaccctagaatgacaagccaaatcgaccccctgaccggcaagatcggctacagaagcaagtacgacaagagaaagttcttcgtgaagagaggcaacaagatcgaggtgatccacgccgacctggccgctgccgagaacatcgccaagagagtgaccaacagaatgctgcccttcgtgaaggccgaaaagacccaagacggctacgtggcctggtgcagcgacgatgacaacagcagacggagacacgtgctggacctgaccttcggcagccacaagatcctgttccgggacgggcagcccgaggtgctggaggagaagcctagcgtgggcgaagaggtgtacctgtacagaatggacgacggctggtggcccggcgaggtgaagtacgcctacctgcagcagctggccaagcagtgcgagggcggcagcagacagaccgccaacgggcagaacgtggccacaggcggcggccccggcggcggcgccgccgccggcagcggcagccctaagaaaaaacgaaaagttggcagcggaagcaaaaggccggcggccacgaaaaaggccggccaggcaaaaaagaaaaagctcgagtacccatacgatgttccagattacgcttgagaattcggtaccttgacagctagctcagtcctaggtataatactagtagtggtagccgctgaagaatgattggcggcctatccaccgcaatgatgatctccgagccgttcggccggcatggtcccagcctcctcgctggcgccggctgggcaacatgcttcggcatggcgaatgggaccgtacgtcgacgctagcataaccccttggggcctctaaacgggtcttgaggggttttttggat

SEQ ID NO: 179 - DNA, 5583 bp, synthetic construct
  source 1..5583: mol_type = other DNA
atcataagatgatcttcttgagatcgttttggtctgcgcgtaatctcttgctctgaaaacgaaaaaaccgccttgcagggcggtttttcgaaggttctctgagctaccaactctttgaaccgaggtaactggcttggaggagcgcagtcaccaaaacttgtcctttcagtttagccttaaccggcgcatgacttcaagactaactcctctaaatcaattaccagtggctgctgccagtggtgcttttgcatgtctttccgggttggactcaagacgatagttaccggataaggcgcagcggtcggactgaacggggggttcgtgcatacagtccagcttggagcgaactgcctacccggaactgagtgtcaggcgtggaatgagacaaacgcggccataacagcggaatgacaccggtaaaccgaaaggcaggaacaggagagcgcacgagggagccgccagggggaaacgcctggtatctttatagtcctgtcgggtttcgccaccactgatttgagcgtcagatttcgtgatgcttgtcaggggggcggagcctatggaaaaacggctttgccgcggccctctcacttccctgttaagtatcttcctggcatcttccaggaaatctccgccccgttcgtaagccatttccgctcgccgcagtcgaacgaccgagcgtagcgagtcagtgagcgaggaagcggaatatatcctgtatcacatattctgctgacgcaccggtgcagccttttttctcctgccacatgaagcacttcactgacaccctcatcagtgccaacatagtaagccagtatacactccgctagcgctgatgtccggcggtgcttttgccgttacgcaccaccccgtcagtagctgaacaggagggacagctgatagaaacagaagccactggagcacctcaaaaacaccatcatacactaaatcagtaagttggcagcatcacccgacgcactttgcgccgaataaatacctgtgacggaagatcacttcgcagaataaataaatcctggtgtccctgttgataccgggaagccccgggccaacttttggcgaaaatgagacgttgatcggcacgtaagaggttccaactttcaccataatgaaataagatcactaccgggcgtattttttgagttatcgagattttcaggagctaaggaagctaaaatggagaaaaaaatcactggatataccaccgttgatatatcccaatggcatcgtaaagaacattttgaggcatttcagtcagttgctcaatgtacctataaccagaccgttcagctggatattacggcctttttaaagaccgtaaagaaaaataagcacaagttttatccggcctttattcacattcttgcccgcctgatgaatgctcatccggaattccgtatggcaatgaaagacggtgagctggtgatatgggatagtgttcacccttgttacaccgttttccatgagcaaactgaaacgttttcatcgctctggagtgaataccacgacgatttccggcagtttctacacatatattcgcaagatgtggcgtgttacggtgaaaacctggcctatttccctaaagggtttattgagaatatgtttttcgtctcagccaatccctgggtgagtttcaccagttttgatttaaacgtggccaatatggacaacttcttcgcccccgttttcaccatgggcaaatattatacgcaaggcgacaaggtgctgatgccgctggcgattcaggttcatcatgccgtttgtgatggcttccatgtcggcagaatgcttaatgaattacaacagtactgcgatgagtggcagggcggggcgtaatttggtacatctcaaataaaacgaaaggctcagtcgaaagactgggcctttcgttttatctgttgtttgtcggtgaacgctctcgttaactagctatactgatttcgtcagactcacagtcaaacatgccggtcagttggcctggtgatggcgggatcgttgtatatttcttgacaccttttcggcaccgccctaaaattctgcgtcctcataatatatgaggcgatttattacgtgtttacgaagcaaaagctaaaaccaggagctatttaatgccggcagctaagaaaaagaaactggatggcagcgtcgacatggcctccaagcacgtggtcagacccttcaacagcgtgtgcaccgccaagggcgacagactgagatacgtgaccgacaccatggactacctgaacggcgtggaaaactacctgcatcagttcatgggcgcctgcctgagctacgtggacgaaaccatcgccaaggagctgttcgacgccgaggaggccctgatcgccccctgcctgagcagattcagactggtgcccaaggagctgccctgcaacatcaagggcggcatcctggatgtgttcgccaaggagttcggcagaagccccaccgacatcgagaaggcctacctgacaagcggcttcgacggcgagaagtacagctggcagaacacaagagaactggccgtgcgggtgagcggcgagatgggcctgagcctggagcagttcggcgacctggccaagacctgcctgctgaacgacatggtgctgaactgcgacgccggcgccggcagcaacaacgccgtgagcatgctgttcggcgacggccccaagagcgactacagcatgaaggccgtgatcgcctccaaggccgccgacgctctggaagccttcaaacccaagaccctggaggcctgcagacaagtggtgatggacgtgtgcggctacagcaaccccgaggacctggtggtggcctacggcaagaccggcagccctagcgccatggctagattcatcagcgacaagaacaccggccccgtggacgagaaggtgctgctgagcaaggtgaagaagttcagaaccgacgccaagaagcaaggcagaaagaagctgatcccccacctggcctccgtgagaaactggctgctggtggccaccggcgccgacgtggagttctacgctagagcctggagcgccgcctgggccaacagcgcctccgagatcaacgccaagttcacccacaactgcaccttcatcgccgacaagatcaaggccctggccgagctggacgccatcgagaagagcaccgagggcctgggcgccgccatcagcgtgctggccgactatatgaaaaccgtggccgaggactgcagatacgtgctggccccctaccacctgggcgacattcagaccgtgagaaacttcatggccggctgcaccggcaacttcgaagaggtgttcaacggcgcctgggagaactacctggagggcatcgacttcaatcagaagccccccgtgagagagctggtgaagttcatcatcgagaagggcggcaagatcagcagcgccgccctgggcagcgcctgcaagtggctgagccaaaaggacagaatcgacaacgtgtacccccaccccttcgtgcaaggcaagcaaggctacaccttcggccctagcaacatcgagggcgccatcaacgaccccatgatgcagatcaagagcggcggcatcgccggcgaaagacccatgatgtgggtgaccaccaagctgctggacaactggaagtggatcaaccaccacctgcccttcgccaacagcagatactacgaagaggtgtactgcagcaaggagggcctggagttcaagcccgaggctcgggacggcaagcacagcttcgtgctgggcaagaccatcgacgccttcgccaccggcagaatcaagacaagcgtgggcagacagaaggccgccaaggccatcgagagaatcaaggccaacctgacccacaacgtgatcttcgaccccaagaccaccttctgcctcagaagaaaggagagccggttcgtgatcgccatcaaccacagacacctgctgacccccatgcccaaggagatgggcatcggcgacagaagcatgggcgtggatcagaacgagggcgcccccacctgctacgccatcagagagaaggtgagcgaggggggcatcctgcactccgacggcagcagaagcaaggtgatcagaatgggcaaggtgagcagcattcagagcggcaaggacgtgttcacctacagcggcgtgcacgtggaggacaaggccaacggcttcgacgtgctgtggaacgagtgcagagagttcctggctcagcacggcacccccgaggacgtggcctactatcagagaagcagagagtggtgcaagaccctgtacccctggcacggcctgtacttcagaatgctgggcaagctgatcagaaagaccaaggccgaaaccctgcccgtgttcagagagcacctgaaccacgtgctgctgaagagccccctgagccccgtgagactgcacagcctgagcctgaagagcctggagagcaccaagaaggtgatcagctgcatcagcagctacttcagcgtgtgcaacatgaaaaccgtggaggagaaggagaagggcgacaagtacctgtacggcgtgtggaacaagctgtacgcctccctggtggagagaagaaaggagagagtgaagctgagcgccggcctgatcatcagaatgtgcagagagcacggcgtgaccttcctgagagtggagggcgacctgcccaccgtggcctccggcaagagcagacagaacaacagcggcaagcaagactggtgcgctagagagctggctaagagagtggccgagatggccgtggtcgtgggcatcagatgcgtgcccgtgttccctcagtggacaagccaccaagacccctttgtgcacagcaagaagaacaaggccatgagagctagatacacaagaatcgaggcctccaagttcagcgaccgggacgccctggccctgagaaacatcatcaacagcaagagcaccggcaccgccgagtactacagactggccgtgaaaaaattcgccgagaagcacggcctgaacctgctggagatgaagaagagaaaggacggcctgtggtacagagagagactgagcggcgaggtgttcgtgcccatgagaggcggcagagtgtacctgagcacccacagactgtgcagcgacgaaacctacgtggacggcaacggcgaggtgctgtacatcaacgacgccgacgaggtggccgccctgaacgtggacctggtgagcacaggcggcggccccggcggcggcgccgccgccggcagcggcagccctaagaaaaaacgaaaagttggcagcggaagcaaaaggccggcggccacgaaaaaggccggccaggcaaaaaagaaaaagctcgagtacccatacgatgttccagattacgcttgagaattcggtaccttgacagctagctcagtcctaggtataatactagtaggcaaaagaatgtccctgctagtgggaccgcaatgatgatctccgagccgttcggccggcatggtcccagcctcctcgctggcgccggctgggcaacatgcttcggcatggcgaatgggaccgtacgtcgacgctagcataaccccttggggcctctaaacgggtcttgaggggttttttggat

SEQ ID NO: 180 - DNA, 5806 bp, synthetic construct
  source 1..5806: mol_type = other DNA
atcataagatgatcttcttgagatcgttttggtctgcgcgtaatctcttgctctgaaaacgaaaaaaccgccttgcagggcggtttttcgaaggttctctgagctaccaactctttgaaccgaggtaactggcttggaggagcgcagtcaccaaaacttgtcctttcagtttagccttaaccggcgcatgacttcaagactaactcctctaaatcaattaccagtggctgctgccagtggtgcttttgcatgtctttccgggttggactcaagacgatagttaccggataaggcgcagcggtcggactgaacggggggttcgtgcatacagtccagcttggagcgaactgcctacccggaactgagtgtcaggcgtggaatgagacaaacgcggccataacagcggaatgacaccggtaaaccgaaaggcaggaacaggagagcgcacgagggagccgccagggggaaacgcctggtatctttatagtcctgtcgggtttcgccaccactgatttgagcgtcagatttcgtgatgcttgtcaggggggcggagcctatggaaaaacggctttgccgcggccctctcacttccctgttaagtatcttcctggcatcttccaggaaatctccgccccgttcgtaagccatttccgctcgccgcagtcgaacgaccgagcgtagcgagtcagtgagcgaggaagcggaatatatcctgtatcacatattctgctgacgcaccggtgcagccttttttctcctgccacatgaagcacttcactgacaccctcatcagtgccaacatagtaagccagtatacactccgctagcgctgatgtccggcggtgcttttgccgttacgcaccaccccgtcagtagctgaacaggagggacagctgatagaaacagaagccactggagcacctcaaaaacaccatcatacactaaatcagtaagttggcagcatcacccgacgcactttgcgccgaataaatacctgtgacggaagatcacttcgcagaataaataaatcctggtgtccctgttgataccgggaagccccgggccaacttttggcgaaaatgagacgttgatcggcacgtaagaggttccaactttcaccataatgaaataagatcactaccgggcgtattttttgagttatcgagattttcaggagctaaggaagctaaaatggagaaaaaaatcactggatataccaccgttgatatatcccaatggcatcgtaaagaacattttgaggcatttcagtcagttgctcaatgtacctataaccagaccgttcagctggatattacggcctttttaaagaccgtaaagaaaaataagcacaagttttatccggcctttattcacattcttgcccgcctgatgaatgctcatccggaattccgtatggcaatgaaagacggtgagctggtgatatgggatagtgttcacccttgttacaccgttttccatgagcaaactgaaacgttttcatcgctctggagtgaataccacgacgatttccggcagtttctacacatatattcgcaagatgtggcgtgttacggtgaaaacctggcctatttccctaaagggtttattgagaatatgtttttcgtctcagccaatccctgggtgagtttcaccagttttgatttaaacgtggccaatatggacaacttcttcgcccccgttttcaccatgggcaaatattatacgcaaggcgacaaggtgctgatgccgctggcgattcaggttcatcatgccgtttgtgatggcttccatgtcggcagaatgcttaatgaattacaacagtactgcgatgagtggcagggcggggcgtaatttggtacatctcaaataaaacgaaaggctcagtcgaaagactgggcctttcgttttatctgttgtttgtcggtgaacgctctcgttaactagctatactgatttcgtcagactcacagtcaaacatgccggtcagttggcctggtgatggcgggatcgttgtatatttcttgacaccttttcggcaccgccctaaaattctgcgtcctcataatatatgaggcgatttattacgtgtttacgaagcaaaagctaaaaccaggagctatttaatgccggcagctaagaaaaagaaactggatggcagcgtcgacatgaacaacaagaacgtgaagagctacaactgtcagatcctgaccaacgacagaaagaagggcttcctggacgaaaccttcaaggccctgaacttcggcagcaaggtgtgcctggacctgggcatggccctgctgggcggcatcgacatgaacctggccatcgagatggccaaggacaagaaggaggacgtgcaagaggccgaggaaaagaacaccaaggcctccaaaaagaccaacaagaccgaggagaagaaggctgtgatcagcgccgagctgatcctggccgcctgcctgttcagaatcgtgcccaagagcaataatgaggtggtcgtggccgctgccctgcctagcctgttcgagagatacagcggcacacagatcaacgagcaagtgaaggagtacttcagcagcaacttcaacagcgagaagtacatgtggaaggacatgagatgcgagtttcagaagctggcctccgagctgaacgtgagcgagaaggacctgttcagcgacgtggccaccatggtggaggccaagttcatcggcctgaagttcggcgagatctggggcatcgtgagcaacctgttcggcaccggcgacaaggtgcccaaggaccccaagatcaacctggtgagcgactgcatcgctagaatcagagagagcaaccccgaaaccgaggacgagctcagcaagatcttcctggagtgcagcaactgcgaggacgctcagagcatgtacctgaagtacttcatcagcggcagaaagcctagcgagtacttctacgccaacaagatcggcagcagcgccaagattgatcagaagaaggtgatcagcaaactgaacaaaaacctgaagaagtacaagatcgtcctggattggaagtgcaacaatcagatcaagagctacctggccaacaagattttcgctttcaatcagaaggcctggagcgagatcttcaacgcctcctggcccatcattcagagcaagaccacaagaaacctgaacttcgtgctggagcagctgcaagacaaggctcagatcgactacagccacgagaagttctacaacaaagtgaatcagttcttcgagagcagctattttaagaccgacaacaagttcatcatcaagagcaagcacgtgggcggcgaggacctgtacaacctgtggcaagactgggacagctgggaggagaacaagatcgagaagaacctggagaagttcagcgagagcatcgaggacaacagcagcaagcccgacctgatgctgctgaagtacatccacagcatcagaaaggagatcagctgcgaccaagtgctgaacggcatcagattcgggcagcagaagttcaaaatcgagaacagattcctgaaccccatcgtggacaacagctacagctacaactggggcgacaagtccaagctgaacgggtgtatcatcagccccgacaagaaaagcaagttcaacctgaagaataacagacccgactacgactacggcatctggatggagctggaggtgctgaacaacggcaactgggagaagcaccacttcctggtgagcaacacaagattcatggaagaggtgtactgcttccccaagagcggcgccaagcccatcgtgtgcctgcccaacggcttcagaaccaagagaaacggcttcgacaacaacgtggtgctgagcgatcagcagattcagaacatcagaaacgcccccaagcacagacggagagccatcaagagacagatgagactggaggccctgagagagcagaacaagctgcccctgttcaactggaacaacgactacaacatcaacattagcaagagcaacaacgggtatagagccatcatcagcaagaagttcgagatcgagatctgcaaggacgtgaaggtggtgctgggcgtggatcagaatcagagcgccaaccacacctacgccgccttcctgctgtgcgacaagaacgaggagggcgccatcgcctactgcgggcagttcgtcagacccatcgagagcggcttcgtggtgagcaagcaagccgtgggcaagaacgagaacaagagagagttcgatcagctgagctacaacggcatcaagtggggcgagttcaacgacctgcacgagcacagaaagaacttcctggagcagtggggcaacgtgttcaaggtgaacaagttcggcgtgaagagcaacgtgagcctgaaggacagcctgatcgccctggagaagaacaaccccgtgctgtactattacaacatgaagtacctgaacttcctcaagaatatcctgtacaaaaagtccaagattgacctgttcaagatcagagaggagatcttcgaaaccatccgggacggcaagttcagcgtgatgaagctgagcagcctgagcggcctgagcttcagcatgatcagaagcgccaagagcctgatcagcagctatttcggcaacctgctggagggcaccacaaccgacgatcagaagtacgagagcgatcccgagatgttcgagctgagacagaagctggagaagaagagaaaggacaagcagaaatccaagaaggagctgaccgccaataaaatcgtgagcaaggccatcgagctgcagaagaagtacggcaccgtgctgatcgtcctggaggacatcggcaacatgacaagcaacagcaacaaaaacagcgtgaacagcgcctccatggactggctggctagaggcgtggccaataaagtgaagcagctgagcaagatgcacgagggcatcctgtactacagcatcaaccccttcatgacaagccatcagatgcccctggtgcacaacaaccccgacagagccttcaaggctagattcggcgcctgcgagcccaagtacctgttcgagaaggacttcaaggccatcaagaagttcagcaaggagtgcaaggacacaagacagaccaccgtgtactacagacaagccatgaaggacttcatggagcactacgacattagcgaggaggacatgagcaagatcgacttcctgagcttcaagagcatgatgagctacaagctcagacagagagaagaggtggagatgctgtaccccaagatgggcggcagagtgtacctgagcacccatcagctggacgacagcgagcagatgctgttcaacggcgtgaagtactggaagagcaacgccgacatcatcgccgccttcaacatcgccctggccaagatcggcaaaaacgagacaagcagcgacgccaagacccccacaggcggcggccccggcggcggcgccgccgccggcagcggcagccctaagaaaaaacgaaaagttggcagcggaagcaaaaggccggcggccacgaaaaaggccggccaggcaaaaaagaaaaagctcgagtacccatacgatgttccagattacgcttgagaattcggtaccttgacagctagctcagtcctaggtataatactagtgtggcaatgtgtgaattttgtgcctctcattggcaccgcaatgatgatctccgagccgttcggccggcatggtcccagcctcctcgctggcgccggctgggcaacatgcttcggcatggcgaatgggaccgtacgtcgacgctagcataaccccttggggcctctaaacgggtcttgaggggttttttggat

SEQ ID NO: 181 - DNA, 28 bp, synthetic construct
  source 1..28: mol_type = other DNA
cagcacaaaaggaaactcaccctaactg

SEQ ID NO: 182 - DNA, 20 bp, synthetic construct
  source 1..20: mol_type = other DNA
tgtggcgcgtggcggggtag

SEQ ID NO: 183 - RNA, 23 nt, synthetic construct
  source 1..23: mol_type = other RNA
aagtggaaatagacaccaaatct

SEQ ID NO: 184 - DNA, 8640 bp, synthetic construct
  source 1..8640: mol_type = other DNA
gacggatcgggagatctcccgatcccctatggtgcactctcagtacaatctgctctgatgccgcatagttaagccagtatctgctccctgcttgtgtgttggaggtcgctgagtagtgcgcgagcaaaatttaagctacaacaaggcaaggcttgaccgacaattgcatgaagaatctgcttagggttaggcgttttgcgctgcttcgcgatgtacgggccagatatacgcgttgacattgattattgactagttattaatagtaatcaattacggggtcattagttcatagcccatatatggagttccgcgttacataacttacggtaaatggcccgcctggctgaccgcccaacgacccccgcccattgacgtcaataatgacgtatgttcccatagtaacgccaatagggactttccattgacgtcaatgggtggagtatttacggtaaactgcccacttggcagtacatcaagtgtatcatatgccaagtacgccccctattgacgtcaatgacggtaaatggcccgcctggcattatgcccagtacatgaccttatgggactttcctacttggcagtacatctacgtattagtcatcgctattaccatggtgatgcggttttggcagtacatcaatgggcgtggatagcggtttgactcacggggatttccaagtctccaccccattgacgtcaatgggagtttgttttggcaccaaaatcaacgggactttccaaaatgtcgtaacaactccgccccattgacgcaaatgggcggtaggcgtgtacggtgggaggtctatataagcagagctctctggctaactagagaacccactgcttactggcttatcgaaattaatacgactcactatagggagacccaagctggctagcgtttaaacttaagcttgccaccatgccggcagctaagaaaaagaaactggatggcagcgtcgacatggccgtgcagaacgacagctgggacattcagagatgtcagaagctgaagctgggcaagaaggagctgagccccatcaacgccaagttctacgacgacatccaagaggactacagaaagctgttccccctgatcctgagcttcaccctgaccccctacaccttcgaggacgagaacggcgtggagcacgtggtgagcagcgagcaagtgctcaagaccctggagaacagcgtgggcaagagcctgatcgatgatgtgctgatcatcggcagcaccgtggccgagatgccccaagcctccgcctcctccttctacggcctcttctacaacaactacagctgcaacgacaaggccaagtggacccaagccaagagcgacttcctggacaagctgctgacctacaccgacgagcagctggaggccaagctggagggcgacagctgcctgagacagatgcccctggtggagtggaagaaggtgaaggagaagctgctggagggcaacgacaagaaagaggtgtgggagagcgtgagcggcaagctggccaacaaggtgaacagcagctacagcagagtgagaaaggagctggagatccaagtgagacagcccgacaacagagagtactgcagcaccctgagcgagatgctgagactgcaagtgaagagctgctatcagaagaacctggaccatcagaaggtgacccaagagctgctgaccaaggtgaacaactgcagccaaaccaaccccaagatcttcgacctgatcgccaacttcagcgacagactgtacagcatcggcaccggcctgagcaagaacgtgctgctgagaagcatcgactgcgtgaacaagggcaccctggcctccaaccccacctacaagatcgccatcgccgagctgctgaagcccgagttcagcgagatcctgaccctgaagaaggaggagctgatcagagcctacaacggcgtgaagatcagagatcagctgaagagaagaaaggtgtaccctagactgcctagcttcaagaatgactacaaggtgatgttcggcctgagcagcctggccaagttcaaaatcagagtggaggacaagaagatcaagatcgccttcagcaacggcgaggaagagctgttcatgaacagccactacttccacgacctggaggtggtgttcgacgagagcaacaagaccgccaagcagttcatcatcaagttcagacacaagctgaagtccaacaagaagttcgccgtgagcgacctgatcaccggctatgtgaaacaaatcggcctgcagaagaaaaacggctccttctatgtgaccctgatgttcaccatgaagcacgacgagaagatcctgaagctggagagattcttcaagaccgcctcccccgacatgagcaagtacaccgacctgcccgacaagatcagagtggccggcttcgacctgaacatcagcaaccccgtggtgggctgcatcgccgagatcgacaagaacggcaagggccccctgaacagcatcgacttcggcaagggcaacctggtggccggccccgacatcgtgtgccaagacaccctgatgagcaacagagtgaagagatgcaagcagctgatcttcaaggtgaaggacgccatcaaggactgcaagttcagcaacagcaacaacaccaagatgaacgacgccaccatcagcttcctgaagagactggcctccccctcccaaagccctagatgcatgattcagacctggatcaagaacctgaagaagagactgaagaagctgcacagcatcatcagagcctccggctatgtgaacattagcgagggcctgagaatgctggaggcccaagacgccatgaaaagcctgatcagcagctacgagagattccacctgaagagcggcgagatgctggccgccaagaagaacatcaccgccaacaaccggagacagaacttcagacagttcatcagcagaaagatcgcctccaagatcgtgcagtacagcaagggctgcgacgtgatcttcatcgaggacctgagcctggacttcgacagcgacaacaagaacaacagcctgatcagactgttcagcgccgacggcctgatcaagtgcatcaccgacgccgcctacaaggccggcatcggcgtggtgctggtggaccccatgggcacaagcaagaccgaccccgtgaccgccaaggtgggctacagaaacctgaagaacaagaactacctgtacgtggagcgggacggcgtgctgggctgggtggacgccgacaagatcgcctccctgaacgtgctgatcagaggcctgggccacagcatcgtgccctacaagttctacgtgaagggcaagaaaaaggacgtgatcggcgtggacctggtggagaaagaggtgggcaagagactgcagagatacttcaccatgcagcacggcagcatcaagcagcccatcttcaagatcgacaacgacaaggtgaccctgctgaagaaggccaacaagggcgacaacctgatcgagaacgccttcctgtacgcccacggcgacgacttctgcaccgccgacaaccacagaaaccaaggcaaggagatcatgcacagagtggacagcggcgagcccgtggtggagttcgacctgaccccctgcagcgagagcggctacaagagcttccaagccaagacaggcggcggccccggcggcggcgccgccgccggcagcggcagccctaagaaaaaacgaaaagttggcagcggaagcaaaaggccggcggccacgaaaaaggccggccaggcaaaaaagaaaaagctcgagtacccatacgatgttccagattacgcttgagaattccccttgagcatctgacttctggctaataaaggaaatttattttcattgcaatagtgtgttggaattttttgtgtctctcaggtaccaaaaaagatttggtgtctatttccacttgtgcttgaaccagcctctaacgagaccgtttcgcacggtgtttcgtcctttccacaagatatataaagccaagaaatcgaaatactttcaagttacggtaagcatatgatagtccattttaaaacataattttaaaactgcaaactacccaagaaattattactttctacgtcacgtattttgtactaatatctttgtgtttacagtcaaattaattccaattatctctctaacagccttgtatcgtatatgcaaatatgaaggaatcatgggaaataggccctctagagggcccgtttaaacccgctgatcagcctcgactgtgccttctagttgccagccatctgttgtttgcccctcccccgtgccttccttgaccctggaaggtgccactcccactgtcctttcctaataaaatgaggaaattgcatcgcattgtctgagtaggtgtcattctattctggggggtggggtggggcaggacagcaagggggaggattgggaagacaatagcaggcatgctggggatgcggtgggctctatggcttctgaggcggaaagaaccagctggggctctagggggtatccccacgcgccctgtagcggcgcattaagcgcggcgggtgtggtggttacgcgcagcgtgaccgctacacttgccagcgccctagcgcccgctcctttcgctttcttcccttcctttctcgccacgttcgccggctttccccgtcaagctctaaatcgggggctccctttagggttccgatttagtgctttacggcacctcgaccccaaaaaacttgattagggtgatggttcacgtagtgggccatcgccctgatagacggtttttcgccctttgacgttggagtccacgttctttaatagtggactcttgttccaaactggaacaacactcaaccctatctcggtctattcttttgatttataagggattttgccgatttcggcctattggttaaaaaatgagctgatttaacaaaaatttaacgcgaattaattctgtggaatgtgtgtcagttagggtgtggaaagtccccaggctccccagcaggcagaagtatgcaaagcatgcatctcaattagtcagcaaccaggtgtggaaagtccccaggctccccagcaggcagaagtatgcaaagcatgcatctcaattagtcagcaaccatagtcccgcccctaactccgcccatcccgcccctaactccgcccagttccgcccattctccgccccatggctgactaattttttttatttatgcagaggccgaggccgcctctgcctctgagctattccagaagtagtgaggaggcttttttggaggcctaggcttttgcaaaaagctcccgggagcttgtatatccattttcggatctgatcaagagacaggatgaggatcgtttcgcatgattgaacaagatggattgcacgcaggttctccggccgcttgggtggagaggctattcggctatgactgggcacaacagacaatcggctgctctgatgccgccgtgttccggctgtcagcgcaggggcgcccggttctttttgtcaagaccgacctgtccggtgccctgaatgaactgcaggacgaggcagcgcggctatcgtggctggccacgacgggcgttccttgcgcagctgtgctcgacgttgtcactgaagcgggaagggactggctgctattgggcgaagtgccggggcaggatctcctgtcatctcaccttgctcctgccgagaaagtatccatcatggctgatgcaatgcggcggctgcatacgcttgatccggctacctgcccattcgaccaccaagcgaaacatcgcatcgagcgagcacgtactcggatggaagccggtcttgtcgatcaggatgatctggacgaagagcatcaggggctcgcgccagccgaactgttcgccaggctcaaggcgcgcatgcccgacggcgaggatctcgtcgtgacccatggcgatgcctgcttgccgaatatcatggtggaaaatggccgcttttctggattcatcgactgtggccggctgggtgtggcggaccgctatcaggacatagcgttggctacccgtgatattgctgaagagcttggcggcgaatgggctgaccgcttcctcgtgctttacggtatcgccgctcccgattcgcagcgcatcgccttctatcgccttcttgacgagttcttctgagcgggactctggggttcgaaatgaccgaccaagcgacgcccaacctgccatcacgagatttcgattccaccgccgccttctatgaaaggttgggcttcggaatcgttttccgggacgccggctggatgatcctccagcgcggggatctcatgctggagttcttcgcccaccccaacttgtttattgcagcttataatggttacaaataaagcaatagcatcacaaatttcacaaataaagcatttttttcactgcattctagttgtggtttgtccaaactcatcaatgtatcttatcatgtctgtataccgtcgacctctagctagagcttggcgtaatcatggtcatagctgtttcctgtgtgaaattgttatccgctcacaattccacacaacatacgagccggaagcataaagtgtaaagcctggggtgcctaatgagtgagctaactcacattaattgcgttgcgctcactgcccgctttccagtcgggaaacctgtcgtgccagctgcattaatgaatcggccaacgcgcggggagaggcggtttgcgtattgggcgctcttccgcttcctcgctcactgactcgctgcgctcggtcgttcggctgcggcgagcggtatcagctcactcaaaggcggtaatacggttatccacagaatcaggggataacgcaggaaagaacatgtgagcaaaaggccagcaaaaggccaggaaccgtaaaaaggccgcgttgctggcgtttttccataggctccgcccccctgacgagcatcacaaaaatcgacgctcaagtcagaggtggcgaaacccgacaggactataaagataccaggcgtttccccctggaagctccctcgtgcgctctcctgttccgaccctgccgcttaccggatacctgtccgcctttctcccttcgggaagcgtggcgctttctcatagctcacgctgtaggtatctcagttcggtgtaggtcgttcgctccaagctgggctgtgtgcacgaaccccccgttcagcccgaccgctgcgccttatccggtaactatcgtcttgagtccaacccggtaagacacgacttatcgccactggcagcagccactggtaacaggattagcagagcgaggtatgtaggcggtgctacagagttcttgaagtggtggcctaactacggctacactagaagaacagtatttggtatctgcgctctgctgaagccagttaccttcggaaaaagagttggtagctcttgatccggcaaacaaaccaccgctggtagcggtttttttgtttgcaagcagcagattacgcgcagaaaaaaaggatctcaagaagatcctttgatcttttctacggggtctgacgctcagtggaacgaaaactcacgttaagggattttggtcatgagattatcaaaaaggatcttcacctagatccttttaaattaaaaatgaagttttaaatcaatctaaagtatatatgagtaaacttggtctgacagttaccaatgcttaatcagtgaggcacctatctcagcgatctgtctatttcgttcatccatagttgcctgactccccgtcgtgtagataactacgatacgggagggcttaccatctggccccagtgctgcaatgataccgcgagacccacgctcaccggctccagatttatcagcaataaaccagccagccggaagggccgagcgcagaagtggtcctgcaactttatccgcctccatccagtctattaattgttgccgggaagctagagtaagtagttcgccagttaatagtttgcgcaacgttgttgccattgctacaggcatcgtggtgtcacgctcgtcgtttggtatggcttcattcagctccggttcccaacgatcaaggcgagttacatgatcccccatgttgtgcaaaaaagcggttagctccttcggtcctccgatcgttgtcagaagtaagttggccgcagtgttatcactcatggttatggcagcactgcataattctcttactgtcatgccatccgtaagatgcttttctgtgactggtgagtactcaaccaagtcattctgagaatagtgtatgcggcgaccgagttgctcttgcccggcgtcaatacgggataataccgcgccacatagcagaactttaaaagtgctcatcattggaaaacgttcttcggggcgaaaactctcaaggatcttaccgctgttgagatccagttcgatgtaacccactcgtgcacccaactgatcttcagcatcttttactttcaccagcgtttctgggtgagcaaaaacaggaaggcaaaatgccgcaaaaaagggaataagggcgacacggaaatgttgaatactcatactcttcctttttcaatattattgaagcatttatcagggttattgtctcatgagcggatacatatttgaatgtatttagaaaaataaacaaataggggttccgcgcacatttccccgaaaagtgccacctgacgtc

SEQ ID NO: 185 - DNA, 21 bp, synthetic construct
  source 1..21: mol_type = other DNA
taatccagactttcacacctt

SEQ ID NO: 186 - DNA, 22 bp, synthetic construct
  source 1..22: mol_type = other DNA
cctggaatgccaaaagcaaaaa

SEQ ID NO: 187 - RNA, 36 nt, synthetic construct
  source 1..36: mol_type = other RNA
gtgcgaaacggtctcgttagagtctgattcaagcac

SEQ ID NO: 188 - RNA, 36 nt, synthetic construct
  source 1..36: mol_type = other RNA
gtgcgaagcggtctcgttagaggctggttcaagcac

SEQ ID NO: 189 - RNA, 36 nt, synthetic construct
  source 1..36: mol_type = other RNA
gtgcgaaacggcttcgttagaggctggttcaagcac

SEQ ID NO: 190 - RNA, 36 nt, synthetic construct
  source 1..36: mol_type = other RNA
gtgcgaaacggtctcgttagaggttggttcaagcac

SEQ ID NO: 191 - RNA, 36 nt, synthetic construct
  source 1..36: mol_type = other RNA
gcgtgaaacaatctcgttagaggttggtttaagcac

SEQ ID NO: 192 - RNA, 36 nt, synthetic construct
  source 1..36: mol_type = other RNA
gtgcgaaatggtctcgttagagactggctcaagcac

SEQ ID NO: 193 - RNA, 36 nt, synthetic construct
  source 1..36: mol_type = other RNA
gtgcgaagcatcctcgttagaggatggttcaagcac

SEQ ID NO: 194 - RNA, 36 nt, synthetic construct
  source 1..36: mol_type = other RNA
gtgcgagacagtatcgttagaatctggctcaagcac

SEQ ID NO: 195 - RNA, 36 nt, synthetic construct
  source 1..36: mol_type = other RNA
gtgcgaaacggtctcgttagagtctggttcaagcac

SEQ ID NO: 196 - RNA, 23 nt, synthetic construct
  source 1..23: mol_type = other RNA
gaacggctcggagatcatcattg

SEQ ID NO: 197 - DNA, 1061 bp, synthetic construct
  source 1..1061: mol_type = other DNA
tctaggccaccatggtgagcaagggcgaggagctgttcaccggggtggtgcccatcctggtcgagctggacggcgacgtaaacggccacaagttcagcgtgtccggcgagggcgagggcgatgccacctacggcaagctgaccctgaagttcatctgcaccaccggcaagctgcccgtgccctggcccaccctcgtgaccaccctgacctacggcgtgcagtgcttcagccgctaccccgaccacatgaagcagcacgacttcttcaagtccgccatgcccgaaggctacgtccaggagcgcaccatcttcttcaaggacgacggcaactacaagacccgcgccgaggtgaagttcgagggcgacaccctggtgaaccgcatcgagctgaagggcatcgacttcaaggaggacggcaacatcctggggcacaagctggagtacaactacaacagccacaacgtctatatcatggccttccctttatctcttagggataacagggtaatagagataaagtaggatggaacggctcggagatcatcattgcgtaaggcctaagatagtaatatagccatgcccgaaggctacgtccaggagcgcaccatcttcttcaaggacgacggcaactacaagacccgcgccgaggtgaagttcgagggcgacaccctggtgaaccgcatcgagctgaagggcatcgacttcaaggaggacggcaacatcctggggcacaagctggagtacaactacaacagccacaacgtctatatcatggccgacaagcagaagaacggcatcaaggtgaacttcaagatccgccacaacatcgaggacggcagcgtgcagctcgccgaccactaccagcagaacacccccatcggcgacggccccgtgctgctgcccgacaaccactacctgagcacccagtccgccctgagcaaagaccccaacgagaagcgcgatcacatggtcctgctggagttcgtgaccgccgccgggatcactctcggcatggacgagctgtacaagtaaagcggccgcgactctagtctaggcggccgc

SEQ ID NO: 198 - RNA, 23 nt, synthetic construct
  source 1..23: mol_type = other RNA
gaacggctcggagatcatcattg

SEQ ID NO: 199 - DNA, 8131 bp, synthetic construct
  source 1..8131: mol_type = other DNA
acgcgtgtagtcttatgcaatactcttgtagtcttgcaacatggtaacgatgagttagcaacatgccttacaaggagagaaaaagcaccgtgcatgccgattggtggaagtaaggtggtacgatcgtgccttattaggaaggcaacagacgggtctgacatggattggacgaaccactgaattgccgcattgcagagatattgtatttaagtgcctagctcgatacaataaacgggtctctctggttagaccagatctgagcctgggagctctctggctaactagggaacccactgcttaagcctcaataaagcttgccttgagtgcttcaagtagtgtgtgcccgtctgttgtgtgactctggtaactagagatccctcagacccttttagtcagtgtggaaaatctctagcagtggcgcccgaacagggacctgaaagcgaaagggaaaccagagctctctcgacgcaggactcggcttgctgaagcgcgcacggcaagaggcgaggggcggcgactggtgagtacgccaaaaattttgactagcggaggctagaaggagagagatgggtgcgagagcgtcagtattaagcgggggagaattagatcgcgatgggaaaaaattcggttaaggccagggggaaagaaaaaatataaattaaaacatatagtatgggcaagcagggagctagaacgattcgcagttaatcctggcctgttagaaacatcagaaggctgtagacaaatactgggacagctacaaccatcccttcagacaggatcagaagaacttagatcattatataatacagtagcaaccctctattgtgtgcatcaaaggatagagataaaagacaccaaggaagctttagacaagatagaggaagagcaaaacaaaagtaagaccaccgcacagcaagcggccactgatcttcagacctggaggaggagatatgagggacaattggagaagtgaattatataaatataaagtagtaaaaattgaaccattaggagtagcacccaccaaggcaaagagaagagtggtgcagagagaaaaaagagcagtgggaataggagctttgttccttgggttcttgggagcagcaggaagcactatgggcgcagcctcaatgacgctgacggtacaggccagacaattattgtctggtatagtgcagcagcagaacaatttgctgagggctattgaggcgcaacagcatctgttgcaactcacagtctggggcatcaagcagctccaggcaagaatcctggctgtggaaagatacctaaaggatcaacagctcctggggatttggggttgctctggaaaactcatttgcaccactgctgtgccttggaatgctagttggagtaataaatctctggaacagattggaatcacacgacctggatggagtgggacagagaaattaacaattacacaagcttaatacactccttaattgaagaatcgcaaaaccagcaagaaaagaatgaacaagaattattggaattagataaatgggcaagtttgtggaattggtttaacataacaaattggctgtggtatataaaattattcataatgatagtaggaggcttggtaggtttaagaatagtttttgctgtactttctatagtgaatagagttaggcagggatattcaccattatcgtttcagacccacctcccaaccccgaggggacccgacaggcccgaaggaatagaagaagaaggtggagagagagacagagacagatccattcgattagtgaacggatctcgacggtatcggttaacttttaaaagaaaaggggggattggggggtacagtgcaggggaaagaatagtagacataatagcaacagacatacaaactaaagaattacaaaaacaaattacaaaattcaaaattttatcgatactagtattatgcccagtacatgaccttatgggactttcctacttggcagtacatctacgtattagtcatcgctattaccatggtgatgcggttttggcagtacatcaatgggcgtggatagcggtttgactcacggggatttccaagtctccaccccattgacgtcaatgggagtttgttttggcaccaaaatcaacgggactttccaaaatgtcgtaacaactccgccccattgacgcaaatgggcggtaggcgtgtacggtgggaggtttatataagcagagctcgtttagtgaaccgtcagatcgcctggagacgccatccacgctgttttgacctccatagaagattctagagcgagaaaagccttgtttgccaccatggaacggctcggagatcatcattgcgtcgcgaggtgagcaagggcgaggagctgttcaccggggtggtgcccatcctggtcgagctggacggcgacgtaaacggccacaagttcagcgtgtccggcgagggcgagggcgatgccacctacggcaagctgaccctgaagttcatctgcaccaccggcaagctgcccgtgccctggcccaccctcgtgaccaccctgacctacggcgtgcagtgcttcagccgctaccccgaccacatgaagcagcacgacttcttcaagtccgccatgcccgaaggctacgtccaggagcgcaccatcttcttcaaggacgacggcaactacaagacccgcgccgaggtgaagttcgagggcgacaccctggtgaaccgcatcgagctgaagggcatcgacttcaaggaggacggcaacatcctggggcacaagctggagtacaactacaacagccacaacgtctatatcatggccgacaagcagaagaacggcatcaaggtgaacttcaagatccgccacaacatcgaggacggcagcgtgcagctcgccgaccactaccagcagaacacccccatcggcgacggccccgtgctgctgcccgacaaccactacctgagcacccagtccaagctgagcaaagaccccaacgagaagcgcgatcacatggtcctgctggagttcgtgaccgccgccgggatcactctcggcatggacgagctgtacaagtaagcggccgcgaaggatctgcgatcgctccggtgcccgtcagtgggcagagcgcacatcgcccacagtccccgagaagttggggggaggggtcggcaattgaacgggtgcctagagaaggtggcgcggggtaaactgggaaagtgatgtcgtgtactggctccgcctttttcccgagggtgggggagaaccgtatataagtgcagtagtcgccgtgaacgttctttttcgcaacgggtttgccgccagaacacagctgaagcttcgaggggctcgcatctctccttcacgcgcccgccgccctacctgaggccgccatccacgccggttgagtcgcgttctgccgcctcccgcctgtggtgcctcctgaactgcgtccgccgtctaggtaagtttaaagctcaggtcgagaccgggcctttgtccggcgctcccttggagcctacctagactcagccggctctccacgctttgcctgaccctgcttgctcaactctacgtctttgtttcgttttctgttctgcgccgttacagatccaagctgtgaccggcgcctacgctagatgaccgagtacaagcccacggtgcgcctcgccacccgcgacgacgtccccagggccgtacgcaccctcgccgccgcgttcgccgactaccccgccacgcgccacaccgtcgatccggaccgccacatcgagcgggtcaccgagctgcaagaactcttcctcacgcgcgtcgggctcgacatcggcaaggtgtgggtcgcggacgacggcgccgcggtggcggtctggaccacgccggagagcgtcgaagcgggggcggtgttcgccgagatcggcccgcgcatggccgagttgagcggttcccggctggccgcgcagcaacagatggaaggcctcctggcgccgcaccggcccaaggagcccgcgtggttcctggccaccgtcggcgtctcgcccgaccaccagggcaagggtctgggcagcgccgtcgtgctccccggagtggaggcggccgagcgcgccggggtgcccgccttcctggagacctccgcgccccgcaacctccccttctacgagcggctcggcttcaccgtcaccgccgacgtcgaggtgcccgaaggaccgcgcacctggtgcatgacccgcaagcccggtgcctgagtcgacaatcaacctctggattacaaaatttgtgaaagattgactggtattcttaactatgttgctccttttacgctatgtggatacgctgctttaatgcctttgtatcatgctattgcttcccgtatggctttcattttctcctccttgtataaatcctggttgctgtctctttatgaggagttgtggcccgttgtcaggcaacgtggcgtggtgtgcactgtgtttgctgacgcaacccccactggttggggcattgccaccacctgtcagctcctttccgggactttcgctttccccctccctattgccacggcggaactcatcgccgcctgccttgcccgctgctggacaggggctcggctgttgggcactgacaattccgtggtgttgtcggggaaatcatcgtcctttccttggctgctcgcctgtgttgccacctggattctgcgcgggacgtccttctgctacgtcccttcggccctcaatccagcggaccttccttcccgcggcctgctgccggctctgcggcctcttccgcgtcttcgccttcgccctcagacgagtcggatctccctttgggccgcctccccgcctggtacctttaagaccaatgacttacaaggcagctgtagatcttagccactttttaaaagaaaaggggggactggaagggctaattcactcccaacgaaaataagatctgctttttgcttgtactgggtctctctggttagaccagatctgagcctgggagctctctggctaactagggaacccactgcttaagcctcaataaagcttgccttgagtgcttcaagtagtgtgtgcccgtctgttgtgtgactctggtaactagagatccctcagacccttttagtcagtgtggaaaatctctagcagtagtagttcatgtcatcttattattcagtatttataacttgcaaagaaatgaatatcagagagtgagaggaacttgtttattgcagcttataatggttacaaataaagcaatagcatcacaaatttcacaaataaagcatttttttcactgcattctagttgtggtttgtccaaactcatcaatgtatcttatcatgtctggctctagctatcccgcccctaactccgcccagttccgcccattctccgccccatggctgactaattttttttatttatgcagaggccgaggccgcctcggcctctgagctattccagaagtagtgaggaggcttttttggaggcctagacttttgcagagacggcccaaattcgtaatcatggtcatagctgtttcctgtgtgaaattgttatccgctcacaattccacacaacatacgagccggaagcataaagtgtaaagcctggggtgcctaatgagtgagctaactcacattaattgcgttgcgctcactgcccgctttccagtcgggaaacctgtcgtgccagctgcattaatgaatcggccaacgcgcggggagaggcggtttgcgtattgggcgctcttccgcttcctcgctcactgactcgctgcgctcggtcgttcggctgcggcgagcggtatcagctcactcaaaggcggtaatacggttatccacagaatcaggggataacgcaggaaagaacatgtgagcaaaaggccagcaaaaggccaggaaccgtaaaaaggccgcgttgctggcgtttttccataggctccgcccccctgacgagcatcacaaaaatcgacgctcaagtcagaggtggcgaaacccgacaggactataaagataccaggcgtttccccctggaagctccctcgtgcgctctcctgttccgaccctgccgcttaccggatacctgtccgcctttctcccttcgggaagcgtggcgctttctcatagctcacgctgtaggtatctcagttcggtgtaggtcgttcgctccaagctgggctgtgtgcacgaaccccccgttcagcccgaccgctgcgccttatccggtaactatcgtcttgagtccaacccggtaagacacgacttatcgccactggcagcagccactggtaacaggattagcagagcgaggtatgtaggcggtgctacagagttcttgaagtggtggcctaactacggctacactagaaggacagtatttggtatctgcgctctgctgaagccagttaccttcggaaaaagagttggtagctcttgatccggcaaacaaaccaccgctggtagcggtggtttttttgtttgcaagcagcagattacgcgcagaaaaaaaggatctcaagaagatcctttgatcttttctacggggtctgacgctcagtggaacgaaaactcacgttaagggattttggtcatgagattatcaaaaaggatcttcacctagatccttttaaattaaaaatgaagttttaaatcaatctaaagtatatatgagtaaacttggtctgacagttaccaatgcttaatcagtgaggcacctatctcagcgatctgtctatttcgttcatccatagttgcctgactccccgtcgtgtagataactacgatacgggagggcttaccatctggccccagtgctgcaatgataccgcgagacccacgctcaccggctccagatttatcagcaataaaccagccagccggaagggccgagcgcagaagtggtcctgcaactttatccgcctccatccagtctattaattgttgccgggaagctagagtaagtagttcgccagttaatagtttgcgcaacgttgttgccattgctacaggcatcgtggtgtcacgctcgtcgtttggtatggcttcattcagctccggttcccaacgatcaaggcgagttacatgatcccccatgttgtgcaaaaaagcggttagctccttcggtcctccgatcgttgtcagaagtaagttggccgcagtgttatcactcatggttatggcagcactgcataattctcttactgtcatgccatccgtaagatgcttttctgtgactggtgagtactcaaccaagtcattctgagaatagtgtatgcggcgaccgagttgctcttgcccggcgtcaatacgggataataccgcgccacatagcagaactttaaaagtgctcatcattggaaaacgttcttcggggcgaaaactctcaaggatcttaccgctgttgagatccagttcgatgtaacccactcgtgcacccaactgatcttcagcatcttttactttcaccagcgtttctgggtgagcaaaaacaggaaggcaaaatgccgcaaaaaagggaataagggcgacacggaaatgttgaatactcatactcttcctttttcaatattattgaagcatttatcagggttattgtctcatgagcggatacatatttgaatgtatttagaaaaataaacaaataggggttccgcgcacatttccccgaaaagtgccacctgacgtctaagaaaccattattatcatgacattaacctataaaaataggcgtatcacgaggccctttcgtctcgcgcgtttcggtgatgacggtgaaaacctctgacacatgcagctcccggagacggtcacagcttgtctgtaagcggatgccgggagcagacaagcccgtcagggcgcgtcagcgggtgttggcgggtgtcggggctggcttaactatgcggcatcagagcagattgtactgagagtgcaccatatgcggtgtgaaataccgcacagatgcgtaaggagaaaataccgcatcaggcgccattcgccattcaggctgcgcaactgttgggaagggcgatcggtgcgggcctcttcgctattacgccagctggcgaaagggggatgtgctgcaaggcgattaagttgggtaacgccagggttttcccagtcacgacgttgtaaaacgacggccagtgccaagctg

SEQ ID NO: 200 - DNA, 8402 bp, synthetic construct
  source 1..8402: mol_type = other DNA
acgcgtgtagtcttatgcaatactcttgtagtcttgcaacatggtaacgatgagttagcaacatgccttacaaggagagaaaaagcaccgtgcatgccgattggtggaagtaaggtggtacgatcgtgccttattaggaaggcaacagacgggtctgacatggattggacgaaccactgaattgccgcattgcagagatattgtatttaagtgcctagctcgatacaataaacgggtctctctggttagaccagatctgagcctgggagctctctggctaactagggaacccactgcttaagcctcaataaagcttgccttgagtgcttcaagtagtgtgtgcccgtctgttgtgtgactctggtaactagagatccctcagacccttttagtcagtgtggaaaatctctagcagtggcgcccgaacagggacctgaaagcgaaagggaaaccagagctctctcgacgcaggactcggcttgctgaagcgcgcacggcaagaggcgaggggcggcgactggtgagtacgccaaaaattttgactagcggaggctagaaggagagagatgggtgcgagagcgtcagtattaagcgggggagaattagatcgcgatgggaaaaaattcggttaaggccagggggaaagaaaaaatataaattaaaacatatagtatgggcaagcagggagctagaacgattcgcagttaatcctggcctgttagaaacatcagaaggctgtagacaaatactgggacagctacaaccatcccttcagacaggatcagaagaacttagatcattatataatacagtagcaaccctctattgtgtgcatcaaaggatagagataaaagacaccaaggaagctttagacaagatagaggaagagcaaaacaaaagtaagaccaccgcacagcaagcggccactgatcttcagacctggaggaggagatatgagggacaattggagaagtgaattatataaatataaagtagtaaaaattgaaccattaggagtagcacccaccaaggcaaagagaagagtggtgcagagagaaaaaagagcagtgggaataggagctttgttccttgggttcttgggagcagcaggaagcactatgggcgcagcctcaatgacgctgacggtacaggccagacaattattgtctggtatagtgcagcagcagaacaatttgctgagggctattgaggcgcaacagcatctgttgcaactcacagtctggggcatcaagcagctccaggcaagaatcctggctgtggaaagatacctaaaggatcaacagctcctggggatttggggttgctctggaaaactcatttgcaccactgctgtgccttggaatgctagttggagtaataaatctctggaacagattggaatcacacgacctggatggagtgggacagagaaattaacaattacacaagcttaatacactccttaattgaagaatcgcaaaaccagcaagaaaagaatgaacaagaattattggaattagataaatgggcaagtttgtggaattggtttaacataacaaattggctgtggtatataaaattattcataatgatagtaggaggcttggtaggtttaagaatagtttttgctgtactttctatagtgaatagagttaggcagggatattcaccattatcgtttcagacccacctcccaaccccgaggggacccgacaggcccgaaggaatagaagaagaaggtggagagagagacagagacagatccattcgattagtgaacggatctcgacggtatcggttaacttttaaaagaaaaggggggattggggggtacagtgcaggggaaagaatagtagacataatagcaacagacatacaaactaaagaattacaaaaacaaattacaaaattcaaaattttatcgatactagtattatgcccagtacatgaccttatgggactttcctacttggcagtacatctacgtattagtcatcgctattaccatggtgatgcggttttggcagtacatcaatgggcgtggatagcggtttgactcacggggatttccaagtctccaccccattgacgtcaatgggagtttgttttggcaccaaaatcaacgggactttccaaaatgtcgtaacaactccgccccattgacgcaaatgggcggtaggcgtgtacggtgggaggtttatataagcagagctcgtttagtgaaccgtcagatcgcctggagacgccatccacgctgttttgacctccatagaagattctaggccaccatggtgagcaagggcgaggagctgttcaccggggtggtgcccatcctggtcgagctggacggcgacgtaaacggccacaagttcagcgtgtccggcgagggcgagggcgatgccacctacggcaagctgaccctgaagttcatctgcaccaccggcaagctgcccgtgccctggcccaccctcgtgaccaccctgacctacggcgtgcagtgcttcagccgctaccccgaccacatgaagcagcacgacttcttcaagtccgccatgcccgaaggctacgtccaggagcgcaccatcttcttcaaggacgacggcaactacaagacccgcgccgaggtgaagttcgagggcgacaccctggtgaaccgcatcgagctgaagggcatcgacttcaaggaggacggcaacatcctggggcacaagctggagtacaactacaacagccacaacgtctatatcatggccttccctttatctcttagggataacagggtaatagagataaagtaggatggaacggctcggagatcatcattgcgtaaggcctaagatagtaatatagccatgcccgaaggctacgtccaggagcgcaccatcttcttcaaggacgacggcaactacaagacccgcgccgaggtgaagttcgagggcgacaccctggtgaaccgcatcgagctgaagggcatcgacttcaaggaggacggcaacatcctggggcacaagctggagtacaactacaacagccacaacgtctatatcatggccgacaagcagaagaacggcatcaaggtgaacttcaagatccgccacaacatcgaggacggcagcgtgcagctcgccgaccactaccagcagaacacccccatcggcgacggccccgtgctgctgcccgacaaccactacctgagcacccagtccgccctgagcaaagaccccaacgagaagcgcgatcacatggtcctgctggagttcgtgaccgccgccgggatcactctcggcatggacgagctgtacaagtaaagcggccgcgactctagtctaggcggccgcgaaggatctgcgatcgctccggtgcccgtcagtgggcagagcgcacatcgcccacagtccccgagaagttggggggaggggtcggcaattgaacgggtgcctagagaaggtggcgcggggtaaactgggaaagtgatgtcgtgtactggctccgcctttttcccgagggtgggggagaaccgtatataagtgcagtagtcgccgtgaacgttctttttcgcaacgggtttgccgccagaacacagctgaagcttcgaggggctcgcatctctccttcacgcgcccgccgccctacctgaggccgccatccacgccggttgagtcgcgttctgccgcctcccgcctgtggtgcctcctgaactgcgtccgccgtctaggtaagtttaaagctcaggtcgagaccgggcctttgtccggcgctcccttggagcctacctagactcagccggctctccacgctttgcctgaccctgcttgctcaactctacgtctttgtttcgttttctgttctgcgccgttacagatccaagctgtgaccggcgcctacgctagatgaccgagtacaagcccacggtgcgcctcgccacccgcgacgacgtccccagggccgtacgcaccctcgccgccgcgttcgccgactaccccgccacgcgccacaccgtcgatccggaccgccacatcgagcgggtcaccgagctgcaagaactcttcctcacgcgcgtcgggctcgacatcggcaaggtgtgggtcgcggacgacggcgccgcggtggcggtctggaccacgccggagagcgtcgaagcgggggcggtgttcgccgagatcggcccgcgcatggccgagttgagcggttcccggctggccgcgcagcaacagatggaaggcctcctggcgccgcaccggcccaaggagcccgcgtggttcctggccaccgtcggcgtctcgcccgaccaccagggcaagggtctgggcagcgccgtcgtgctccccggagtggaggcggccgagcgcgccggggtgcccgccttcctggagacctccgcgccccgcaacctccccttctacgagcggctcggcttcaccgtcaccgccgacgtcgaggtgcccgaaggaccgcgcacctggtgcatgacccgcaagcccggtgcctgagtcgacaatcaacctctggattacaaaatttgtgaaagattgactggtattcttaactatgttgctccttttacgctatgtggatacgctgctttaatgcctttgtatcatgctattgcttcccgtatggctttcattttctcctccttgtataaatcctggttgctgtctctttatgaggagttgtggcccgttgtcaggcaacgtggcgtggtgtgcactgtgtttgctgacgcaacccccactggttggggcattgccaccacctgtcagctcctttccgggactttcgctttccccctccctattgccacggcggaactcatcgccgcctgccttgcccgctgctggacaggggctcggctgttgggcactgacaattccgtggtgttgtcggggaaatcatcgtcctttccttggctgctcgcctgtgttgccacctggattctgcgcgggacgtccttctgctacgtcccttcggccctcaatccagcggaccttccttcccgcggcctgctgccggctctgcggcctcttccgcgtcttcgccttcgccctcagacgagtcggatctccctttgggccgcctccccgcctggtacctttaagaccaatgacttacaaggcagctgtagatcttagccactttttaaaagaaaaggggggactggaagggctaattcactcccaacgaaaataagatctgctttttgcttgtactgggtctctctggttagaccagatctgagcctgggagctctctggctaactagggaacccactgcttaagcctcaataaagcttgccttgagtgcttcaagtagtgtgtgcccgtctgttgtgtgactctggtaactagagatccctcagacccttttagtcagtgtggaaaatctctagcagtagtagttcatgtcatcttattattcagtatttataacttgcaaagaaatgaatatcagagagtgagaggaacttgtttattgcagcttataatggttacaaataaagcaatagcatcacaaatttcacaaataaagcatttttttcactgcattctagttgtggtttgtccaaactcatcaatgtatcttatcatgtctggctctagctatcccgcccctaactccgcccagttccgcccattctccgccccatggctgactaattttttttatttatgcagaggccgaggccgcctcggcctctgagctattccagaagtagtgaggaggcttttttggaggcctagacttttgcagagacggcccaaattcgtaatcatggtcatagctgtttcctgtgtgaaattgttatccgctcacaattccacacaacatacgagccggaagcataaagtgtaaagcctggggtgcctaatgagtgagctaactcacattaattgcgttgcgctcactgcccgctttccagtcgggaaacctgtcgtgccagctgcattaatgaatcggccaacgcgcggggagaggcggtttgcgtattgggcgctcttccgcttcctcgctcactgactcgctgcgctcggtcgttcggctgcggcgagcggtatcagctcactcaaaggcggtaatacggttatccacagaatcaggggataacgcaggaaagaacatgtgagcaaaaggccagcaaaaggccaggaaccgtaaaaaggccgcgttgctggcgtttttccataggctccgcccccctgacgagcatcacaaaaatcgacgctcaagtcagaggtggcgaaacccgacaggactataaagataccaggcgtttccccctggaagctccctcgtgcgctctcctgttccgaccctgccgcttaccggatacctgtccgcctttctcccttcgggaagcgtggcgctttctcatagctcacgctgtaggtatctcagttcggtgtaggtcgttcgctccaagctgggctgtgtgcacgaaccccccgttcagcccgaccgctgcgccttatccggtaactatcgtcttgagtccaacccggtaagacacgacttatcgccactggcagcagccactggtaacaggattagcagagcgaggtatgtaggcggtgctacagagttcttgaagtggtggcctaactacggctacactagaaggacagtatttggtatctgcgctctgctgaagccagttaccttcggaaaaagagttggtagctcttgatccggcaaacaaaccaccgctggtagcggtggtttttttgtttgcaagcagcagattacgcgcagaaaaaaaggatctcaagaagatcctttgatcttttctacggggtctgacgctcagtggaacgaaaactcacgttaagggattttggtcatgagattatcaaaaaggatcttcacctagatccttttaaattaaaaatgaagttttaaatcaatctaaagtatatatgagtaaacttggtctgacagttaccaatgcttaatcagtgaggcacctatctcagcgatctgtctatttcgttcatccatagttgcctgactccccgtcgtgtagataactacgatacgggagggcttaccatctggccccagtgctgcaatgataccgcgagacccacgctcaccggctccagatttatcagcaataaaccagccagccggaagggccgagcgcagaagtggtcctgcaactttatccgcctccatccagtctattaattgttgccgggaagctagagtaagtagttcgccagttaatagtttgcgcaacgttgttgccattgctacaggcatcgtggtgtcacgctcgtcgtttggtatggcttcattcagctccggttcccaacgatcaaggcgagttacatgatcccccatgttgtgcaaaaaagcggttagctccttcggtcctccgatcgttgtcagaagtaagttggccgcagtgttatcactcatggttatggcagcactgcataattctcttactgtcatgccatccgtaagatgcttttctgtgactggtgagtactcaaccaagtcattctgagaatagtgtatgcggcgaccgagttgctcttgcccggcgtcaatacgggataataccgcgccacatagcagaactttaaaagtgctcatcattggaaaacgttcttcggggcgaaaactctcaaggatcttaccgctgttgagatccagttcgatgtaacccactcgtgcacccaactgatcttcagcatcttttactttcaccagcgtttctgggtgagcaaaaacaggaaggcaaaatgccgcaaaaaagggaataagggcgacacggaaatgttgaatactcatactcttcctttttcaatattattgaagcatttatcagggttattgtctcatgagcggatacatatttgaatgtatttagaaaaataaacaaataggggttccgcgcacatttccccgaaaagtgccacctgacgtctaagaaaccattattatcatgacattaacctataaaaataggcgtatcacgaggccctttcgtctcgcgcgtttcggtgatgacggtgaaaacctctgacacatgcagctcccggagacggtcacagcttgtctgtaagcggatgccgggagcagacaagcccgtcagggcgcgtcagcgggtgttggcgggtgtcggggctggcttaactatgcggcatcagagcagattgtactgagagtgcaccatatgcggtgtgaaataccgcacagatgcgtaaggagaaaataccgcatcaggcgccattcgccattcaggctgcgcaactgttgggaagggcgatcggtgcgggcctcttcgctattacgccagctggcgaaagggggatgtgctgcaaggcgattaagttgggtaacgccagggttttcccagtcacgacgttgtaaaacgacggccagtgccaagctg

SEQ ID NO: 201 - DNA, 8640 bp, synthetic construct
  source 1..8640: mol_type = other DNA
gacggatcgggagatctcccgatcccctatggtgcactctcagtacaatctgctctgatgccgcatagttaagccagtatctgctccctgcttgtgtgttggaggtcgctgagtagtgcgcgagcaaaatttaagctacaacaaggcaaggcttgaccgacaattgcatgaagaatctgcttagggttaggcgttttgcgctgcttcgcgatgtacgggccagatatacgcgttgacattgattattgactagttattaatagtaatcaattacggggtcattagttcatagcccatatatggagttccgcgttacataacttacggtaaatggcccgcctggctgaccgcccaacgacccccgcccattgacgtcaataatgacgtatgttcccatagtaacgccaatagggactttccattgacgtcaatgggtggagtatttacggtaaactgcccacttggcagtacatcaagtgtatcatatgccaagtacgccccctattgacgtcaatgacggtaaatggcccgcctggcattatgcccagtacatgaccttatgggactttcctacttggcagtacatctacgtattagtcatcgctattaccatggtgatgcggttttggcagtacatcaatgggcgtggatagcggtttgactcacggggatttccaagtctccaccccattgacgtcaatgggagtttgttttggcaccaaaatcaacgggactttccaaaatgtcgtaacaactccgccccattgacgcaaatgggcggtaggcgtgtacggtgggaggtctatataagcagagctctctggctaactagagaacccactgcttactggcttatcgaaattaatacgactcactatagggagacccaagctggctagcgtttaaacttaagcttgccaccatgccggcagctaagaaaaagaaactggatggcagcgtcgacatggccgtgcagaacgacagctgggacattcagagatgtcagaagctgaagctgggcaagaaggagctgagccccatcaacgccaagttctacgacgacatccaagaggactacagaaagctgttccccctgatcctgagcttcaccctgaccccctacaccttcgaggacgagaacggcgtggagcacgtggtgagcagcgagcaagtgctcaagaccctggagaacagcgtgggcaagagcctgatcgatgatgtgctgatcatcggcagcaccgtggccgagatgccccaagcctccgcctcctccttctacggcctcttctacaacaactacagctgcaacgacaaggccaagtggacccaagccaagagcgacttcctggacaagctgctgacctacaccgacgagcagctggaggccaagctggagggcgacagctgcctgagacagatgcccctggtggagtggaagaaggtgaaggagaagctgctggagggcaacgacaagaaagaggtgtgggagagcgtgagcggcaagctggccaacaaggtgaacagcagctacagcagagtgagaaaggagctggagatccaagtgagacagcccgacaacagagagtactgcagcaccctgagcgagatgctgagactgcaagtgaagagctgctatcagaagaacctggaccatcagaaggtgacccaagagctgctgaccaaggtgaacaactgcagccaaaccaaccccaagatcttcgacctgatcgccaacttcagcgacagactgtacagcatcggcaccggcctgagcaagaacgtgctgctgagaagcatcgactgcgtgaacaagggcaccctggcctccaaccccacctacaagatcgccatcgccgagctgctgaagcccgagttcagcgagatcctgaccctgaagaaggaggagctgatcagagcctacaacggcgtgaagatcagagatcagctgaagagaagaaaggtgtaccctagactgcctagcttcaagaatgactacaaggtgatgttcggcctgagcagcctggccaagttcaaaatcagagtggaggacaagaagatcaagatcgccttcagcaacggcgaggaagagctgttcatgaacagccactacttccacgacctggaggtggtgttcgacgagagcaacaagaccgccaagcagttcatcatcaagttcagacacaagctgaagtccaacaagaagttcgccgtgagcgacctgatcaccggctatgtgaaacaaatcggcctgcagaagaaaaacggctccttctatgtgaccctgatgttcaccatgaagcacgacgagaagatcctgaagctggagagattcttcaagaccgcctcccccgacatgagcaagtacaccgacctgcccgacaagatcagagtggccggcttcgacctgaacatcagcaaccccgtggtgggctgcatcgccgagatcgacaagaacggcaagggccccctgaacagcatcgacttcggcaagggcaacctggtggccggccccgacatcgtgtgccaagacaccctgatgagcaacagagtgaagagatgcaagcagctgatcttcaaggtgaaggacgccatcaaggactgcaagttcagcaacagcaacaacaccaagatgaacgacgccaccatcagcttcctgaagagactggcctccccctcccaaagccctagatgcatgattcagacctggatcaagaacctgaagaagagactgaagaagctgcacagcatcatcagagcctccggctatgtgaacattagcgagggcctgagaatgctggaggcccaagacgccatgaaaagcctgatcagcagctacgagagattccacctgaagagcggcgagatgctggccgccaagaagaacatcaccgccaacaaccggagacagaacttcagacagttcatcagcagaaagatcgcctccaagatcgtgcagtacagcaagggctgcgacgtgatcttcatcgaggacctgagcctggacttcgacagcgacaacaagaacaacagcctgatcagactgttcagcgccgacggcctgatcaagtgcatcaccgacgccgcctacaaggccggcatcggcgtggtgctggtggaccccatgggcacaagcaagaccgaccccgtgaccgccaaggtgggctacagaaacctgaagaacaagaactacctgtacgtggagcgggacggcgtgctgggctgggtggacgccgacaagatcgcctccctgaacgtgctgatcagaggcctgggccacagcatcgtgccctacaagttctacgtgaagggcaagaaaaaggacgtgatcggcgtggacctggtggagaaagaggtgggcaagagactgcagagatacttcaccatgcagcacggcagcatcaagcagcccatcttcaagatcgacaacgacaaggtgaccctgctgaagaaggccaacaagggcgacaacctgatcgagaacgccttcctgtacgcccacggcgacgacttctgcaccgccgacaaccacagaaaccaaggcaaggagatcatgcacagagtggacagcggcgagcccgtggtggagttcgacctgaccccctgcagcgagagcggctacaagagcttccaagccaagacaggcggcggccccggcggcggcgccgccgccggcagcggcagccctaagaaaaaacgaaaagttggcagcggaagcaaaaggccggcggccacgaaaaaggccggccaggcaaaaaagaaaaagctcgagtacccatacgatgttccagattacgcttgagaattccccttgagcatctgacttctggctaataaaggaaatttattttcattgcaatagtgtgttggaattttttgtgtctctcaggtaccaaaaacaatgatgatctccgagccgttcgtgcttgaaccagcctctaacgagaccgtttcgcacggtgtttcgtcctttccacaagatatataaagccaagaaatcgaaatactttcaagttacggtaagcatatgatagtccattttaaaacataattttaaaactgcaaactacccaagaaattattactttctacgtcacgtattttgtactaatatctttgtgtttacagtcaaattaattccaattatctctctaacagccttgtatcgtatatgcaaatatgaaggaatcatgggaaataggccctctagagggcccgtttaaacccgctgatcagcctcgactgtgccttctagttgccagccatctgttgtttgcccctcccccgtgccttccttgaccctggaaggtgccactcccactgtcctttcctaataaaatgaggaaattgcatcgcattgtctgagtaggtgtcattctattctggggggtggggtggggcaggacagcaagggggaggattgggaagacaatagcaggcatgctggggatgcggtgggctctatggcttctgaggcggaaagaaccagctggggctctagggggtatccccacgcgccctgtagcggcgcattaagcgcggcgggtgtggtggttacgcgcagcgtgaccgctacacttgccagcgccctagcgcccgctcctttcgctttcttcccttcctttctcgccacgttcgccggctttccccgtcaagctctaaatcgggggctccctttagggttccgatttagtgctttacggcacctcgaccccaaaaaacttgattagggtgatggttcacgtagtgggccatcgccctgatagacggtttttcgccctttgacgttggagtccacgttctttaatagtggactcttgttccaaactggaacaacactcaaccctatctcggtctattcttttgatttataagggattttgccgatttcggcctattggttaaaaaatgagctgatttaacaaaaatttaacgcgaattaattctgtggaatgtgtgtcagttagggtgtggaaagtccccaggctccccagcaggcagaagtatgcaaagcatgcatctcaattagtcagcaaccaggtgtggaaagtccccaggctccccagcaggcagaagtatgcaaagcatgcatctcaattagtcagcaaccatagtcccgcccctaactccgcccatcccgcccctaactccgcccagttccgcccattctccgccccatggctgactaattttttttatttatgcagaggccgaggccgcctctgcctctgagctattccagaagtagtgaggaggcttttttggaggcctaggcttttgcaaaaagctcccgggagcttgtatatccattttcggatctgatcaagagacaggatgaggatcgtttcgcatgattgaacaagatggattgcacgcaggttctccggccgcttgggtggagaggctattcggctatgactgggcacaacagacaatcggctgctctgatgccgccgtgttccggctgtcagcgcaggggcgcccggttctttttgtcaagaccgacctgtccggtgccctgaatgaactgcaggacgaggcagcgcggctatcgtggctggccacgacgggcgttccttgcgcagctgtgctcgacgttgtcactgaagcgggaagggactggctgctattgggcgaagtgccggggcaggatctcctgtcatctcaccttgctcctgccgagaaagtatccatcatggctgatgcaatgcggcggctgcatacgcttgatccggctacctgcccattcgaccaccaagcgaaacatcgcatcgagcgagcacgtactcggatggaagccggtcttgtcgatcaggatgatctggacgaagagcatcaggggctcgcgccagccgaactgttcgccaggctcaaggcgcgcatgcccgacggcgaggatctcgtcgtgacccatggcgatgcctgcttgccgaatatcatggtggaaaatggccgcttttctggattcatcgactgtggccggctgggtgtggcggaccgctatcaggacatagcgttggctacccgtgatattgctgaagagcttggcggcgaatgggctgaccgcttcctcgtgctttacggtatcgccgctcccgattcgcagcgcatcgccttctatcgccttcttgacgagttcttctgagcgggactctggggttcgaaatgaccgaccaagcgacgcccaacctgccatcacgagatttcgattccaccgccgccttctatgaaaggttgggcttcggaatcgttttccgggacgccggctggatgatcctccagcgcggggatctcatgctggagttcttcgcccaccccaacttgtttattgcagcttataatggttacaaataaagcaatagcatcacaaatttcacaaataaagcatttttttcactgcattctagttgtggtttgtccaaactcatcaatgtatcttatcatgtctgtataccgtcgacctctagctagagcttggcgtaatcatggtcatagctgtttcctgtgtgaaattgttatccgctcacaattccacacaacatacgagccggaagcataaagtgtaaagcctggggtgcctaatgagtgagctaactcacattaattgcgttgcgctcactgcccgctttccagtcgggaaacctgtcgtgccagctgcattaatgaatcggccaacgcgcggggagaggcggtttgcgtattgggcgctcttccgcttcctcgctcactgactcgctgcgctcggtcgttcggctgcggcgagcggtatcagctcactcaaaggcggtaatacggttatccacagaatcaggggataacgcaggaaagaacatgtgagcaaaaggccagcaaaaggccaggaaccgtaaaaaggccgcgttgctggcgtttttccataggctccgcccccctgacgagcatcacaaaaatcgacgctcaagtcagaggtggcgaaacccgacaggactataaagataccaggcgtttccccctggaagctccctcgtgcgctctcctgttccgaccctgccgcttaccggatacctgtccgcctttctcccttcgggaagcgtggcgctttctcatagctcacgctgtaggtatctcagttcggtgtaggtcgttcgctccaagctgggctgtgtgcacgaaccccccgttcagcccgaccgctgcgccttatccggtaactatcgtcttgagtccaacccggtaagacacgacttatcgccactggcagcagccactggtaacaggattagcagagcgaggtatgtaggcggtgctacagagttcttgaagtggtggcctaactacggctacactagaagaacagtatttggtatctgcgctctgctgaagccagttaccttcggaaaaagagttggtagctcttgatccggcaaacaaaccaccgctggtagcggtttttttgtttgcaagcagcagattacgcgcagaaaaaaaggatctcaagaagatcctttgatcttttctacggggtctgacgctcagtggaacgaaaactcacgttaagggattttggtcatgagattatcaaaaaggatcttcacctagatccttttaaattaaaaatgaagttttaaatcaatctaaagtatatatgagtaaacttggtctgacagttaccaatgcttaatcagtgaggcacctatctcagcgatctgtctatttcgttcatccatagttgcctgactccccgtcgtgtagataactacgatacgggagggcttaccatctggccccagtgctgcaatgataccgcgagacccacgctcaccggctccagatttatcagcaataaaccagccagccggaagggccgagcgcagaagtggtcctgcaactttatccgcctccatccagtctattaattgttgccgggaagctagagtaagtagttcgccagttaatagtttgcgcaacgttgttgccattgctacaggcatcgtggtgtcacgctcgtcgtttggtatggcttcattcagctccggttcccaacgatcaaggcgagttacatgatcccccatgttgtgcaaaaaagcggttagctccttcggtcctccgatcgttgtcagaagtaagttggccgcagtgttatcactcatggttatggcagcactgcataattctcttactgtcatgccatccgtaagatgcttttctgtgactggtgagtactcaaccaagtcattctgagaatagtgtatgcggcgaccgagttgctcttgcccggcgtcaatacgggataataccgcgccacatagcagaactttaaaagtgctcatcattggaaaacgttcttcggggcgaaaactctcaaggatcttaccgctgttgagatccagttcgatgtaacccactcgtgcacccaactgatcttcagcatcttttactttcaccagcgtttctgggtgagcaaaaacaggaaggcaaaatgccgcaaaaaagggaataagggcgacacggaaatgttgaatactcatactcttcctttttcaatattattgaagcatttatcagggttattgtctcatgagcggatacatatttgaatgtatttagaaaaataaacaaataggggttccgcgcacatttccccgaaaagtgccacctgacgtc

SEQ ID NO: 202 - RNA, 23 nt, synthetic construct
  source 1..23: mol_type = other RNA
caatgatgatctccgagccgttc

SEQ ID NO: 203 - DNA, 27 bp, synthetic construct
  source 1..27: mol_type = other DNA
ccaagctggctagcgtttaaacttaag

SEQ ID NO: 204 - DNA, 46 bp, synthetic construct
  source 1..46: mol_type = other DNA
tcggagatcatcattgtttttggtacctgagagacacaaaaaattc

SEQ ID NO: 205 - DNA, 25 bp, synthetic construct
  source 1..25: mol_type = other DNA
gctgcagagacaaggccaagtggac

SEQ ID NO: 206 - DNA, 34 bp, synthetic construct
  source 1..34: mol_type = other DNA
cttggccttgtctctgcagctgtagttgttgtag

SEQ ID NO: 207 - DNA, 26 bp, synthetic construct
  source 1..26: mol_type = other DNA
gcgccagaggcctgatcaagtgcatc

SEQ ID NO: 208 - DNA, 34 bp, synthetic construct
  source 1..34: mol_type = other DNA
cttgatcaggcctctggcgctgaacagtctgatc

SEQ ID NO: 209 - RNA, 24 nt, synthetic construct
  source 1..24: mol_type = other RNA
ccacgacgccagggctgcgggtcg

SEQ ID NO: 210 - RNA, 22 nt, synthetic construct
  source 1..22: mol_type = other RNA
acgccagggctgcgggtcgcca

SEQ ID NO: 211 - RNA, 22 nt, synthetic construct
  source 1..22: mol_type = other RNA
aaccaggttatgaccttgattt

SEQ ID NO: 212 - RNA, 22 nt, synthetic construct
  source 1..22: mol_type = other RNA
tgctgaggatttggaaagggtg

SEQ ID NO: 213 - RNA, 23 nt, synthetic construct
  source 1..23: mol_type = other RNA
gaaagggtgtttattcctcatgg

SEQ ID NO: 214 - RNA, 60 nt, synthetic construct
  source 1..60: mol_type = other RNA
gtgcgaaacggtctcgttagaggctggttcaagcacccacgacgccagggctgcgggtcg

SEQ ID NO: 215 - RNA, 58 nt, synthetic construct
  source 1..58: mol_type = other RNA
gtgcgaaacggtctcgttagaggctggttcaagcacacgccagggctgcgggtcgcca

SEQ ID NO: 216 - RNA, 58 nt, synthetic construct
  source 1..58: mol_type = other RNA
gtgcgaaacggtctcgttagaggctggttcaagcacaaccaggttatgaccttgattt

SEQ ID NO: 217 - RNA, 58 nt, synthetic construct
  source 1..58: mol_type = other RNA
gtgcgaaacggtctcgttagaggctggttcaagcactgctgaggatttggaaagggtg

SEQ ID NO: 218 - RNA, 59 nt, synthetic construct
  source 1..59: mol_type = other RNA
gtgcgaaacggtctcgttagaggctggttcaagcacgaaagggtgtttattcctcatgg

SEQ ID NO: 219 - DNA, 2746 bp, synthetic construct
  source 1..2746: mol_type = other DNA
tcgcgcgtttcggtgatgacggtgaaaacctctgacacatgcagctcccggagactgtcacagcttgtctgtaagcggatgccgggagcagacaagcccgtcagggcgcgtcagcgggtgttggcgggtgtcggggctggcttaactatgcggcatcagagcagattgtactgagagtgcaccatagagggcctatttcccatgattccttcatatttgcatatacgatacaaggctgttagagagataattggaattaatttgactgtaaacacaaagatattagtacaaaatacgtgacgtagaaagtaataatttcttgggtagtttgcagttttaaaattatgttttaaaatggactatcatatgcttaccgtaacttgaaagtatttcgatttcttggctttatatatcttgtggaaaggacgaaacaccgggtcttcgagaagacctgttttagagctagaaatagcaagttaaaataaggctagtccgttatcaacttgaaaaagtggcaccgagtcggtgcttttttatcccaatggcgcgccgagcttggctcgagcatggtcatagctgtttcctgtgtgaaattgttatccgctcacaattccacacaacatacgagccggaagcataaagtgtaaagcctggggtgcctaatgagtgagctaactcacattaattgcgttgcgctcactgcccgctttccagtcgggaaacctgtcgtgccagctgcattaatgaatcggccaacgcgcggggagaggcggtttgcgtattgggcgctgttccgcttcctcgctcactgactcgctgcgctcggtcgttcggctgcggcgagcggtatcagctcactcaaaggcggtaatacggttatccacagaatcaggggataacgcaggaaagaacatgtgagcaaaaggccagcaaaaggccaggaaccgtaaaaaggccgcgttgctggcgtttttccataggctccgcccccctgacgagcatcacaaaaatcgacgctcaagtcagaggtggcgaaacccgacaggactataaagataccaggcgtttccccctggaagctccctcgtgcgctctcctgttccgaccctgccgcttaccggatacctgtccgcctttctcccttcgggaagcgtggcgctttctcatagctcacgctgtaggtatctcagttcggtgtaggtcgttcgctccaagctgggctgtgtgcacgaaccccccgttcagcccgaccgctgcgccttatccggtaactatcgtcttgagtccaacccggtaagacacgacttatcgccactggcagcagccactggtaacaggattagcagagcgaggtatgtaggcggtgctacagagttcttgaagtggtggcctaactacggctacactagaagaacagtatttggtatctgcgctctgctgaagccagttaccttcggaaaaagagttggtagctcttgatccggcaaacaaaccaccgctggtagcggtggtttttttgtttgcaagcagcagattacgcgcagaaaaaaaggatctcaagaagatcctttgatcttttctacggggtctgacgctcagtggaacgaaaactcacgttaagggattttggtcatgagattatcaaaaaggatcttcacctagatccttttaaattaaaaatgaagttttaaatcaatctaaagtatatatgagtaaacttggtctgacagttagaaaaactcatcgagcatcaaatgaaactgcaatttattcatatcaggattatcaataccatatttttgaaaaagccgtttctgtaatgaaggagaaaactcaccgaggcagttccataggatggcaagatcctggtatcggtctgcgattccgactcgtccaacatcaatacaacctattaatttcccctcgtcaaaaataaggttatcaagtgagaaatcaccatgagtgacgactgaatccggtgagaatggcaaaagtttatgcatttctttccagacttgttcaacaggccagccattacgctcgtcatcaaaatcactcgcatcaaccaaaccgttattcattcgtgattgcgcctgagcgaaacgaaatacgcgatcgctgttaaaaggacaattacaaacaggaatcgaatgcaaccggcgcaggaacactgccagcgcatcaacaatattttcacctgaatcaggatattcttctaatacctggaatgctgttttcccagggatcgcagtggtgagtaaccatgcatcatcaggagtacggataaaatgcttgatggtcggaagaggcataaattccgtcagccagtttagtctgaccatctcatctgtaacatcattggcaacgctacctttgccatgtttcagaaacaactctggcgcatcgggcttcccatacaatcgatagattgtcgcacctgattgcccgacattatcgcgagcccatttatacccatataaatcagcatccatgttggaatttaatcgcggcctagagcaagacgtttcccgttgaatatggctcatactcttcctttttcaatattattgaagcatttatcagggttattgtctcatgagcggatacatatttgaatgtatttagaaaaataaacaaataggggttccgcgcacatttccccgaaaagtgccacctgacgtctaagaaaccattattatcatgacattaacctataaaaataggcgtatcacgaggcccttttgtc

SEQ ID NO: 220 - DNA, 20 bp, synthetic construct
  source 1..20: mol_type = other DNA
tgcgacgagccctcaggcga

SEQ ID NO: 221 - DNA, 22 bp, synthetic construct
  source 1..22: mol_type = other DNA
cttccagggaagggcctctccc

SEQ ID NO: 222 - DNA, 24 bp, synthetic construct
  source 1..24: mol_type = other DNA
gcccggcctgttgttttcttacat

SEQ ID NO: 223 - DNA, 28 bp, synthetic construct
  source 1..28: mol_type = other DNA
agactctggctagagttccttcttccat

SEQ ID NO: 224 - RNA, 73 nt, synthetic construct
  source 1..73: mol_type = other RNA
  modified_base 1: mod_base = OTHER; note = 2'- deoxyribose, 3'- thiophosphate
  modified_base 2: mod_base = OTHER; note = 2'- deoxyribose, 3'- thiophosphate
  modified_base 3: mod_base = OTHER; note = 2'- deoxyribose, 3'- thiophosphate
  modified_base 4: mod_base = OTHER; note = 2'- deoxyribose
  modified_base 5: mod_base = OTHER; note = 2'- deoxyribose
  modified_base 6: mod_base = OTHER; note = 2'- deoxyribose
  modified_base 7: mod_base = OTHER; note = 2'- deoxyribose
  modified_base 8: mod_base = OTHER; note = 2'- deoxyribose
  modified_base 9: mod_base = OTHER; note = 2'- deoxyribose
  modified_base 10: mod_base = OTHER; note = 2'- deoxyribose
  modified_base 11: mod_base = OTHER; note = 2'- deoxyribose
  modified_base 12: mod_base = OTHER; note = 2'- deoxyribose
  modified_base 13: mod_base = OTHER; note = 2'- deoxyribose
  modified_base 14: mod_base = OTHER; note = 2'- deoxyribose
  modified_base 71..73: mod_base = OTHER; note = 2'-O- methyl, 3'- thiophosphate
gttgcaatcccaaggtgcgaaacggtctcgttagaggctggttcaagcacgaaagggtgtttattcctcatgg

SEQ ID NO: 225 - DNA, 28 bp, synthetic construct
  source 1..28: mol_type = other DNA
caaatgtttgtatcctgtaatgctctca

SEQ ID NO: 226 - DNA, 29 bp, synthetic construct
  source 1..29: mol_type = other DNA
tggcctagtttatgttcaaatagcaagta

SEQ ID NO: 227 - DNA, 273 bp, synthetic construct
  source 1..273: mol_type = other DNA
ggagttcagacgtgtgctcttccgatctcagcacaaaaggaaactcaccctaactgtaaagtaattgtgtgttttgagactataaatatgcatgcgagaaaagccttgtttgccaccatggaacggctcggagatcatcattgcgnnnnnnngtgagcaagggcgaggagctgttcaccggggtggtgcccatcctggtcgagctggacggcgacgtaaacggccacaagttcagcgtgtccggcagatcggaagagcacacgtctgaactcc

SEQ ID NO: 228 - RNA, 24 nt, synthetic construct
  source 1..24: mol_type = other RNA
gtgagcaagggcgaggagctgttc

SEQ ID NO: 229 - RNA, 26 nt, synthetic construct
  source 1..26: mol_type = other RNA
cgcaatgatgatctccgagccgttcc

SEQ ID NO: 230 - protein, 9 aa, synthetic construct
ETFSDLWKL

SEQ ID NO: 231 - protein, 9 aa, synthetic construct
DDIEQWFTE

SEQ ID NO: 232 - protein, 9 aa, synthetic construct
SDIMDFVLK

SEQ ID NO: 233 - protein, 9 aa, synthetic construct
DLLDFSMMF

SEQ ID NO: 234 - protein, 9 aa, synthetic construct
ETLDFSLVT

SEQ ID NO: 235 - protein, 9 aa, synthetic construct
RKILNDLSS

SEQ ID NO: 236 - protein, 9 aa, synthetic construct
EAILAELKK

SEQ ID NO: 237 - protein, 9 aa, synthetic construct
DDVVQYLNS

SEQ ID NO: 238 - protein, 9 aa, synthetic construct
DDVYNYLFD

SEQ ID NO: 239 - protein, 9 aa, synthetic construct
DLFDYDFLV

SEQ ID NO: 240 - protein, 9 aa, synthetic construct
DFFDYDLLF

SEQ ID NO: 241 - protein, 9 aa, synthetic construct
EDLYSILWS

SEQ ID NO: 242 - protein, 9 aa, synthetic construct
TDLYHTLWN

SEQ ID NO: 243 - protein, 7 aa, synthetic construct
PKKKRKV

SEQ ID NO: 244 - protein, 16 aa, synthetic construct
KRPAATKKAGQAKKKK

SEQ ID NO: 245 - protein, 9 aa, synthetic construct
PAAKRVKLD

SEQ ID NO: 246 - protein, 11 aa, synthetic construct
RQRRNELKRSP

SEQ ID NO: 247 - protein, 38 aa, synthetic construct
NQSSNFGPMKGGNFGGRSSGPYGGGGQYFAKPRNQGGY

SEQ ID NO: 248 - protein, 42 aa, synthetic construct
RMRIZFKNKGKDTAELRRRRVEVSVELRKAKKDEQILKRRNV

SEQ ID NO: 249 - protein, 8 aa, synthetic construct
VSRKRPRP

SEQ ID NO: 250 - protein, 8 aa, synthetic construct
PPKKARED

SEQ ID NO: 251 - protein, 8 aa, synthetic construct
PQPKKKPL

SEQ ID NO: 252 - protein, 12 aa, synthetic construct
SALIKKKKKMAP

SEQ ID NO: 253 - protein, 5 aa, synthetic construct
DRLRR

SEQ ID NO: 254 - protein, 7 aa, synthetic construct
PKQKKRK

SEQ ID NO: 255 - protein, 10 aa, synthetic construct
RKLKKKIKKL

SEQ ID NO: 256 - protein, 10 aa, synthetic construct
REKKKFLKRR

SEQ ID NO: 257 - protein, 20 aa, synthetic construct
KRKGDEVDGVDEVAKKKSKK

SEQ ID NO: 258 - protein, 17 aa, synthetic construct
RKCLQAGMNLEARKTKK

SEQ ID NO: 259 - DNA, 270 bp, synthetic construct
  source 1..270: mol_type = other DNA
ttattattttaaaaaacagcacaaaaggaaactcaccctaactgtaaagtaattgtgtgttttgagactataaatatgcatgcgagaaaagccttgtttgccaccatggaacggctcggagatcatcattgcgnnnnnnnaccgagtacaagcccacggtgcgcctcgccacccgcgacgacgtccccagggccgtacgcaccctcgccgccgcgttcgccgactaccccgccacgcgccacaccgtcgatccggaccgccacatcgagc

SEQ ID NO: 260 - DNA, 45 bp, synthetic construct
  source 1..45: mol_type = other DNA
atatacaaagtggaaatagacaccaaatcttactggaaggcactt

SEQ ID NO: 261 - DNA, 31 bp, synthetic construct
  source 1..31: mol_type = other DNA
atatacaaagtggaaatactggaaggcactt

SEQ ID NO: 262 - DNA, 33 bp, synthetic construct
  source 1..33: mol_type = other DNA
atatacaaagtggaaatagactggaaggcactt

SEQ ID NO: 263 - DNA, 41 bp, synthetic construct
  source 1..41: mol_type = other DNA
atatacaaagtggaaatagacaccaatactggaaggcactt

SEQ ID NO: 264 - DNA, 35 bp, synthetic construct
  source 1..35: mol_type = other DNA
atatacaaagtggaaatagatactggaaggcactt

SEQ ID NO: 265 - DNA, 40 bp, synthetic construct
  source 1..40: mol_type = other DNA
atatacaaagtggaaatagacaccatactggaaggcactt

SEQ ID NO: 266 - DNA, 42 bp, synthetic construct
  source 1..42: mol_type = other DNA
atatacaaagtggaaatagacaccaaatactggaaggcactt

SEQ ID NO: 267 - DNA, 32 bp, synthetic construct
  source 1..32: mol_type = other DNA
atatacaaagtggaaattactggaaggcactt

SEQ ID NO: 268 - DNA, 34 bp, synthetic construct
  source 1..34: mol_type = other DNA
atatacaaagtggaaatagtactggaaggcactt

SEQ ID NO: 269 - DNA, 51 bp, synthetic construct
  source 1..51: mol_type = other DNA
aggatttggaaagggtgtttattcctcatggactaattatggacaggtaag

SEQ ID NO: 270 - DNA, 40 bp, synthetic construct
  source 1..40: mol_type = other DNA
aggatttggaaagggtgtttactaattatggacaggtaag

SEQ ID NO: 271 - DNA, 37 bp, synthetic construct
  source 1..37: mol_type = other DNA
aggatttggaaagggtgtttaattatggacaggtaag

SEQ ID NO: 272 - DNA, 49 bp, synthetic construct
  source 1..49: mol_type = other DNA
aggatttggaaagggtgtttattcctcatactaattatggacaggtaag

SEQ ID NO: 273 - DNA, 50 bp, synthetic construct
  source 1..50: mol_type = other DNA
aggatttggaaagggtgtttattcctcatgactaattatggacaggtaag

SEQ ID NO: 274 - DNA, 33 bp, synthetic construct
  source 1..33: mol_type = other DNA
aggatttggaaagggtgtttatggacaggtaag

SEQ ID NO: 275 - DNA, 36 bp, synthetic construct
  source 1..36: mol_type = other DNA
aggatttggaaagggtgtttattatggacaggtaag

SEQ ID NO: 276 - DNA, 44 bp, synthetic construct
  source 1..44: mol_type = other DNA
aggatttggaaagggtgtttactaattatggacaggtaagtaag

SEQ ID NO: 277 - DNA, 55 bp, synthetic construct
  source 1..55: mol_type = other DNA
aggatttggaaagggtgtttattcctcatggactaattatggacaggtaagtaag

SEQ ID NO: 278 - DNA, 37 bp, synthetic construct
  source 1..37: mol_type = other DNA
aggatttggaaagggtgtttatggacaggtaagtaag

SEQ ID NO: 279 - DNA, 22 bp, synthetic construct
  source 1..22: mol_type = other DNA
aggatttggacaggtaagtaag

SEQ ID NO: 280 - DNA, 41 bp, synthetic construct
  source 1..41: mol_type = other DNA
aggatttggaaagggtgtttaattatggacaggtaagtaag

SEQ ID NO: 281 - DNA, 45 bp, synthetic construct
  source 1..45: mol_type = other DNA
aggatttggaaagggtgtttgactaattatggacaggtaagtaag

SEQ ID NO: 282 - DNA, 22 bp, synthetic construct
  source 1..22: mol_type = other DNA
aggatttggaaaggtaagtaag

SEQ ID NO: 283 - DNA, 40 bp, synthetic construct
  source 1..40: mol_type = other DNA
aggatttggaaagggtgtttattatggacaggtaagtaag

SEQ ID NO: 284 - DNA, 43 bp, synthetic construct
  source 1..43: mol_type = other DNA
aggatttggaaagggtgttactaattatggacaggtaagtaag

SEQ ID NO: 285 - DNA, 23 bp, synthetic construct
  source 1..23: mol_type = other DNA
aggattatggacaggtaagtaag

SEQ ID NO: 286 - DNA, 44 bp, synthetic construct
  source 1..44: mol_type = other DNA
aggatttggaaagggtgttgactaattatggacaggtaagtaag

SEQ ID NO: 287 - DNA, 270 bp, synthetic construct
  source 1..270: mol_type = other DNA
gctcgatgtggcggtccggatcgacggtgtggcgcgtggcggggtagtcggcgaacgcggcggcgagggtgcgtacggccctggggacgtcgtcgcgggtggcgaggcgcaccgtgggcttgtactcggtnnnnnnncgcaatgatgatctccgagccgttccatggtggcaaacaaggcttttctcgcatgcatatttatagtctcaaaacacacaattactttacagttagggtgagtttccttttgtgctgttttttaaaataataa